European Patent Specification EP 3 820 991 B1, published September 2, 2026. Title: ENGINEERED PANTOTHENATE KINASE VARIANT ENZYMES. Applicant: CODEXIS, INC. The sequence listing filed with the application follows.

SEQUENCE LISTING (276 sequences)

SEQ ID NO: 1 - DNA, 951 bp, Artificial Sequence
  Pantothenate Kinase from Escherichia coli
atgagcatcaaagagcagaccctgatgaccccgtacctgcagttcgaccgtaaccaatgggcggcgctgcgtgatagcgttccgatgaccctgagcgaggacgaaatcgcgcgtctgaagggtattaacgaggatctgagcctggaggaagtggcggaaatctacctgccgctgagccgtctgctgaacttctatattagcagcaacctgcgtcgtcaggcggttctggaacaatttctgggtaccaacggccagcgtatcccgtatatcattagcattgcgggtagcgtggcggttggcaaaagcaccaccgcgcgtgtgctgcaggcgctgctgagccgttggccggagcaccgtcgtgttgaactgatcaccaccgacggcttcctgcacccgaaccaagtgctgaaggagcgtggtctgatgaagaaaaagggcttcccggaaagctacgatatgcaccgtctggtgaaatttgttagcgacctgaagagcggtgtgccgaacgttaccgcgccggtgtacagccacctgatctatgatgttattccggacggcgataaaaccgtggttcagccggacatcctgattctggagggtctgaacgtgctgcaaagcggcatggactatccgcacgatccgcaccacgtgtttgttagcgacttcgtggattttagcatctacgttgacgcgccggaggatctgctgcagacctggtatattaaccgtttcctgaaatttcgtgagggtgcgttcaccgacccggatagctactttcacaactatgcgaaactgaccaaggaagaggcgatcaaaaccgcgatgaccctgtggaaggagatcaactggctgaacctgaagcaaaacattctgccgacccgtgaacgtgcgagcctgattctgaccaaaagcgcgaaccacgcggtggaggaagttcgtctgcgtaagtaa

SEQ ID NO: 2 - protein, 316 aa, Artificial Sequence
  Pantothenate Kinase from Escherichia coli
MSIKEQTLMTPYLQFDRNQWAALRDSVPMTLSEDEIARLKGINEDLSLEEVAEIYLPLSRLLNFYISSNLRRQAVLEQFLGTNGQRIPYIISIAGSVAVGKSTTARVLQALLSRWPEHRRVELITTDGFLHPNQVLKERGLMKKKGFPESYDMHRLVKFVSDLKSGVPNVTAPVYSHLIYDVIPDGDKTVVQPDILILEGLNVLQSGMDYPHDPHHVFVSDFVDFSIYVDAPEDLLQTWYINRFLKFREGAFTDPDSYFHNYAKLTKEEAIKTAMTLWKEINWLNLKQNILPTRERASLILTKSANHAVEEVRLRK

SEQ ID NO: 3 - DNA, 951 bp, Artificial Sequence
  Pantothenate Kinase from Escherichia coli variant
atgagcatcaaagagcagaccctgatgaccccgtacctgcagttcgaccgtaaccaatgggcggcgctgcgtgatagcgttccgatgaccctgagcgaggacgaaatcgcgcgtctgaagggtattaacgaggatctgagcctggaggaagtggcggaaatctacctgccgctgagccgtctgctgaacttctatattagcagcaacctgcgtcgtcaggcggttctggaacaatttctgggtaccaacggccagcgtatcccgtatatcattagcattgcgggtagcgtggcggttggcaaaagcaccaccgcgcgtgtgctgcaggcgctgctgagccgttggccggagcaccgtcgtgttgaactgatcaccaccgacggcttcctgcacccgaaccaagtgctgaaggagcgtggtctgatgaagaaaaagggtttcccggaaagctacgatatgcaccgtctggtgaaatttgttagcgacctgaagagcggtgtgccgaacgttaccgcgccggtgtacagccacctgatctatgatgttattccggacggcgataaaaccgtggttcagccggacatcctgattctggagggtctgaacgtgctgcaaagcggcatggactatccgcacgatccgcaccacgtgtttgttagcgacttcgtggattttagcatctacgttgacgcgccggaggatctgctgcagacctggttcattaaccgtttcctgaaatttcgtgagggtgcgttcaccgacccggatagctactttcacaactatgcgaaactgaccaaggaagaggcgatcaaaaccgcgatgaccatgtggaaggagatgatgtggctgaacctgaagcaaaacattctgccgacccgtgaacgtgcgagcctgattctgaccaaaagcgcgaaccacgcggtggaggaagttcgtctgcgtaagtaa

SEQ ID NO: 4 - protein, 316 aa, Artificial Sequence
  Pantothenate Kinase from Escherichia coli variant
MSIKEQTLMTPYLQFDRNQWAALRDSVPMTLSEDEIARLKGINEDLSLEEVAEIYLPLSRLLNFYISSNLRRQAVLEQFLGTNGQRIPYIISIAGSVAVGKSTTARVLQALLSRWPEHRRVELITTDGFLHPNQVLKERGLMKKKGFPESYDMHRLVKFVSDLKSGVPNVTAPVYSHLIYDVIPDGDKTVVQPDILILEGLNVLQSGMDYPHDPHHVFVSDFVDFSIYVDAPEDLLQTWFINRFLKFREGAFTDPDSYFHNYAKLTKEEAIKTAMTMWKEMMWLNLKQNILPTRERASLILTKSANHAVEEVRLRK

SEQ ID NO: 5 - DNA, 951 bp, Artificial Sequence
  Pantothenate Kinase from Escherichia coli variant
atgagcatcaaagagcagaccctgatgaccccgtacctgcagttcgaccgtaaccaatgggcggcgctgcgtgatagcgttccgatgaccctgagcgaggacgaaatcgcgcgtctgaagggtattaacgaggatctgagcctggaggaagtggcggaaatctacctgccgctgagccgtctgctgaacttctatattagcagcaacctgcgtcgtcaggcggttctggaacaatttctgggtaccaacggccagcgtatcccgtatatcattagcattgcgggtagcgtggcggttggcaaaagcaccaccgcgcgtgtgctgcaggcgctgctgagccgttggccggagcaccgtcgtgttgaactgatcaccaccgacggcttcctgcacccgaaccaagtgctgaaggagcgtggtctgatgaagaaaaagggtttcccggaaagctacgatatgcaccgtctggtgaaatttgttagcgacctgaagagcggtgtgccgaacgttaccgcgccggtgtacagccacctgatctatgatgttattccggacggcgataaaaccgtggttcagccggacatcctgattctggagggtctgaacgtgctgcaaagcggcatggactatccgcacgatccgcaccacgtgtttgttagcgacttcgtggattttagcatctacgttgacgcgccggaggatctgctgcagacctggttcattaaccgtttcctgaaatttcgtgagggtgcgttcaccgacccggatagctactttcacaactatgcgaaactgaccaaggaagaggcgatcaaaaccgcgatgaccatttggaaggagattaactggctgaacctgaagcaaaacattctgccgacccgtgaacgtgcgagcctgattctgaccaaaagcgcgaaccacgcggtggaggaagttcgtctgcgtaagtaa

SEQ ID NO: 6 - protein, 316 aa, Artificial Sequence
  Pantothenate Kinase from Escherichia coli variant
MSIKEQTLMTPYLQFDRNQWAALRDSVPMTLSEDEIARLKGINEDLSLEEVAEIYLPLSRLLNFYISSNLRRQAVLEQFLGTNGQRIPYIISIAGSVAVGKSTTARVLQALLSRWPEHRRVELITTDGFLHPNQVLKERGLMKKKGFPESYDMHRLVKFVSDLKSGVPNVTAPVYSHLIYDVIPDGDKTVVQPDILILEGLNVLQSGMDYPHDPHHVFVSDFVDFSIYVDAPEDLLQTWFINRFLKFREGAFTDPDSYFHNYAKLTKEEAIKTAMTIWKEINWLNLKQNILPTRERASLILTKSANHAVEEVRLRK

SEQ ID NO: 7 - DNA, 951 bp, Artificial Sequence
  Pantothenate Kinase from Escherichia coli variant
atgagcatcaaagagcagaccctgatgaccccgtacctgcagttcgaccgtaaccaatgggcggcgctgcgtgatagcgttccgatgaccctgagcgaggacgaaatcgcgcgtctgaagggtattaacgaggatctgagcctggaggaagtggcggaaatctacctgccgctgagccgtctgctgaacttctatattagcagcaacctgcgtcgtcaggcggttctggaacaatttctgggtaccaacggccagcgtatcccgtatatcattagcattgcgggtagcgtggcggttggcaaaagcaccaccgcgcgtgtgctgcaggcgctgctgagccgttggccggagcaccgtcgtgttgaactgatcaccaccgacggcttcctgcacccgaaccaagtgctgaaggagcgtggtctgatgaagaaaaagggcttcccggaaagctacgatatgcaccgtctggtgaaatttgttagcgacctgaagagcggtgtgccgaacgttaccgcgccggtgtacagccacctgatctatgatgttattccggacggcgataaaaccgtggttcagccggacatcctgattctggagggtctgaacgtgctgcaaagcggcatggactatccgcacgatccgcaccacgtgtttgttagcgacttcgtggattttagcatctacgttgacgcgccggaggatctgctgcagacctggtacattaaccgtttcctgaaatttcgtgagggtgcgttcaccgacccggatagctactttcacaactatgcgaaactgaccaaggaagaggcgatcaaaaccgcgatgaccatgtggaaggagattaactggctgaacctgaagcaaaacattctgccgacccgtgaacgtgcgagcctgattctgaccaaaagcgcgaaccacgcggtggaggaagttcgtctgcgtaagtaa

SEQ ID NO: 8 - protein, 316 aa, Artificial Sequence
  Pantothenate Kinase from Escherichia coli variant
MSIKEQTLMTPYLQFDRNQWAALRDSVPMTLSEDEIARLKGINEDLSLEEVAEIYLPLSRLLNFYISSNLRRQAVLEQFLGTNGQRIPYIISIAGSVAVGKSTTARVLQALLSRWPEHRRVELITTDGFLHPNQVLKERGLMKKKGFPESYDMHRLVKFVSDLKSGVPNVTAPVYSHLIYDVIPDGDKTVVQPDILILEGLNVLQSGMDYPHDPHHVFVSDFVDFSIYVDAPEDLLQTWYINRFLKFREGAFTDPDSYFHNYAKLTKEEAIKTAMTMWKEINWLNLKQNILPTRERASLILTKSANHAVEEVRLRK

SEQ ID NO: 9 - DNA, 951 bp, Artificial Sequence
  Pantothenate Kinase from Escherichia coli variant
atgagcatcaaagagcagaccctgatgaccccgtacctgcagttcgaccgtaaccaatgggcggcgctgcgtgatagcgttccgatgaccctgagcgaggacgaaatcgcgcgtctgaagggtattaacgaggatctgagcctggaggaagtggcggaaagctacctgccgctgagccgtctgctgaacttctatattagcagcaacctgcgtcgtcaggcggttctggaacaatttctgggtaccaacggccagcgtatcccgtatatcattagcattgcgggtagcgtggcggttggcaaaagcaccaccgcgcgtgtgctgcaggcgctgctgagccgttggccggagcaccgtcgtgttgaactgatcaccaccgacggcttcctgcacccgaaccaagtgctgaaggagcgtggtctgatgaagaaaaagggtttcccggaaagctacgatatgcaccgtctggtgaaatttgttagcgacctgaagagcggtgtgccgaacgttaccgcgccggtgtacagccacctgatctatgatgttattccggacggcgataaaaccgtggttcagccggacatcctgattctggagggtctgaacgtgctgcaaagcggcatggactatccgcacgatccgcaccacgtgtttgttagcgacttcgtggattttagcatctacgttgacgcgccggaggatctgctgcagacctggtggattaaccgtttcctgaaatttcgtgagggtgcgttcaccgacccggatagctactttcacaactatgcgaaactgaccaaggaagaggcgatcaaaaccgcgatgaccatgtggaaggagatgaactggctgaacctgaagcaaaacattctgccgacccgtgaacgtgcgagcctgattctgaccaaaagcgcgaaccacgcggtggaggaagttcgtctgcgtaagtaa

SEQ ID NO: 10 - protein, 316 aa, Artificial Sequence
  Pantothenate Kinase from Escherichia coli variant
MSIKEQTLMTPYLQFDRNQWAALRDSVPMTLSEDEIARLKGINEDLSLEEVAESYLPLSRLLNFYISSNLRRQAVLEQFLGTNGQRIPYIISIAGSVAVGKSTTARVLQALLSRWPEHRRVELITTDGFLHPNQVLKERGLMKKKGFPESYDMHRLVKFVSDLKSGVPNVTAPVYSHLIYDVIPDGDKTVVQPDILILEGLNVLQSGMDYPHDPHHVFVSDFVDFSIYVDAPEDLLQTWWINRFLKFREGAFTDPDSYFHNYAKLTKEEAIKTAMTMWKEMNWLNLKQNILPTRERASLILTKSANHAVEEVRLRK

SEQ ID NO: 11 - DNA, 951 bp, Artificial Sequence
  Pantothenate Kinase from Escherichia coli variant
atgagcatcaaagagcagaccctgatgaccccgtacctgcagttcgaccgtaaccaatgggcggcgctgcgtgatagcgttccgatgaccctgagcgaggacgaaatcgcgcgtctgaagggtattaacgaggatctgagcctggaggaagtggcggaaatctacctgccgctgagccgtctgctgaacttctatattagcagcaacctgcgtcgtcaggcggttctggaacaatttctgggtaccaacggccagcgtatcccgtatatcattagcattgcgggtagcgtggcggttggcaaaagcaccaccgcgcgtgtgctgcaggcgctgctgagccgttggccggagcaccgtcgtgttgaactgatcaccaccgacggcttcctgcacccgaaccaagtgctgaaggagcgtggtctgatgaagaaaaagggcttcccggaaagctacgatatgcaccgtctggtgaaatttgttagcgacctgaagagcggtgtgccgaacgttaccgcgccggtgtacagccacctgatctatgatgttattccggacggcgataaaaccgtggttcagccggacatcctgattctggagggtctgaacgtgctgcaaagcggcatggactatccgcacgatccgcaccacgtgtttgttagcgacttcgtggattttagcatctacgttgacgcgccggaggatctgctgcagacctggttcattaaccgtttcctgaaatttcgtgagggtgcgttcaccgacccggatagctactttcacaactatgcgaaactgaccaaggaagaggcgatcaaaaccgcgatgaccatgtggaaggagatgaactggctgaacctgaagcaaaacattctgccgacccgtgaacgtgcgagcctgattctgaccaaaagcgcgaaccacgcggtggaggaagttcgtctgcgtaagtaa

SEQ ID NO: 12 - protein, 316 aa, Artificial Sequence
  Pantothenate Kinase from Escherichia coli variant
MSIKEQTLMTPYLQFDRNQWAALRDSVPMTLSEDEIARLKGINEDLSLEEVAEIYLPLSRLLNFYISSNLRRQAVLEQFLGTNGQRIPYIISIAGSVAVGKSTTARVLQALLSRWPEHRRVELITTDGFLHPNQVLKERGLMKKKGFPESYDMHRLVKFVSDLKSGVPNVTAPVYSHLIYDVIPDGDKTVVQPDILILEGLNVLQSGMDYPHDPHHVFVSDFVDFSIYVDAPEDLLQTWFINRFLKFREGAFTDPDSYFHNYAKLTKEEAIKTAMTMWKEMNWLNLKQNILPTRERASLILTKSANHAVEEVRLRK

SEQ ID NO: 13 - DNA, 951 bp, Artificial Sequence
  Pantothenate Kinase from Escherichia coli variant
atgagcatcaaagagcagaccctgatgaccccgtacctgcagttcgaccgtaaccaatgggcggcgctgcgtgatagcgttccgatgaccctgagcgaggacgaaatcgcgcgtctgaagggtattaacgaggatctgagcctggaggaagtggcggaaatctacctgccgctgagccgtctgctgaacttctatattagcagcaacctgcgtcgtcaggcggttctggaacaatttctgggtaccaacggccagcgtatcccgtatatcattagcattgcgggtagcgtggcggttggcaaaagcaccaccgcgcgtgtgctgcaggcgctgctgagccgttggccggagcaccgtcgtgttgaactgatcaccaccgacggcttcctgcacccgaaccaagtgctgaaggagcgtggtctgatgaagaaaaagggcttcccggaaagctacgatatgcaccgtctggtgaaatttgttagcgacctgaagagcggtgtgccgaacgttaccgcgccggtgtacagccacctgatctatgatgttattccggacggcgataaaaccgtggttcagccggacatcctgattctggagggtctgaacgtgctgcaaagcggcatggactatccgcacgatccgcaccacgtgtttgttagcgacttcgtggattttagcatctacgttgacgcgccggaggatctgctgcagacctggtacattaaccgtttcctgaaatttcgtgagggtgcgttcaccgacccggatagctactttcacaactatgcgaaactgaccaaggaagaggcgatcaaaaccgcgatgaccatgtggaaggagatgaactggctgaacctgaagcaaaacattctgccgacccgtgaacgtgcgagcctgattctgaccaaaagcgcgaaccacgcggtggaggaagttcgtctgcgtaagtaa

SEQ ID NO: 14 - protein, 316 aa, Artificial Sequence
  Pantothenate Kinase from Escherichia coli variant
MSIKEQTLMTPYLQFDRNQWAALRDSVPMTLSEDEIARLKGINEDLSLEEVAEIYLPLSRLLNFYISSNLRRQAVLEQFLGTNGQRIPYIISIAGSVAVGKSTTARVLQALLSRWPEHRRVELITTDGFLHPNQVLKERGLMKKKGFPESYDMHRLVKFVSDLKSGVPNVTAPVYSHLIYDVIPDGDKTVVQPDILILEGLNVLQSGMDYPHDPHHVFVSDFVDFSIYVDAPEDLLQTWYINRFLKFREGAFTDPDSYFHNYAKLTKEEAIKTAMTMWKEMNWLNLKQNILPTRERASLILTKSANHAVEEVRLRK

SEQ ID NO: 15 - DNA, 951 bp, Artificial Sequence
  Pantothenate Kinase from Escherichia coli variant
atgagcatcaaagagcagaccctgatgaccccgtacctgcagttcgaccgtaaccaatgggcggcgctgcgtgatagcgttccgatgaccctgagcgaggacgaaatcgcgcgtctgaagggtattaacgaggatctgagcctggaggaagtggcggaaatctacctgccgctgagccgtctgctgaacttctatattagcagcaacctgcgtcgtcaggcggttctggaacaatttctgggtaccaacggccagcgtatcccgtatatcattagcattgcgggtagcgtggcggttggcaaaagcaccaccgcgcgtgtgctgcaggcgctgctgagccgttggccggagcaccgtcgtgttgaactgatcaccaccgacggcttcctgcacccgaaccaagtgctgaaggagcgtggtctgatgaagaaaaagggtttcccggaaagctacgatatgcaccgtctggtgaaatttgttagcgacctgaagagcggtgtgccgaacgttaccgcgccggtgtacagccacctgatctatgatgttattccggacggcgataaaaccgtggttcagccggacatcctgattctggagggtctgaacgtgctgcaaagcggcatggactatccgcacgatccgcaccacgtgtttgttagcgacttcgtggattttagcatctacgttgacgcgccggaggatctgctgcagacctggttcattaaccgtttcctgaaatttcgtgagggtgcgttcaccgacccggatagctactttcacaactatgcgaaactgaccaaggaagaggcgatcaaaaccgcgatgaccttgtggaaggagatgaactggctgaacctgaagcaaaacattctgccgacccgtgaacgtgcgagcctgattctgaccaaaagcgcgaaccacgcggtggaggaagttcgtctgcgtaagtaa

SEQ ID NO: 16 - protein, 316 aa, Artificial Sequence
  Pantothenate Kinase from Escherichia coli variant
MSIKEQTLMTPYLQFDRNQWAALRDSVPMTLSEDEIARLKGINEDLSLEEVAEIYLPLSRLLNFYISSNLRRQAVLEQFLGTNGQRIPYIISIAGSVAVGKSTTARVLQALLSRWPEHRRVELITTDGFLHPNQVLKERGLMKKKGFPESYDMHRLVKFVSDLKSGVPNVTAPVYSHLIYDVIPDGDKTVVQPDILILEGLNVLQSGMDYPHDPHHVFVSDFVDFSIYVDAPEDLLQTWFINRFLKFREGAFTDPDSYFHNYAKLTKEEAIKTAMTLWKEMNWLNLKQNILPTRERASLILTKSANHAVEEVRLRK

SEQ ID NO: 17 - DNA, 951 bp, Artificial Sequence
  Pantothenate Kinase from Escherichia coli variant
atgagcatcaaagagcagaccctgatgaccccgtacctgcagttcgaccgtaaccaatgggcggcgctgcgtgatagcgttccgatgaccctgagcgaggacgaaatcgcgcgtctgaagggtattaacgaggatctgagcctggaggaagtggcggaaatctacctgccgctgagccgtctgctgaacttctatattagcagcaacctgcgtcgtcaggcggttctggaacaatttctgggtaccaacggccagcgtatcccgtatatcattagcattgcgggtagcgtggcggttggcaaaagcaccaccgcgcgtgtgctgcaggcgctgctgagccgttggccggagcaccgtcgtgttgaactgatcaccaccgacggcttcctgcacccgaaccaagtgctgaaggagcgtggtctgatgaagaaaaagggtttcccggaaagctacgatatgcaccgtctggtgaaatttgttagcgacctgaagagcggtgtgccgaacgttaccgcgccggtgtacagccacctgatctatgatgttattccggacggcgataaaaccgtggttcagccggacatcctgattctggagggtctgaacgtgctgcaaagcggcatggactatccgcacgatccgcaccacgtgtttgttagcgacttcgtggattttagcatctacgttgacgcgccggaggatctgctgcagacctggtatattaaccgtttcctgaaatttcgtgagggtgcgttcaccgacccggatagctactttcacaactatgcgaaactgaccaaggaagaggcgatcaaaaccgcgatgaccatttggaaggagttgaactggctgaacctgaagcaaaacattctgccgacccgtgaacgtgcgagcctgattctgaccaaaagcgcgaaccacgcggtggaggaagttcgtctgcgtaagtaa

SEQ ID NO: 18 - protein, 316 aa, Artificial Sequence
  Pantothenate Kinase from Escherichia coli variant
MSIKEQTLMTPYLQFDRNQWAALRDSVPMTLSEDEIARLKGINEDLSLEEVAEIYLPLSRLLNFYISSNLRRQAVLEQFLGTNGQRIPYIISIAGSVAVGKSTTARVLQALLSRWPEHRRVELITTDGFLHPNQVLKERGLMKKKGFPESYDMHRLVKFVSDLKSGVPNVTAPVYSHLIYDVIPDGDKTVVQPDILILEGLNVLQSGMDYPHDPHHVFVSDFVDFSIYVDAPEDLLQTWYINRFLKFREGAFTDPDSYFHNYAKLTKEEAIKTAMTIWKELNWLNLKQNILPTRERASLILTKSANHAVEEVRLRK

SEQ ID NO: 19 - DNA, 951 bp, Artificial Sequence; identical to SEQ ID NO: 11
  Pantothenate Kinase from Escherichia coli variant

SEQ ID NO: 20 - protein, 316 aa, Artificial Sequence; identical to SEQ ID NO: 12
  Pantothenate Kinase from Escherichia coli variant

SEQ ID NO: 21 - DNA, 951 bp, Artificial Sequence
  Pantothenate Kinase from Escherichia coli variant
atgagcatcaaagagcagaccctgatgaccccgtacctgcagttcgaccgtaaccaatgggcggcgctgcgtgatagcgttccgatgaccctgagcgaggacgaaatcgcgcgtctgaagggtattaacgaggatctgagcctggaggaagtggcggaaatctacctgccgctgagccgtctgctgaacttctatattagcagcaacctgcgtcgtcaggcggttctggaacaatttctgggtaccaacggccagcgtatcccgtatatcattagcattgcgggtagcgtggcggttggcaaaagcaccaccgcgcgtgtgctgcaggcgctgctgagccgttggccggagcaccgtcgtgttgaactgatcaccaccgacggcttcctgcacccgaaccaagtgctgaaggagcgtggtctgatgaagaaaaagggtttcccggaaagctacgatatgcaccgtctggtgaaatttgttagcgacctgaagagcggtgtgccgaacgttaccgcgccggtgtacagccacctgatctatgatgttattccggacggcgataaaaccgtggttcagccggacatcctgattctggagggtctgaacgtgctgcaaagcggcatggactatccgcacgatccgcaccacgtgtttgttagcgacttcgtggattttagcatctacgttgacgcgccggaggatctgctgcagacctggtggattaaccgtttcctgaaatttcgtgagggtgcgttcaccgacccggatagctactttcacaactatgcgaaactgaccaaggaagaggcgatcaaaaccgcgatgaccatttggaaggagatgaactggctgaacctgaagcaaaacattctgccgacccgtgaacgtgcgagcctgattctgaccaaaagcgcgaaccacgcggtggaggaagttcgtctgcgtaagtaa

SEQ ID NO: 22 - protein, 316 aa, Artificial Sequence
  Pantothenate Kinase from Escherichia coli variant
MSIKEQTLMTPYLQFDRNQWAALRDSVPMTLSEDEIARLKGINEDLSLEEVAEIYLPLSRLLNFYISSNLRRQAVLEQFLGTNGQRIPYIISIAGSVAVGKSTTARVLQALLSRWPEHRRVELITTDGFLHPNQVLKERGLMKKKGFPESYDMHRLVKFVSDLKSGVPNVTAPVYSHLIYDVIPDGDKTVVQPDILILEGLNVLQSGMDYPHDPHHVFVSDFVDFSIYVDAPEDLLQTWWINRFLKFREGAFTDPDSYFHNYAKLTKEEAIKTAMTIWKEMNWLNLKQNILPTRERASLILTKSANHAVEEVRLRK

SEQ ID NO: 23 - DNA, 951 bp, Artificial Sequence
  Pantothenate Kinase from Escherichia coli variant
atgagcatcaaagagcagaccctgatgaccccgtacctgcagttcgaccgtaaccaatgggcggcgctgcgtgatagcgttccgatgaccctgagcgaggacgaaatcgcgcgtctgaagggtattaacgaggatctgagcctggaggaagtggcggaaatctacctgccgctgagccgtctgctgaacttctatattagcagcaacctgcgtcgtcaggcggttctggaacaatttctgggtaccaacggccagcgtatcccgtatatcattagcattgcgggtagcgtggcggttggcaaaagcaccaccgcgcgtgtgctgcaggcgctgctgagccgttggccggagcaccgtcgtgttgaactgatcaccaccgacggcttcctgcacccgaaccaagtgctgaaggagcgtggtctgatgaagaaaaagggtttcccggaaagctacgatatgcaccgtctggtgaaatttgttagcgacctgaagagcggtgtgccgaacgttaccgcgccggtgtacagccacctgatctatgatgttattccggacggcgataaaaccgtggttcagccggacatcctgattctggagggtctgaacgtgctgcaaagcggcatggactatccgcacgatccgcaccacgtgtttgttagcgacttcgtggattttagcatctacgttgacgcgccggaggatctgctgcagacctggtggattaaccgtttcctgaaatttcgtgagggtgcgttcaccgacccggatagctactttcacaactatgcgaaactgaccaaggaagaggcgatcaaaaccgcgatgaccctgtggaaggagatgaactggctgaacctgaagcaaaacattctgccgacccgtgaacgtgcgagcctgattctgaccaaaagcgcgaaccacgcggtggaggaagttcgtctgcgtaagtaa

SEQ ID NO: 24 - protein, 316 aa, Artificial Sequence
  Pantothenate Kinase from Escherichia coli variant
MSIKEQTLMTPYLQFDRNQWAALRDSVPMTLSEDEIARLKGINEDLSLEEVAEIYLPLSRLLNFYISSNLRRQAVLEQFLGTNGQRIPYIISIAGSVAVGKSTTARVLQALLSRWPEHRRVELITTDGFLHPNQVLKERGLMKKKGFPESYDMHRLVKFVSDLKSGVPNVTAPVYSHLIYDVIPDGDKTVVQPDILILEGLNVLQSGMDYPHDPHHVFVSDFVDFSIYVDAPEDLLQTWWINRFLKFREGAFTDPDSYFHNYAKLTKEEAIKTAMTLWKEMNWLNLKQNILPTRERASLILTKSANHAVEEVRLRK

SEQ ID NO: 25 - DNA, 951 bp, Artificial Sequence
  Pantothenate Kinase from Escherichia coli variant
atgagcatcaaagagcagaccctgatgaccccgtacctgcagttcgaccgtaaccaatgggcggcgctgcgtgatagcgttccgatgaccctgagcgaggacgaaatcgcgcgtctgaagggtattaacgaggatctgagcctggaggaagtggcggaaatctacctgccgctgagccgtctgctgaacttctatattagcagcaacctgcgtcgtcaggcggttctggaacaatttctgggtaccaacggccagcgtatcccgtatatcattagcattgcgggtagcgtggcggttggcaaaagcaccaccgcgcgtgtgctgcaggcgctgctgagccgttggccggagcaccgtcgtgttgaactgatcaccaccgacggcttcctgcacccgaaccaagtgctgaaggagcgtggtctgatgaagaaaaagggcttcccggaaagctacgatatgcaccgtctggtgaaatttgttagcgacctgaagagcggtgtgccgaacgttaccgcgccggtgtacagccacctgatctatgatgttattccggacggcgataaaaccgtggttcagccggacatcctgattctggagggtctgaacgtgctgcaaagcggcatggactatccgcacgatccgcaccacgtgtttgttagcgacttcgtggattttagcatctacgttgacgcgccggaggatctgctgcagacctggttcattaaccgtttcctgaaatttcgtgagggtgcgttcaccgacccggatagctactttcacaactatgcgaaactgaccaaggaagaggcgatcaaaaccgcgatgaccatgtggaaggagattaactggctgaacctgaagcaaaacattctgccgacccgtgaacgtgcgagcctgattctgaccaaaagcgcgaaccacgcggtggaggaagttcgtctgcgtaagtaa

SEQ ID NO: 26 - protein, 316 aa, Artificial Sequence
  Pantothenate Kinase from Escherichia coli variant
MSIKEQTLMTPYLQFDRNQWAALRDSVPMTLSEDEIARLKGINEDLSLEEVAEIYLPLSRLLNFYISSNLRRQAVLEQFLGTNGQRIPYIISIAGSVAVGKSTTARVLQALLSRWPEHRRVELITTDGFLHPNQVLKERGLMKKKGFPESYDMHRLVKFVSDLKSGVPNVTAPVYSHLIYDVIPDGDKTVVQPDILILEGLNVLQSGMDYPHDPHHVFVSDFVDFSIYVDAPEDLLQTWFINRFLKFREGAFTDPDSYFHNYAKLTKEEAIKTAMTMWKEINWLNLKQNILPTRERASLILTKSANHAVEEVRLRK

SEQ ID NO: 27 - DNA, 951 bp, Artificial Sequence
  Pantothenate Kinase from Escherichia coli variant
atgagcatcaaagagcagaccctgatgaccccgtacctgcagttcgaccgtaaccaatgggcggcgctgcgtgatagcgttccgatgaccctgagcgaggacgaaatcgcgcgtctgaagggtattaacgaggatctgagcctggaggaagtggcggaaatctacctgccgctgagccgtctgctgaacttctatattagcagcaacctgcgtcgtcaggcggttctggaacaatttctgggtaccaacggccagcgtatcccgtatatcattagcattgcgggtagcgtggcggttggcaaaagcaccaccgcgcgtgtgctgcaggcgctgctgagccgttggccggagcaccgtcgtgttgaactgatcaccaccgacggcttcctgcacccgaaccaagtgctgaaggagcgtggtctgatgaagaaaaagggtttcccggaaagctacgatatgcaccgtctggtgaaatttgttagcgacctgaagagcggtgtgccgaacgttaccgcgccggtgtacagccacctgatctatgatgttattccggacggcgataaaaccgtggttcagccggacatcctgattctggagggtctgaacgtgctgcaaagcggcatggactatccgcacgatccgcaccacgtgtttgttagcgacttcgtggattttagcatctacgttgacgcgccggaggatctgctgcagacctggttcattaaccgtttcctgaaatttcgtgagggtgcgttcaccgacccggatagctactttcacaactatgcgaaactgaccaaggaagaggcgatcaaaaccgcgatgaccatgtggaaggagattaactggctgaacctgaagcaaaacattctgccgacccgtgaacgtgcgagcctgattctgaccaaaagcgcgaaccacgcggtggaggaagttcgtctgcgtaagtaa

SEQ ID NO: 28 - protein, 316 aa, Artificial Sequence; identical to SEQ ID NO: 26
  Pantothenate Kinase from Escherichia coli variant

SEQ ID NO: 29 - DNA, 951 bp, Artificial Sequence
  Pantothenate Kinase from Escherichia coli variant
atgagcatcaaagagcagaccctgatgaccccgtacctgcagttcgaccgtaaccaatgggcggcgctgcgtgatagcgttccgatgaccctgagcgaggacgaaatcgcgcgtctgaagggtattaacgaggatctgagcctggaggaagtggcggaaatctacctgccgctgagccgtctgctgaacttctatattagcagcaacctgcgtcgtcaggcggttctggaacaatttctgggtaccaacggccagcgtatcccgtatatcattagcattgcgggtagcgtggcggttggcaaaagcaccaccgcgcgtgtgctgcaggcgctgctgagccgttggccggagcaccgtcgtgttgaactgatcaccaccgacggcttcctgcacccgaaccaagtgctgaaggagcgtggtctgatgaagaaaaagggtttcccggaaagctacgatatgcaccgtctggtgaaatttgttagcgacctgaagagcggtgtgccgaacgttaccgcgccggtgtacagccacctgatctatgatgttattccggacggcgataaaaccgtggttcagccggacatcctgattctggagggtctgaacgtgctgcaaagcggcatggactatccgcacgatccgcaccacgtgtttgttagcgacttcgtggattttagcatctacgttgacgcgccggaggatctgctgcagacctggtacattaaccgtttcctgaaatttcgtgagggtgcgttcaccgacccggatagctactttcacaactatgcgaaactgaccaaggaagaggcgatcaaaaccgcgatgaccatttggaaggagatgaactggctgaacctgaagcaaaacattctgccgacccgtgaacgtgcgagcctgattctgaccaaaagcgcgaaccacgcggtggaggaagttcgtctgcgtaagtaa

SEQ ID NO: 30 - protein, 316 aa, Artificial Sequence
  Pantothenate Kinase from Escherichia coli variant
MSIKEQTLMTPYLQFDRNQWAALRDSVPMTLSEDEIARLKGINEDLSLEEVAEIYLPLSRLLNFYISSNLRRQAVLEQFLGTNGQRIPYIISIAGSVAVGKSTTARVLQALLSRWPEHRRVELITTDGFLHPNQVLKERGLMKKKGFPESYDMHRLVKFVSDLKSGVPNVTAPVYSHLIYDVIPDGDKTVVQPDILILEGLNVLQSGMDYPHDPHHVFVSDFVDFSIYVDAPEDLLQTWYINRFLKFREGAFTDPDSYFHNYAKLTKEEAIKTAMTIWKEMNWLNLKQNILPTRERASLILTKSANHAVEEVRLRK

SEQ ID NO: 31 - DNA, 951 bp, Artificial Sequence; identical to SEQ ID NO: 21
  Pantothenate Kinase from Escherichia coli variant

SEQ ID NO: 32 - protein, 316 aa, Artificial Sequence; identical to SEQ ID NO: 22
  Pantothenate Kinase from Escherichia coli variant

SEQ ID NO: 33 - DNA, 951 bp, Artificial Sequence
  Pantothenate Kinase from Escherichia coli variant
atgagcatcaaagagcagaccctgatgaccccgtacctgcagttcgaccgtaaccaatgggcggcgctgcgtgatagcgttccgatgaccctgagcgaggacgaaatcgcgcgtctgaagggtattaacgaggatctgagcctggaggaagtggcggaaatctacctgccgctgagccgtctgctgaacttctatattagcagcaacctgcgtcgtcaggcggttctggaacaatttctgggtaccaacggccagcgtatcccgtatatcattagcattgcgggtagcgtggcggttggcaaaagcaccaccgcgcgtgtgctgcaggcgctgctgagccgttggccggagcaccgtcgtgttgaactgatcaccaccgacggcttcctgcacccgaaccaagtgctgaaggagcgtggtctgatgaagaaaaagggtttcccggaaagctacgatatgcaccgtctggtgaaatttgttagcgacctgaagagcggtgtgccgaacgttaccgcgccggtgtacagccacctgatctatgatgttattccggacggcgataaaaccgtggttcagccggacatcctgattctggagggtctgaacgtgctgcaaagcggcatggactatccgcacgatccgcaccacgtgtttgttagcgacttcgtggattttagcatctacgttgacgcgccggaggatctgctgcagacctggttcattaaccgtttcctgaaatttcgtgagggtgcgttcaccgacccggatagctactttcacaactatgcgaaactgaccaaggaagaggcgatcaaaaccgcgatgaccttgtggaaggagatgatgtggctgaacctgaagcaaaacattctgccgacccgtgaacgtgcgagcctgattctgaccaaaagcgcgaaccacgcggtggaggaagttcgtctgcgtaagtaa

SEQ ID NO: 34 - protein, 316 aa, Artificial Sequence
  Pantothenate Kinase from Escherichia coli variant
MSIKEQTLMTPYLQFDRNQWAALRDSVPMTLSEDEIARLKGINEDLSLEEVAEIYLPLSRLLNFYISSNLRRQAVLEQFLGTNGQRIPYIISIAGSVAVGKSTTARVLQALLSRWPEHRRVELITTDGFLHPNQVLKERGLMKKKGFPESYDMHRLVKFVSDLKSGVPNVTAPVYSHLIYDVIPDGDKTVVQPDILILEGLNVLQSGMDYPHDPHHVFVSDFVDFSIYVDAPEDLLQTWFINRFLKFREGAFTDPDSYFHNYAKLTKEEAIKTAMTLWKEMMWLNLKQNILPTRERASLILTKSANHAVEEVRLRK

SEQ ID NO: 35 - DNA, 951 bp, Artificial Sequence
  Pantothenate Kinase from Escherichia coli variant
atgagcatcaaagagcagaccctgatgaccccgtacctgcagttcgaccgtaaccaatgggcggcgctgcgtgatagcgttccgatgaccctgagcgaggacgaaatcgcgcgtctgaagggtattaacgaggatctgagcctggaggaagtggcggaaatctacctgccgctgagccgtctgctgaacttctatattagcagcaacctgcgtcgtcaggcggttctggaacaatttctgggtaccaacggccagcgtatcccgtatatcattagcattgcgggtagcgtggcggttggcaaaagcaccaccgcgcgtgtgctgcaggcgctgctgagccgttggccggagcaccgtcgtgttgaactgatcaccaccgacggcttcctgcacccgaaccaagtgctgaaggagcgtggtctgatgaagaaaaagggtttcccggaaagctacgatatgcaccgtctggtgaaatttgttagcgacctgaagagcggtgtgccgaacgttaccgcgccggtgtacagccacctgatctatgatgttattccggacggcgataaaaccgtggttcagccagacatcctgattctggagggtctgaacgtgctgcaaagcggcatggactatccgcacgatccgcaccacgtgtttgttagcgacttcgtggattttagcatctacgttgacgcgccggaggatctgctgcagacctggttcattaaccgtttcctgaaatttcgtgagggtgcgttcaccgacccggatagctactttcacaactatgcgaaactgaccaaggaagaggcgatcaaaaccgcgatgaccatttggaaggagttgaactggctgaacctgaagcaaaacattctgccgacccgtgaacgtgcgagcctgattctgaccaaaagcgcgaaccacgcggtggaggaagttcgtctgcgtaagtaa

SEQ ID NO: 36 - protein, 316 aa, Artificial Sequence
  Pantothenate Kinase from Escherichia coli variant
MSIKEQTLMTPYLQFDRNQWAALRDSVPMTLSEDEIARLKGINEDLSLEEVAEIYLPLSRLLNFYISSNLRRQAVLEQFLGTNGQRIPYIISIAGSVAVGKSTTARVLQALLSRWPEHRRVELITTDGFLHPNQVLKERGLMKKKGFPESYDMHRLVKFVSDLKSGVPNVTAPVYSHLIYDVIPDGDKTVVQPDILILEGLNVLQSGMDYPHDPHHVFVSDFVDFSIYVDAPEDLLQTWFINRFLKFREGAFTDPDSYFHNYAKLTKEEAIKTAMTIWKELNWLNLKQNILPTRERASLILTKSANHAVEEVRLRK

SEQ ID NO: 37 - DNA, 951 bp, Artificial Sequence
  Pantothenate Kinase from Escherichia coli variant
atgagcatcaaagagcagaccctgatgaccccgtacctgcagttcgaccgtaaccaatgggcggcgctgcgtgatagcgttccgatgaccctgagcgaggacgaaatcgcgcgtctgaagggtattaacgaggatctgagcctggaggaagtggcggaaatctacctgccgctgagccgtctgctgaacttctatattagcagcaacctgcgtcgtcaggcggttctggaacaatttctgggtaccaacggccagcgtatcccgtatatcattagcattgcgggtagcgtggcggttggcaaaagcaccaccgcgcgtgtgctgcaggcgctgctgagccgttggccggagcaccgtcgtgttgaactgatcaccaccgacggcttcctgcacccgaaccaagtgctgaaggagcgtggtctgatgaagaaaaagggtttcccggaaagctacgatatgcaccgtctggtgaaatttgttagcgacctgaagagcggtgtgccgaacgttaccgcgccggtgtacagccacctgatctatgatgttattccggacggcgataaaaccgtggttcagccggacatcctgattctggagggtctgaacgtgctgcaaagcggcatggactatccgcacgatccgcaccacgtgtttgttagcgacttcgtggattttagcatctacgttgacgcgccggaggatctgctgcagacctggtacattaaccgtttcctgaaatttcgtgagggtgcgttcaccgacccggatagctactttcacaactatgcgaaactgaccaaggaagaggcgatcaaaaccgcgatgaccatttggaaggagttgaactggctgaacctgaagcaaaacattctgccgacccgtgaacgtgcgagcctgattctgaccaaaagcgcgaaccacgcggtggaggaagttcgtctgcgtaagtaa

SEQ ID NO: 38 - protein, 316 aa, Artificial Sequence; identical to SEQ ID NO: 18
  Pantothenate Kinase from Escherichia coli variant

SEQ ID NO: 39 - DNA, 951 bp, Artificial Sequence
  Pantothenate Kinase from Escherichia coli variant
atgagcatcaaagagcagaccctgatgaccccgtacctgcagttcgaccgtaaccaatgggcggcgctgcgtgatagcgttccgatgaccctgagcgaggacgaaatcgcgcgtctgaagggtattaacgaggatctgagcctggaggaagtggcggaaatctacctgccgctgagccgtctgctgaacttctatattagcagcaacctgcgtcgtcaggcggttctggaacaatttctgggtaccaacggccagcgtatcccgtatatcattagcattgcgggtagcgtggcggttggcaaaagcaccaccgcgcgtgtgctgcaggcgctgctgagccgttggccggagcaccgtcgtgttgaactgatcaccaccgacggcttcctgcacccgaaccaagtgctgaaggagcgtggtctgatgaagaaaaagggtttcccggaaagctacgatatgcaccgtctggtgaaatttgttagcgacctgaagagcggtgtgccgaacgttaccgcgccggtgtacagccacctgatctatgatgttattccggacggcgataaaaccgtggttcagccggacatcctgattctggagggtctgaacgtgctgcaaagcggcatggactatccgcacgatccgcaccacgtgtttgttagcgacttcgtggattttagcatctacgttgacgcgccggaggatctgctgcagacctggttcattaaccgtttcctgaaatttcgtgagggtgcgttcaccgacccggatagctactttcacaactatgcgaaactgaccaaggaagaggcgatcaaaaccgcgatgaccttgtggaaggagattaactggctgaacctgaagcaaaacattctgccgacccgtgaacgtgcgagcctgattctgaccaaaagcgcgaaccacgcggtggaggaagttcgtctgcgtaagtaa

SEQ ID NO: 40 - protein, 316 aa, Artificial Sequence
  Pantothenate Kinase from Escherichia coli variant
MSIKEQTLMTPYLQFDRNQWAALRDSVPMTLSEDEIARLKGINEDLSLEEVAEIYLPLSRLLNFYISSNLRRQAVLEQFLGTNGQRIPYIISIAGSVAVGKSTTARVLQALLSRWPEHRRVELITTDGFLHPNQVLKERGLMKKKGFPESYDMHRLVKFVSDLKSGVPNVTAPVYSHLIYDVIPDGDKTVVQPDILILEGLNVLQSGMDYPHDPHHVFVSDFVDFSIYVDAPEDLLQTWFINRFLKFREGAFTDPDSYFHNYAKLTKEEAIKTAMTLWKEINWLNLKQNILPTRERASLILTKSANHAVEEVRLRK

SEQ ID NO: 41 - DNA, 951 bp, Artificial Sequence
  Pantothenate Kinase from Escherichia coli variant
atgagcatcaaagagcagaccctgatgaccccgtacctgcagttcgaccgtaaccaatgggcggcgctgcgtgatagcgttccgatgaccctgagcgaggacgaaatcgcgcgtctgaagggtattaacgaggatctgagcctggaggaagtggcggaaatctacctgccgctgagccgtctgctgaacttctatattagcagcaacctgcgtcgtcaggcggttctggaacaatttctgggtaccaacggccagcgtatcccgtatatcattagcattgcgggtagcgtggcggttggcaaaagcaccaccgcgcgtgtgctgcaggcgctgctgagccgttggccggagcaccgtcgtgttgaactgatcaccaccgacggcttcctgcacccgaaccaagtgctgaaggagcgtggtctgatgaagaaaaagggtttcccggaaagctacgatatgcaccgtctggtgaaatttgttagcgacctgaagagcggtgtgccgaacgttaccgcgccggtgtacagccacctgatctatgatgttattccggacggcgataaaaccgtggttcagccggacatcctgattctggagggtctgaacgtgctgcaaagcggcatggactatccgcacgatccgcaccacgtgtttgttagcgacttcgtggattttagcatctacgttgacgcgccggaggatctgctgcagacctggtacattaaccgtttcctgaaatttcgtgagggtgcgttcaccgacccggatagctactttcacaactatgcgaaactgaccaaggaagaggcgatcaaaaccgcgatgaccatgtggaaggagatgaactggctgaacctgaagcaaaacattctgccgacccgtgaacgtgcgagcctgattctgaccaaaagcgcgaaccacgcggtggaggaagttcgtctgcgtaagtaa

SEQ ID NO: 42 - protein, 316 aa, Artificial Sequence; identical to SEQ ID NO: 14
  Pantothenate Kinase from Escherichia coli variant

SEQ ID NO: 43 - DNA, 951 bp, Artificial Sequence
  Pantothenate Kinase from Escherichia coli variant
atgagcatcaaagagcagaccctgatgaccccgtacctgcagttcgaccgtaaccaatgggcggcgctgcgtgatagcgttccgatgaccctgagcgaggacgaaatcgcgcgtctgaagggtattaacgaggatctgagcctggaggaagtggcggaaatctacctgccgctgagccgtctgctgaacttctatattagcagcaacctgcgtcgtcaggcggttctggaacaatttctgggtaccaacggccagcgtatcccgtatatcattagcattgcgggtagcgtggcggttggcaaaagcaccaccgcgcgtgtgctgcaggcgctgctgagccgttggccggagcaccgtcgtgttgaactgatcaccaccgacggcttcctgcacccgaaccaagtgctgaaggagcgtggtctgatgaagaaaaagggtttcccggaaagctacgatatgcaccgtctggtgaaatttgttagcgacctgaagagcggtgtgccgaacgttaccgcgccggtgtacagccacctgatctatgatgttattccggacggcgataaaaccgtggttcagccggacatcctgattctggagggtctgaacgtgctgcaaagcggcatggactatccgcacgatccgcaccacgtgtttgttagcgacttcgtggattttagcatctacgttgacgcgccggaggatctgctgcagacctggttcattaaccgtttcctgaaatttcgtgagggtgcgttcaccgacccggatagctactttcacaactatgcgaaactgaccaaggaagaggcgatcaaaaccgcgatgaccctgtggaaggagatcaactggctgaacctgaagcaaaacattctgccgacccgtgaacgtgcgagcctgattctgaccaaaagcgcgaaccacgcggtggaggaagttcgtctgcgtaagtaa

SEQ ID NO: 44 - protein, 316 aa, Artificial Sequence; identical to SEQ ID NO: 40
  Pantothenate Kinase from Escherichia coli variant

SEQ ID NO: 45 - DNA, 948 bp, Artificial Sequence
  Pantothenate Kinase from Escherichia coli variant
atgagcatcaaagagcagaccctgatgaccccgtacgatgaattcgaccgtaacacttgggcgggcctgcgtgatagcgttccgatgaccctgagcgaggacgaaatcgcacgtctgaagggtattaacgaggatctgagcctggaggaagtggcggaaatctacctgccgctgagccgtctgctgaacttctatattagcagcaacctgcgtcgtcaggcggttctggaacaatttctgggtaccaacggccagcgtatcccgtatatcattagcattgcgggtagcgtggcggttggcaaaagcaccaccgcgcgtgtgctgcaggcgctgctgagccgttggccggagcaccgtcgtgttgaactgatcaccaccgacggcttcctgcacccgaaccaagtgctgaaggagcgtggtctgatgaagaaaaagggtttcccggaaagctacgatatgcaccgtctggtgaaatttgttagcgacctgaagagcggtgtgccgaacgttaccgcgccggtgtacagccacctgatctatgatgttattccggacggcgataaaaccgtggttcagccggacatcctgattctggagggtctgaacgtgctgcaaagcggcatggactatccgcacgatccgcaccacgtgttcgttagcgacttcgtggattttagcatctacgttgacgcgccggaggatctgctgcagacctggtacattaaccgtttcctgaaatttcgtgagggtgcgttcaccgacccggatagctactttcacaactatgcgaaactgaccaaggaagaggcgatcaaaaccgcgatgaccatttggaaggagatgaactggctgaacctgaagcaaaacattctgccgacccgtgaacgtgcgagcctgattctgaccaaaagcgcgaaccacgcggtggaggaagttcgtctgcgtaag

SEQ ID NO: 46 - protein, 316 aa, Artificial Sequence
  Pantothenate Kinase from Escherichia coli variant
MSIKEQTLMTPYDEFDRNTWAGLRDSVPMTLSEDEIARLKGINEDLSLEEVAEIYLPLSRLLNFYISSNLRRQAVLEQFLGTNGQRIPYIISIAGSVAVGKSTTARVLQALLSRWPEHRRVELITTDGFLHPNQVLKERGLMKKKGFPESYDMHRLVKFVSDLKSGVPNVTAPVYSHLIYDVIPDGDKTVVQPDILILEGLNVLQSGMDYPHDPHHVFVSDFVDFSIYVDAPEDLLQTWYINRFLKFREGAFTDPDSYFHNYAKLTKEEAIKTAMTIWKEMNWLNLKQNILPTRERASLILTKSANHAVEEVRLRK

SEQ ID NO: 47 - DNA, 948 bp, Artificial Sequence
  Pantothenate Kinase from Escherichia coli variant
atgagcatcaaagagcagaccctgatgaccccgtacgatgaattcgaccgtaaccaatgggcgggcctgcgtgatagcgttccgatgaccctgagcgaggacgaaatcgcgcgtctgaagggtattaacgaggatctgagcctggaggaagtggcggaaatctacctgccgctgagccgtctgctgaacttctatattagcagcaacctgcgtcgtcaggcggttctggaacaatttctgggtaccaacggccagcgtatcccgtatatcattagcattgcgggtagcgtggcggttggcaaaagcaccaccgcgcgtgtgctgcaggcgctgctgagccgttggccggagcaccgtcgtgttgaactgatcaccaccgacggcttcctgcacccgaaccaagtgctgaaggagcgtggtctgatgaagaaaaagggtttcccggaaagctacgatatgcaccgtctggtgaaatttgttagcgacctgaagagcggtgtgccgaacgttaccgcgccggtgtacagccacctgatctatgatgttattccggacggcgataaaaccgtggttcagccggacatcctgattctggagggtctgaacgtgctgcaaagcggcatggactatccgcacgatccgcaccacgtgtttgttagcgacttcgtggattttagcatctacgttgacgcgccggaggatctgctgcagacctggtacattaaccgtttcctgaaatttcgtgagggtgcgttcaccgacccggatagctactttcacaactatgcgaaactgaccaaggaagaggcgatcaaaaccgcgatgaccatttggaaggagatgaactggctgaacctgaagcaaaacattctgccgacccgtgaacgtgcgagcctgattctgaccaaaagcgcgaaccacgcggtggaggaagttcgtctgcgtaag

SEQ ID NO: 48 - protein, 316 aa, Artificial Sequence
  Pantothenate Kinase from Escherichia coli variant
MSIKEQTLMTPYDEFDRNQWAGLRDSVPMTLSEDEIARLKGINEDLSLEEVAEIYLPLSRLLNFYISSNLRRQAVLEQFLGTNGQRIPYIISIAGSVAVGKSTTARVLQALLSRWPEHRRVELITTDGFLHPNQVLKERGLMKKKGFPESYDMHRLVKFVSDLKSGVPNVTAPVYSHLIYDVIPDGDKTVVQPDILILEGLNVLQSGMDYPHDPHHVFVSDFVDFSIYVDAPEDLLQTWYINRFLKFREGAFTDPDSYFHNYAKLTKEEAIKTAMTIWKEMNWLNLKQNILPTRERASLILTKSANHAVEEVRLRK

SEQ ID NO: 49 - DNA, 948 bp, Artificial Sequence
  Pantothenate Kinase from Escherichia coli variant
atgagcatcaaagagcagaccctgatgaccccgtacctgcaattcgaccgtaaccaatgggcgggcctgcgtgatagcgttccgatgaccctgagcgaggacgaaatcgcgcgtctgaagggtattaacgaggatctgagcctggaggaagtggcggaaatctacctgccgctgagccgtctgctgaacttctatattagcagcaacctgcgtcgtcaggcggttctggaacaatttctgggtaccaacggccagcgtatcccgtatatcattagcattgcgggtagcgtggcggttggcaaaagcaccaccgcgcgtgtgctgcaggcgctgctgagccgttggccggagcaccgtcgtgttgaactgatcaccaccgacggcttcctgcacccgaaccaagtgctgaaggagcgtggtctgatgaagaaaaagggtttcccggaaagctacgatatgcaccgtctggtgaaatttgttagcgacctgaagagcggtgtgccgaacgttaccgcgccggtgtacagccacctgatctatgatgttattccggacggcgataaaaccgtggttcagccggacatcctgattctggagggtctgaacgtgctgcaaagcggcatggactatccgcacgatccgcaccacgtggaggttagcgacttcgtggattttagcatctacgttgacgcgccggaggatctgctgcagacctggtacattaaccgtttcctgaaatttcgtgagggtgcgttcaccgacccggatagctactttcacaactatgcgaaactgaccaaggaagaggcgatcaaaaccgcgatgaccatctggaaggagatgaactggctgaacctgaagcaaaacattctgccgacccgtgaacgtgcgagcctgattctgaccaaaagcgcgaaccacgcggtggaggaagttcgtctgcgtaag

SEQ ID NO: 50 - protein, 316 aa, Artificial Sequence
  Pantothenate Kinase from Escherichia coli variant
MSIKEQTLMTPYLQFDRNQWAGLRDSVPMTLSEDEIARLKGINEDLSLEEVAEIYLPLSRLLNFYISSNLRRQAVLEQFLGTNGQRIPYIISIAGSVAVGKSTTARVLQALLSRWPEHRRVELITTDGFLHPNQVLKERGLMKKKGFPESYDMHRLVKFVSDLKSGVPNVTAPVYSHLIYDVIPDGDKTVVQPDILILEGLNVLQSGMDYPHDPHHVEVSDFVDFSIYVDAPEDLLQTWYINRFLKFREGAFTDPDSYFHNYAKLTKEEAIKTAMTIWKEMNWLNLKQNILPTRERASLILTKSANHAVEEVRLRK

SEQ ID NO: 51 - DNA, 948 bp, Artificial Sequence
  Pantothenate Kinase from Escherichia coli variant
atgagcatcaaagagcagaccctgatgaccccgtacctgcagtttgaccgtaaccaatgggcggcgctgcgtgatagtaacccgatgaccctgagcgaggacgaaatcgcgcgtctgaagggtattaacgaggatctgagcctggaggaagtggcggaaatctacctgccgctgagccgtctgctgaacttctatattagcagcaacctgcgtcgtcaggcggttctggaacaatttctgggtaccaacggccagcgtatcccgtatatcattagcattgcgggtagcgtggcggttggcaaaagcaccaccgcgcgtgtgctgcaggcgctgctgagccgttggccggagcaccgtcgtgttgaactgatcaccaccgacggcttcctgcacccgaaccaagtgctgaaggagcgtggtctgatgaagaaaaagggtttcccggaaagctacgatatgcaccgtctggtgaaatttgttagcgacctgaagagcggtgtgccgaacgttaccgcgccggtgtacagccacctgatctatgatgttattccggacggcgataaaaccgtggttcagccggacatcctgattctggagggtctgaacgtgctgcaaagcggcatggactatccgcacgatccgcaccacgtgtttgttagcgacttcgtggattttagcatctacgttgacgcgccggaggatctgctgcagacctggtacattaaccgtttcctgaaatttcgtgagggtgcgttcaccgacccggatagctactttcacaactatgcgaaactgaccaaggaagaggcgatcaaaaccgcgatgaccatttggaaggagatgaaccacctgaacctgaagcaaaacattctgccgacccgtgaacgtgcgagcctgattctgaccaaaagcgcgaaccacgcggtggaggaagttcgtctgcgtaag

SEQ ID NO: 52 - protein, 316 aa, Artificial Sequence
  Pantothenate Kinase from Escherichia coli variant
MSIKEQTLMTPYLQFDRNQWAALRDSNPMTLSEDEIARLKGINEDLSLEEVAEIYLPLSRLLNFYISSNLRRQAVLEQFLGTNGQRIPYIISIAGSVAVGKSTTARVLQALLSRWPEHRRVELITTDGFLHPNQVLKERGLMKKKGFPESYDMHRLVKFVSDLKSGVPNVTAPVYSHLIYDVIPDGDKTVVQPDILILEGLNVLQSGMDYPHDPHHVFVSDFVDFSIYVDAPEDLLQTWYINRFLKFREGAFTDPDSYFHNYAKLTKEEAIKTAMTIWKEMNHLNLKQNILPTRERASLILTKSANHAVEEVRLRK

SEQ ID NO: 53 - DNA, 948 bp, Artificial Sequence
  Pantothenate Kinase from Escherichia coli variant
atgagcatcaaagagcagaccctgatgaccccgtacgatgaattcgaccgtaaccaatgggcgggcctgcgtgatagcgttccgatgaccctgagcgaggacgaaatcctgcgtctgaagggtattaacgaggatctgagcctggaggaagtggcggaaatctacctgccgctgagccgtctgctgaacttctatattagcagcaacctgcgtcgtcaggcggttctggaacaatttctgggtaccaacggccagcgtatcccgtatatcattagcattgcgggtagcgtggcggttggcaaaagcaccaccgcgcgtgtgctgcaggcgctgctgagccgttggccggagcaccgtcgtgttgaactgatcaccaccgacggcttcctgcacccgaaccaagtgctgaaggagcgtggtctgatgaagaaaaagggtttcccggaaagctacgatatgcaccgtctggtgaaatttgttagcgacctgaagagcggtgtgccgaacgttaccgcgccggtgtacagccacctgatctatgatgttattccggacggcgataaaaccgtggttcagccggacatcctgattctggagggtctgaacgtgctgcaaagcggcatggactatccgcacgatccgcaccacgtgtttgttagcgacttcgtggattttagcatctacgttgacgcgccggaggatctgctgcagacctggtacattaaccgtttcctgaaatttcgtgagggtgcgttcaccgacccggatagctactttcacaactatgcgaaactgaccaaggaagaggcgatcaaaaccgcgatgaccatttggaaggagatgaactggctgaacctgaagcaaaacattctgccgacccgtgaacgtgcgagcctgattctgaccaaaagcgcgaaccacgcggtggaggaagttcgtctgcgtaag

SEQ ID NO: 54 - protein, 316 aa, Artificial Sequence
  Pantothenate Kinase from Escherichia coli variant
MSIKEQTLMTPYDEFDRNQWAGLRDSVPMTLSEDEILRLKGINEDLSLEEVAEIYLPLSRLLNFYISSNLRRQAVLEQFLGTNGQRIPYIISIAGSVAVGKSTTARVLQALLSRWPEHRRVELITTDGFLHPNQVLKERGLMKKKGFPESYDMHRLVKFVSDLKSGVPNVTAPVYSHLIYDVIPDGDKTVVQPDILILEGLNVLQSGMDYPHDPHHVFVSDFVDFSIYVDAPEDLLQTWYINRFLKFREGAFTDPDSYFHNYAKLTKEEAIKTAMTIWKEMNWLNLKQNILPTRERASLILTKSANHAVEEVRLRK

SEQ ID NO: 55 - DNA, 948 bp, Artificial Sequence
  Pantothenate Kinase from Escherichia coli variant
atgagcatcaaagagcagaccctgatgaccccgtacctgcagttcgaccgtaaccaaatggcggcgctgcgcgatagcgttccgatgacgctgagcgaggacgaaatcgcgcgtctgaagggtattaacgaggatctgagcctggaggaagtggcggaaatctacctgccgctgagccgtctgctgaacttctatattagcagcaacctgcgtcgtcaggcggttctggaacaatttctgggtaccaacggccagcgtatcccgtatatcattagcattgcgggtagcgtggcggttggcaaaagcaccaccgcgcgtgtgctgcaggcgctgctgagccgttggccggagcaccgtcgtgttgaactgatcaccaccgacggcttcctgcacccgaaccaagtgctgaaggagcgtggtctgatgaagaaaaagggtttcccggaaagctacgatatgcaccgtctggtgaaatttgttagcgacctgaagagcggtgtgccgaacgttaccgcgccggtgtacagccacctgatctatgatgttattccggacggcgataaaaccgtggttcagccggacatcctgattctggagggtctgaacgtgctgcaaagcggcatggactatccgcacgatccgcaccacgtgtttgttagcgacttcgtggattttagcatctacgttgacgcgccggaggatctgctgcagacctggtacattaaccgtttcctgaaatttcgtgagggtgcgttcaccgacccggatagctactttcacaactatgcgaaactgaccaaggaagaggcgatcaaaaccgcgatgaccatttggaaggagatgaactggctgaacctgaagcaaaacattctgccgacccgtgaacgtgcgagcctgattctgaccaaaagcgcgaaccacgcggtggaggaagttcgtctgcgtaag

SEQ ID NO: 56 - protein, 316 aa, Artificial Sequence
  Pantothenate Kinase from Escherichia coli variant
MSIKEQTLMTPYLQFDRNQMAALRDSVPMTLSEDEIARLKGINEDLSLEEVAEIYLPLSRLLNFYISSNLRRQAVLEQFLGTNGQRIPYIISIAGSVAVGKSTTARVLQALLSRWPEHRRVELITTDGFLHPNQVLKERGLMKKKGFPESYDMHRLVKFVSDLKSGVPNVTAPVYSHLIYDVIPDGDKTVVQPDILILEGLNVLQSGMDYPHDPHHVFVSDFVDFSIYVDAPEDLLQTWYINRFLKFREGAFTDPDSYFHNYAKLTKEEAIKTAMTIWKEMNWLNLKQNILPTRERASLILTKSANHAVEEVRLRK

SEQ ID NO: 57 - DNA, 948 bp, Artificial Sequence
  Pantothenate Kinase from Escherichia coli variant
atgagcatcaaagagcagaccctgatgaccccgtacctgcagttcgaccgtaaccaatgggcggctctgcgtgatccggttccgatgaccctgagcgaggacgaaatcgcgcgtctgaagggtattaacgaggatctgagcctggaggaagtggcggaaatctacctgccgctgagccgtctgctgaacttctatattagcagcaacctgcgtcgtcaggcggttctggaacaatttctgggtaccaacggccagcgtatcccgtatatcattagcattgcgggtagcgtggcggttggcaaaagcaccaccgcgcgtgtgctgcaggcgctgctgagccgttggccggagcaccgtcgtgttgaactgatcaccaccgacggcttcctgcacccgaaccaagtgctgaaggagcgtggtctgatgaagaaaaagggtttcccggaaagctacgatatgcaccgtctggtgaaatttgttagcgacctgaagagcggtgtgccgaacgttaccgcgccggtgtacagccacctgatctatgatgttattccggacggcgataaaaccgtggttcagccggacatcctgattctggagggtctgaacgtgctgcaaagcggcatggactatccgcacgatccgcaccacgtgtttgttagcgacttcgtggattttagcatctacgttgacgcgccggaggatctgctgcagacctggtacattaaccgtttcctgaaatttcgtgagggtgcgttcaccgacccggatagctactttcacaactatgcgaaactgaccaaggaagaggcgatcaaaaccgcgatgaccatttggaaggagatgaactggctgaacctgaagcaaaacattctgccgacccgtgaacgtgcgagcctgattctgaccaaaagcgcgaaccacgcggtggaggaagttcgtctgcgtaag

SEQ ID NO: 58 - protein, 316 aa, Artificial Sequence
  Pantothenate Kinase from Escherichia coli variant
MSIKEQTLMTPYLQFDRNQWAALRDPVPMTLSEDEIARLKGINEDLSLEEVAEIYLPLSRLLNFYISSNLRRQAVLEQFLGTNGQRIPYIISIAGSVAVGKSTTARVLQALLSRWPEHRRVELITTDGFLHPNQVLKERGLMKKKGFPESYDMHRLVKFVSDLKSGVPNVTAPVYSHLIYDVIPDGDKTVVQPDILILEGLNVLQSGMDYPHDPHHVFVSDFVDFSIYVDAPEDLLQTWYINRFLKFREGAFTDPDSYFHNYAKLTKEEAIKTAMTIWKEMNWLNLKQNILPTRERASLILTKSANHAVEEVRLRK

SEQ ID NO: 59 - DNA, 948 bp, Artificial Sequence
  Pantothenate Kinase from Escherichia coli variant
atgagcatcaaagagcagaccctgatgaccccgtacctgcagctggaccgtaaccaatgggcggcgctgcgtgatagtaacccgatgaccctgagcgaggacgaaatcgcgcgtctgaagggtattaacgaggatctgagcctggaggaagtggcggaaatctacctgccgctgagccgtctgctgaacttctatattagcagcaacctgcgtcgtcaggcggttctggaacagtttctgggtaccaacggccagcgtatcccgtatatcattagcattgcgggtagcgtggcggttggcaaaagcaccaccgcgcgtgtgctgcaggcgctgctgagccgttggccggagcaccgtcgtgttgaactgatcaccaccgacggcttcctgcacccgaaccaagtgctgaaggagcgtggtctgatgaagaaaaagggtttcccggaaagctacgatatgcaccgtctggtgaaatttgttagcgacctgaagagcggtgtgccgaacgttaccgcgccggtgtacagccacctgatctatgatgttattccggacggcgataaaaccgtggttcagccggacatcctgattctggagggtctgaacgtgctgcaaagcggcatggactatccgcacgatccgcaccacgtgtttgttagcgacttcgtggattttagcatctacgttgacgcgccggaggatctgctgcagacctggtacattaaccgtttcctgaaatttcgtgagggtgcgttcaccgacccggatagctactttcacaactatgcgaaactgaccaaggaagaggcgatcaaaaccgcgatgaccatttggaaggagatgaaccacctgaacctgaagcaaaacattctgccgacccgtgaacgtgcgagcctgattctgaccaaaagcgcaaaccacgcggtggaggaagttcgtctgcgtaag

SEQ ID NO: 60 - protein, 316 aa, Artificial Sequence
  Pantothenate Kinase from Escherichia coli variant
MSIKEQTLMTPYLQLDRNQWAALRDSNPMTLSEDEIARLKGINEDLSLEEVAEIYLPLSRLLNFYISSNLRRQAVLEQFLGTNGQRIPYIISIAGSVAVGKSTTARVLQALLSRWPEHRRVELITTDGFLHPNQVLKERGLMKKKGFPESYDMHRLVKFVSDLKSGVPNVTAPVYSHLIYDVIPDGDKTVVQPDILILEGLNVLQSGMDYPHDPHHVFVSDFVDFSIYVDAPEDLLQTWYINRFLKFREGAFTDPDSYFHNYAKLTKEEAIKTAMTIWKEMNHLNLKQNILPTRERASLILTKSANHAVEEVRLRK

SEQ ID NO: 61 - DNA, 948 bp, Artificial Sequence
  Pantothenate Kinase from Escherichia coli variant
atgagcatcaaagagcagaccctgatgaccccgtacctgcagtttgaccgtaaccaatgggcggcgctgcgtgatagtaacccgatgaccctgagcgaggacgaaatcgcgcgtctgaagggtattaacgaggatctgagcctggaggaagtggcggaaatctacctgccgctgagccgtctgctgaacttctatattagcagcaacctgcgtcgtcaggcggttctggaagcgtttctgggtaccaacggccagcgtatcccgtatatcattagcattgcgggtagcgtggcggttggcaaaagcaccaccgcgcgtgtgctgcaggcgctgctgagccgttggccggagcaccgtcgtgttgaatggatcaccaccgacggcttcctgcacccgaaccaagtgctgaaggagcgtggtctgatgaagaaaaagggtttcccggaaagctacgatatgcaccgtctggtgaaatttgttagcgacctgaagagcggtgtgccgaacgttaccgcgccggtgtacagccacctgatctatgatgttattccggacggcgataaaaccgtggttcagccggacatcctgattctggagggtctgaacgtgctgcaaagcggcatggactatccgcacgatccgcaccacgtgtttgttagcgacttcgtggattttagcatctacgttgacgcgccggaggatctgctgcagacctggtacattaaccgtttcctgaaatttcgtgagggtgcgttcaccgacccggatagctactttcacaactatgcgaaactgaccaaggaagaggcgatcaaaaccgcgatgaccatttggaaggagatgaaccacctgaacctgaagcaaaacattctgccgacccgtgaacgtgcgagcctgattctgaccaaaagcgcgaaccacgcggtggaggaagttcgtctgcgtaag

SEQ ID NO: 62 - protein, 316 aa, Artificial Sequence
  Pantothenate Kinase from Escherichia coli variant
MSIKEQTLMTPYLQFDRNQWAALRDSNPMTLSEDEIARLKGINEDLSLEEVAEIYLPLSRLLNFYISSNLRRQAVLEAFLGTNGQRIPYIISIAGSVAVGKSTTARVLQALLSRWPEHRRVEWITTDGFLHPNQVLKERGLMKKKGFPESYDMHRLVKFVSDLKSGVPNVTAPVYSHLIYDVIPDGDKTVVQPDILILEGLNVLQSGMDYPHDPHHVFVSDFVDFSIYVDAPEDLLQTWYINRFLKFREGAFTDPDSYFHNYAKLTKEEAIKTAMTIWKEMNHLNLKQNILPTRERASLILTKSANHAVEEVRLRK

SEQ ID NO: 63 - DNA, 948 bp, Artificial Sequence
  Pantothenate Kinase from Escherichia coli variant
atgagcatcaaagagcagaccctgatgaccccgtacctgcagttcgaccgtaaccaaatggcggcgctggcggatagcgttccgatgcgcctgagcgaggacgaaatcgcgcgtctgaagggtattaacgaggatctgagcctggaggaagtggcggaaatctacctgccgctgagccgtctgctgaacttctatattagcagcaacctgcgtcgtcaggcggaactggaacaatttctgggtaccaacggccagcgtatcccgtatatcattagcattgcgggtagcgtggcggttggcaaaagcaccaccgcgcgtgtgctgcaggcgctgctgagccgttggccggagcaccgtcgtgttgaactgatcaccaccgacggcttcctgcacccgaaccaagtgctgaaggagcgtggtctgatgaagaaaaagggtttcccggaaagctacgatatgcaccgtctggtgaaatttgttagcgacctgaagagcggtgtgccgaacgttaccgcgccggtgtacagccacctgatctatgatgttattccggacggcgataaaaccgtggttcagccggacatcctgattctggagggtctgaacgtgctgcaaagcggcatggactatccgcacgatccgcaccacgtgtttgttagcgacttcgtggattttagcatctacgttgacgcgccggaggatctgctgcagacctggtacattaaccgtttcctgaaatttcgtgagggtgcgttcaccgacccggatagctactttcacaactatgcgaaactgaccaaggaagaggcgatcaaaaccgcgatgaccatttggaaggagatgaactggctgaacctgaagcaaaacattctgccgacccgtgaacgtgcgagcctgattctgaccaaaagcgcgaaccacgcggtggaggaagttcgtctgcgtaag

SEQ ID NO: 64 - protein, 316 aa, Artificial Sequence
  Pantothenate Kinase from Escherichia coli variant
MSIKEQTLMTPYLQFDRNQMAALADSVPMRLSEDEIARLKGINEDLSLEEVAEIYLPLSRLLNFYISSNLRRQAELEQFLGTNGQRIPYIISIAGSVAVGKSTTARVLQALLSRWPEHRRVELITTDGFLHPNQVLKERGLMKKKGFPESYDMHRLVKFVSDLKSGVPNVTAPVYSHLIYDVIPDGDKTVVQPDILILEGLNVLQSGMDYPHDPHHVFVSDFVDFSIYVDAPEDLLQTWYINRFLKFREGAFTDPDSYFHNYAKLTKEEAIKTAMTIWKEMNWLNLKQNILPTRERASLILTKSANHAVEEVRLRK

SEQ ID NO: 65 - DNA, 948 bp, Artificial Sequence
  Pantothenate Kinase from Escherichia coli variant
atgagcatcaaagagcagaccctgatgaccccgtacctgcagttcgaccgtaaccaaatggcggcgctgcgcgatagcgttccgatgacgctgagcgaggacgaaatcgcgcgtctgaagggtattaacgaggatctgagcctggaggaagtggcggaaatctacctgccgctgagccgtctgctgaacttctatattagcagcaacgatcgtcgtcaggcggaactggaacaatttctgggtaccaacggccagcgtatcccgtatatcattagcattgcgggtagcgtggcggttggcaaaagcaccaccgcgcgtgtgctgcaggcgctgctgagccgttggccggagcaccgtcgtgttgaactgatcaccaccgacggcttcctgcacccgaaccaagtgctgaaggagcgtggtctgatgaagaaaaagggtttcccggaaagctacgatatgcaccgtctggtgaaatttgttagcgacctgaagagcggtgtgccgaacgttaccgcgccggtgtacagccacctgatctatgatgttattccggacggcgataaaaccgtggttcagccggacatcctgatcctggagggtctgaacgtgctgcaaagcggcatggactatccgcacgatccgcaccacgtgtttgttagcgacttcgtggattttagcatctacgttgacgcgccggaggatctgctgcagacctggtacattaaccgtttcctgaaatttcgtgagggtgcgttcaccgacccggatagctactttcacaactatgcgaaactgaccaaggaagaggcgatcaaaaccgcgatgaccatttggaaggagatgaactggctgaacctgaagcaaaacattctgccgacccgtgaacgtgcgagcctgattctgaccaaaagcgcgaaccacgcggtggaggaagttcgtctgcgtaag

SEQ ID NO: 66 - protein, 316 aa, Artificial Sequence
  Pantothenate Kinase from Escherichia coli variant
MSIKEQTLMTPYLQFDRNQMAALRDSVPMTLSEDEIARLKGINEDLSLEEVAEIYLPLSRLLNFYISSNDRRQAELEQFLGTNGQRIPYIISIAGSVAVGKSTTARVLQALLSRWPEHRRVELITTDGFLHPNQVLKERGLMKKKGFPESYDMHRLVKFVSDLKSGVPNVTAPVYSHLIYDVIPDGDKTVVQPDILILEGLNVLQSGMDYPHDPHHVFVSDFVDFSIYVDAPEDLLQTWYINRFLKFREGAFTDPDSYFHNYAKLTKEEAIKTAMTIWKEMNWLNLKQNILPTRERASLILTKSANHAVEEVRLRK

SEQ ID NO: 67 - DNA, 948 bp, Artificial Sequence
  Pantothenate Kinase from Escherichia coli variant
atgagcatcaaagagcagaccctgatgaccccgtacgatcaattcgaccgtaacacttgggcggccctgcgtgatagcgttccgatgaccctgagcgaggacgaaatcgcgcgtctgaagggtattaacgaggatctgagcctggaggaagtggcggaaatctacctgccgctgagccgtctgctgaacttctatattagcagcaacctgcgtcgtcaggcggttctggaacaatttctgggtaccaacggccagcgtatcccgtatatcattagcattgcgggtagcgtggcggttggcaaaagcaccaccgcgcgtgtgctgcaggcgctgctgagccgttggccggagcaccgtcgtgttgaactgatcaccaccgacggcttcctgcacccgaaccaagtgctgaaggagcgtggtctgatgaagaaaaagggtttcccggaaagctacgatatgcaccgtctggtgaaatttgttagcgacctgaagagcggtgtgccgaacgttaccgcgccggtgtacagccacctgatctatgatgttattccggacggcgataaaaccgtggttcagccggacatcctgattctggagggtctgaacgtgctgcaaagcggcatggactatccgcacgatccgcaccacgtgtttgttagcgacttcgtggattttagcatctacgttgacgcgccggaggatctgctgcagacctggtacattaaccgtttcctgaaatttcgtgagggtgcgttcaccgacccggatagctactttcacaactatgcgaaactgaccaaggaagaggcgatcaaaaccgcgatgaccatctggaaggagatgaactggctgaacctgaagcaaaacattctgccgacccgtgaacgtgcgagcctgattctgaccaaaagcgcgaaccacgcggtggaggaagttcgtctgcgtaag

SEQ ID NO: 68 - protein, 316 aa, Artificial Sequence
  Pantothenate Kinase from Escherichia coli variant
MSIKEQTLMTPYDQFDRNTWAALRDSVPMTLSEDEIARLKGINEDLSLEEVAEIYLPLSRLLNFYISSNLRRQAVLEQFLGTNGQRIPYIISIAGSVAVGKSTTARVLQALLSRWPEHRRVELITTDGFLHPNQVLKERGLMKKKGFPESYDMHRLVKFVSDLKSGVPNVTAPVYSHLIYDVIPDGDKTVVQPDILILEGLNVLQSGMDYPHDPHHVFVSDFVDFSIYVDAPEDLLQTWYINRFLKFREGAFTDPDSYFHNYAKLTKEEAIKTAMTIWKEMNWLNLKQNILPTRERASLILTKSANHAVEEVRLRK

SEQ ID NO: 69 - DNA, 948 bp, Artificial Sequence
  Pantothenate Kinase from Escherichia coli variant
atgagcatcaaagagcagaccctgatgaccccgtacctgcagtttgaccgtaaccaatgggcggcgctgcgtgatagtaacccgatgaccctgagcgaggacgaaatcgcgcgtctgaagggtattaacgaggatctgagcctggaggaagtggcggaaatctacctgccgctgagccgtctgctgaacttctatattagcagcaacctgcgtcgtcaggcggttctggaacagtttctgggtaccaacggccagcgtatcccgtatatcattagcattgcgggtagcgtggcggttggcaaaagcaccaccgcgcgtgtgctgcaggcgctgctgagccgttggcctgagcaccgtcgtgttgaactgatcaccaccgacggcttcctgcacccgaaccaagtgctgaaggagcgtggtctgatgaagaaaaagggtttcccggaaagctacgatatgcaccgtctggtgaaatttgttagcgacctgaagagcggtgtgccgaacgttaccgcgccggtgtacagccacctgatctatgatgttattccggacggcgataaaaccgtggttcagccggacatcctgattctggagggtctgaacgtgctgcaaagcggcatggactatccgcacgatccgcaccacgtgtttgttagcgacttcgtggattttagcatctacgttgacgcgccggaggatctgctgcagacctggtacattaaccgtttcctgaaatttcgtgagggtgcgttcaccgacccggatagctactttcacaactatgcgaaactgaccaaggaagaggcgatcaaaaccgcgatgaccatttggaaggagatgaactggctgaacctgaagcaaaacattctgccgacccgtgaacgtgcgagcctgattctgaccaaaagcgcaaaccacgcggtggaggaagttcgtctgcgtaag

SEQ ID NO: 70 - protein, 316 aa, Artificial Sequence
  Pantothenate Kinase from Escherichia coli variant
MSIKEQTLMTPYLQFDRNQWAALRDSNPMTLSEDEIARLKGINEDLSLEEVAEIYLPLSRLLNFYISSNLRRQAVLEQFLGTNGQRIPYIISIAGSVAVGKSTTARVLQALLSRWPEHRRVELITTDGFLHPNQVLKERGLMKKKGFPESYDMHRLVKFVSDLKSGVPNVTAPVYSHLIYDVIPDGDKTVVQPDILILEGLNVLQSGMDYPHDPHHVFVSDFVDFSIYVDAPEDLLQTWYINRFLKFREGAFTDPDSYFHNYAKLTKEEAIKTAMTIWKEMNWLNLKQNILPTRERASLILTKSANHAVEEVRLRK

SEQ ID NO: 71 - DNA, 948 bp, Artificial Sequence
  Pantothenate Kinase from Escherichia coli variant
atgagcatcaaagagcagaccctgatgaccccgtacctgcagctggaccgtaaccaatgggcggcgctgcgtgatagtaacccgatgaccctgagcgaggacgaaatcgcgcgtctgaagggtattaacgaggatctgagcctggaggaagtggcggaaatctacctgccgctgagccgtctgctgaacttctatattagcagcaacctgcgtcgtcaggcggttctggaacagtttctgggtaccaacggccagcgtatcccgtatatcattagcattgcgggtagcgtggcggttggcaaaagcaccaccgcgcgtgtgctgcaggcgctgctgagccgttggccggagcaccgtcgtgttgaactgatcaccaccgacggcttcctgcacccgaaccaagtgctgaaggagcgtggtctgatgaagaaaaagggtttcccggaaagctacgatatgcaccgtctggtgaaatttgttagcgacctgaagagcggtgtgccgaacgttaccgcgccggtgtacagccacctgatctatgatgttattccggacggcgataaaaccgtggttcagccggacatcctgattctggagggtctgaacgtgctgcaaagcggcatggactatccgcacgatccgcaccacgtgtttgttagcgacttcgtggattttagcatctacgttgacgcgccggaggatctgctgcagacctggtacattaaccgtttcctgaaatttcgtgagggtgcgttcaccgacccggatagctactttcacaactatgcgaaactgaccaaggaagaggcgatcaaaaccgcgatgaccatttggaaggagatgaactggctgaacctgaagcaaaacattctgccgacccgtgaacgtgcgagcctgattctgaccaaaagcgcgaaccacgcggtggaggaagttcgtctgcgtaag

SEQ ID NO: 72 - protein, 316 aa, Artificial Sequence
  Pantothenate Kinase from Escherichia coli variant
MSIKEQTLMTPYLQLDRNQWAALRDSNPMTLSEDEIARLKGINEDLSLEEVAEIYLPLSRLLNFYISSNLRRQAVLEQFLGTNGQRIPYIISIAGSVAVGKSTTARVLQALLSRWPEHRRVELITTDGFLHPNQVLKERGLMKKKGFPESYDMHRLVKFVSDLKSGVPNVTAPVYSHLIYDVIPDGDKTVVQPDILILEGLNVLQSGMDYPHDPHHVFVSDFVDFSIYVDAPEDLLQTWYINRFLKFREGAFTDPDSYFHNYAKLTKEEAIKTAMTIWKEMNWLNLKQNILPTRERASLILTKSANHAVEEVRLRK

SEQ ID NO: 73 - DNA, 948 bp, Artificial Sequence
  Pantothenate Kinase from Escherichia coli variant
atgagcatcaaagagcagaccctgatgaccccgtacctgcagttcgaccgtaaccaatgggcggcgctgagcgatagcgttccgatgcgcctgagcgaggacgaaatcgcgcgtctgaagggtattaacgaggatctgagcctggaggaagtggcggaaatctacctgccgctgagccgtctgctgaacttctatattagcagcaacctgcgtcgtcaggcggaactggaacaatttctgggtaccaacggccagcgtatcccgtatatcattagcattgcgggtagcgtggcggttggcaaaagcaccaccgcgcgtgtgctgcaggcgctgctgagccgttggccggagcaccgtcgtgttgaactgatcaccaccgacggcttcctgcacccgaaccaagtgctgaaggagcgtggtctgatgaagaaaaagggtttcccggaaagctacgatatgcaccgtctggtgaaatttgttagcgacctgaagagcggtgtgccgaacgttaccgcgccggtgtacagccacctgatctatgatgttattccggacggcgataaaaccgtggttcagccggacatcctgatcctggagggtctgaacgtgctgcaaagcggcatggactatccgcacgatccgcaccacgtgtttgttagcgacttcgtggattttagcatctacgttgacgcgccggaggatctgctgcagacctggtacattaaccgtttcctgaaatttcgtgagggtgcgttcaccgacccggatagctactttcacaactatgcgaaactgaccaaggaagaggcgatcaaaaccgcgatgaccatttggaaggagatgaactggctgaacctgaagcaaaacattctgccgacccgtgaacgtgcgagcctgattctgaccaaaagcgcgaaccacgcggtggaggaagttcgtctgcgtaag

SEQ ID NO: 74 - protein, 316 aa, Artificial Sequence
  Pantothenate Kinase from Escherichia coli variant
MSIKEQTLMTPYLQFDRNQWAALSDSVPMRLSEDEIARLKGINEDLSLEEVAEIYLPLSRLLNFYISSNLRRQAELEQFLGTNGQRIPYIISIAGSVAVGKSTTARVLQALLSRWPEHRRVELITTDGFLHPNQVLKERGLMKKKGFPESYDMHRLVKFVSDLKSGVPNVTAPVYSHLIYDVIPDGDKTVVQPDILILEGLNVLQSGMDYPHDPHHVFVSDFVDFSIYVDAPEDLLQTWYINRFLKFREGAFTDPDSYFHNYAKLTKEEAIKTAMTIWKEMNWLNLKQNILPTRERASLILTKSANHAVEEVRLRK

SEQ ID NO: 75 - DNA, 948 bp, Artificial Sequence
  Pantothenate Kinase from Escherichia coli variant
atgagcatcaaagagcagaccctgatgaccccgtacctgcagttcgaccgtaaccgctgggcggctctgcgtgattcggttccgtcgaccctgagcgaggacgaaatcgcgcgtctgaagggtattaacgaggatctgagcctggaggaagtggcggaaatctacctgccgctgagccgtctgctgaacttctatattagcagcaacctgcgtcgtcaggcggttctggaacaatttctgggtaccaacggccagcgtatcccgtatatcattagcattgcgggtagcgtggcggttggcaaaagcaccaccgcgcgtgtgctgcaggcgctgctgagccgttggccggagcaccgtcgtgttgaactgatcaccaccgacggcttcctgcacccgaaccaagtgctgaaggagcgtggtctgatgaagaaaaagggtttcccggaaagctacgatatgcaccgtctggtgaaatttgttagcgacctgaagagcggtgtgccgaacgttaccgcgccggtgtacagccacctgatctatgatgttattccggacggcgataaaaccgtggttcagccggacatcctgattctggagggtctgaacgtgctgcaaagcggcatggactatccgcacgatccgcaccatgtgtttgttagcgacttcgtggattttagcatctacgttgacgcgccggaggatctgctgcagacctggtacattaaccgtttcctgaaatttcgtgagggtgcgttcaccgacccggatagctactttcacaactatgcgaaactgaccaaggaagaggcgatcaaaaccgcgatgaccatttggaaggagatgaactggctgaacctgaagcaaaacattctgccgacccgtgaacgtgcgagcctgattctgaccaaaagcgcgaaccacgcggtggaggaagttcgtctgcgtaag

SEQ ID NO: 76 - protein, 316 aa, Artificial Sequence
  Pantothenate Kinase from Escherichia coli variant
MSIKEQTLMTPYLQFDRNRWAALRDSVPSTLSEDEIARLKGINEDLSLEEVAEIYLPLSRLLNFYISSNLRRQAVLEQFLGTNGQRIPYIISIAGSVAVGKSTTARVLQALLSRWPEHRRVELITTDGFLHPNQVLKERGLMKKKGFPESYDMHRLVKFVSDLKSGVPNVTAPVYSHLIYDVIPDGDKTVVQPDILILEGLNVLQSGMDYPHDPHHVFVSDFVDFSIYVDAPEDLLQTWYINRFLKFREGAFTDPDSYFHNYAKLTKEEAIKTAMTIWKEMNWLNLKQNILPTRERASLILTKSANHAVEEVRLRK

SEQ ID NO: 77 - DNA, 948 bp, Artificial Sequence
  Pantothenate Kinase from Escherichia coli variant
atgagcatcaaagagcagaccctgatgaccccgtacctgcagttcgaccgtaaccgctgggcggatctgcgtgatccggttccgatgaccctgagcgaggacgaaatcgcgcgtctgaagggtattaacgaggatctgagcctggaggaagtggcggaaatctacctgccgctgagccgtctgctgaacttctatattagcagctacctgcgtcgtcaggcggttctggaacaatttctgggtaccaacggccagcgtatcccgtatatcattagcattgcgggtagcgtggcggttggcaaaagcaccaccgcgcgtgtgctgcaggcgctgctgagccgttggccggagcaccgtcgtgttgaactgatcaccaccgacggcttcctgcacccgaaccaagtgctgaaggagcgtggtctgatgaagaaaaagggtttcccggaaagctacgatatgcaccgtctggtgaaatttgttagcgacctgaagagcggtgtgccgaacgttaccgcgccggtgtacagccacctgatctatgatgttattccggacggcgataaaaccgtggttcagccggacatcctgattctggagggtctgaacgtgctgcaaagcggcatggactatccgcacgatccgcaccacgtgtttgttagcgacttcgtggattttagcatctacgttgacgcgccggaggatctgctgcagacctggtacattaaccgtttcctgaaatttcgtgagggtgcgttcaccgacccggatagctactttcacaactatgcgaaactgaccaaggaagaggcgatcaaaaccgcgatgaccatttggaaggagatgaactggctgaacctgaagcaaaacattctgccgacccgtgaacgtgcgagcctgattctgaccaaaagcgcgaaccacgcggtggaggaagttcgtctgcgtaag

SEQ ID NO: 78 - protein, 316 aa, Artificial Sequence
  Pantothenate Kinase from Escherichia coli variant
MSIKEQTLMTPYLQFDRNRWADLRDPVPMTLSEDEIARLKGINEDLSLEEVAEIYLPLSRLLNFYISSYLRRQAVLEQFLGTNGQRIPYIISIAGSVAVGKSTTARVLQALLSRWPEHRRVELITTDGFLHPNQVLKERGLMKKKGFPESYDMHRLVKFVSDLKSGVPNVTAPVYSHLIYDVIPDGDKTVVQPDILILEGLNVLQSGMDYPHDPHHVFVSDFVDFSIYVDAPEDLLQTWYINRFLKFREGAFTDPDSYFHNYAKLTKEEAIKTAMTIWKEMNWLNLKQNILPTRERASLILTKSANHAVEEVRLRK

SEQ ID NO: 79 - DNA, 948 bp, Artificial Sequence
  Pantothenate Kinase from Escherichia coli variant
atgagcatcaaagagcagaccctgatgaccccgtacctgcagtttgaccgtaaccaatgggcggcgctgcgtgatagtaacccgatgaccctgagcgaggacgaaatcgcgcgtctgaagggtattaacgaggatctgagcctggaggaagtggcggaaatctacctgccgctgagccgtctgctgaacttctatattagcagcaacctgcgtcgtcaggcggttctggaacaatttctgggtaccaacggccagcgtatcccgtatatcattagcattgcgggtagcgtggcggttggcaaaagcaccaccgcgcgtgtgctgcaggcgctgctgagccgttggccggagcaccgtcgtgttgaactgatcaccaccgacggcttcctgcacccgaaccaagtgctgaaggagcgtggtctgatgaagaaaaagggtttcccggaaagctacgatatgcaccgtctggtgaaatttgttagcgacctgaagagcggtgtgccgaacgttaccgcgccggtgtacagccacctgatctatgatgttattccggacggcgataaaaccgtggttcagccggacatcctgattctggagggtctgaacgtgctgcaaagcggcatggactatccgcacgatccgcaccacgtgtttgttagcgacttcgtggattttagcatctacgttgacgcgccggaggatctgctgcagacctggtacattaaccgtttcctgaaatttcgtgagggtgcgttcaccgacccggatagctactttcacaactatgcgaaactgaccaaggaagaggcgatcaaaaccgcgatgaccatttggaaggagatgaacctgctgaacctgaagcaaaacattctgccgacccgtgaacgtgcgagcctgattctgaccaaaagcgcgaaccacgcggtggaggaagttcgtctgcgtaag

SEQ ID NO: 80 - protein, 316 aa, Artificial Sequence
  Pantothenate Kinase from Escherichia coli variant
MSIKEQTLMTPYLQFDRNQWAALRDSNPMTLSEDEIARLKGINEDLSLEEVAEIYLPLSRLLNFYISSNLRRQAVLEQFLGTNGQRIPYIISIAGSVAVGKSTTARVLQALLSRWPEHRRVELITTDGFLHPNQVLKERGLMKKKGFPESYDMHRLVKFVSDLKSGVPNVTAPVYSHLIYDVIPDGDKTVVQPDILILEGLNVLQSGMDYPHDPHHVFVSDFVDFSIYVDAPEDLLQTWYINRFLKFREGAFTDPDSYFHNYAKLTKEEAIKTAMTIWKEMNLLNLKQNILPTRERASLILTKSANHAVEEVRLRK

SEQ ID NO: 81 - DNA, 948 bp, Artificial Sequence
  Pantothenate Kinase from Escherichia coli variant
atgagcatcaaagagcagaccctgatgaccccgtacctgcagctggaccgtaaccaatgggcggcgctgcgtgatagtaacccgatgaccctgagcgaggacgaaatcgcgcgtctgaagggtattaacgaggatctgagcctggaggaagtggcggaaatctacctgccgctgagccgtctgctgaacttctatattagcagcaacctgcgtcgtcaggcggttctggaacaatttctgggtaccaacggccagcgtatcccgtatatcattagcattgcgggtagcgtggcggttggcaaaagcaccaccgcgcgtgtgctgcaggcgctgctgagccgttggccggagcaccgtcgtgttgaactgatcaccaccgacggcttcctgcacccgaaccaagtgctgaaggagcgtggtctgatgaagaaaaagggtttcccggaaagctacgatatgcaccgtctggtgaaatttgttagcgacctgaagagcggtgtgccgaacgttaccgcgccggtgtacagccacctgatctatgatgttattccggacggcgataaaaccgtggttcagccggacatcctgattctggagggtctgaacgtgctgcaaagcggcatggactatccgcacgatccgcaccacgtgtttgttagcgacttcgtggattttagcatctacgttgacgcgccggaggatctgctgcagacctggtacattaaccgtttcctgaaatttcgtgagggtgcgttcaccgacccggatagctactttcacaactatgcgaaactgaccaaggaagaggcgatcaaaaccgcgatgaccatttggaaggagatgaacctgctgaacctgaagcaaaacattctgccgacccgtgaacgtgcgagcctgattctgaccaaaagcatcaaccacgcggtggaggaagttcgtctgcgtaag

SEQ ID NO: 82 - protein, 316 aa, Artificial Sequence
  Pantothenate Kinase from Escherichia coli variant
MSIKEQTLMTPYLQLDRNQWAALRDSNPMTLSEDEIARLKGINEDLSLEEVAEIYLPLSRLLNFYISSNLRRQAVLEQFLGTNGQRIPYIISIAGSVAVGKSTTARVLQALLSRWPEHRRVELITTDGFLHPNQVLKERGLMKKKGFPESYDMHRLVKFVSDLKSGVPNVTAPVYSHLIYDVIPDGDKTVVQPDILILEGLNVLQSGMDYPHDPHHVFVSDFVDFSIYVDAPEDLLQTWYINRFLKFREGAFTDPDSYFHNYAKLTKEEAIKTAMTIWKEMNLLNLKQNILPTRERASLILTKSINHAVEEVRLRK

SEQ ID NO: 83 - DNA, 948 bp, Artificial Sequence
  Pantothenate Kinase from Escherichia coli variant
atgagcatcaaagagcagaccctgatgaccccgtacctgcagttcgaccgtaaccaaatggcggcgctgagcactagcgttccgatgacgctgagcgaggacgaaatcgcgcgtctgaagggtattaacgaggatctgagcctggaggaagtggcggaaatctacctgccgctgagccgtctgctgaacttctatattagcagcaccctgcgtcgtcaggcggaactggaacaatttctgggtaccaacggccagcgtatcccgtatatcattagcattgcgggtagcgtggcggttggcaaaagcaccaccgcgcgtgtgctgcaggcgctgctgagccgttggccggagcaccgtcgtgttgaactgatcaccaccgacggcttcctgcacccgaaccaagtgctgaaggagcgtggtctgatgaagaaaaagggtttcccggaaagctacgatatgcaccgtctggtgaaatttgttagcgacctgaagagcggtgtgccgaacgttaccgcgccggtgtacagccacctgatctatgatgttattccggacggcgataaaaccgtggttcagccggacatcctgatcctggagggtctgaacgtgctgcaaagcggcatggactatccgcacgatccgcaccacgtgtttgttagcgacttcgtggattttagcatctacgttgacgcgccggaggatctgctgcagacctggtacattaaccgtttcctgaaatttcgtgagggtgcgttcaccgacccggatagctactttcacaactatgcgaaactgaccaaggaagaggcgatcaaaaccgcgatgaccatttggaaggagatgaactggctgaacctgaagcaaaacattctgccgacccgtgaacgtgcgagcctgattctgaccaaaagcgcgaaccacgcggtggaggaagttcgtctgcgtaag

SEQ ID NO: 84 - protein, 316 aa, Artificial Sequence
  Pantothenate Kinase from Escherichia coli variant
MSIKEQTLMTPYLQFDRNQMAALSTSVPMTLSEDEIARLKGINEDLSLEEVAEIYLPLSRLLNFYISSTLRRQAELEQFLGTNGQRIPYIISIAGSVAVGKSTTARVLQALLSRWPEHRRVELITTDGFLHPNQVLKERGLMKKKGFPESYDMHRLVKFVSDLKSGVPNVTAPVYSHLIYDVIPDGDKTVVQPDILILEGLNVLQSGMDYPHDPHHVFVSDFVDFSIYVDAPEDLLQTWYINRFLKFREGAFTDPDSYFHNYAKLTKEEAIKTAMTIWKEMNWLNLKQNILPTRERASLILTKSANHAVEEVRLRK

SEQ ID NO: 85 - DNA, 948 bp, Artificial Sequence
  Pantothenate Kinase from Escherichia coli variant
atgagcatcaaagagcagaccctgatgaccccgtacctgcagctggaccgtaaccaatgggcggcgctgcgtgatagtaacccgatgaccctgagcgaggacgaaatcgcgcgtctgaagggtattaacgaggatctgagcctggaggaagtggcggaaatctacctgccgctgagccgtctgctgaacttctatattagcagcaacctgcgtcgtcaggcggttctggaacaatttctgggtaccaacggccagcgtatcccgtatatcattagcattgcgggtagcgtggcggttggcaaaagcaccaccgcgcgtgtgctgcaggcgctgctgagccgttggccggagcaccgtcgtgttgaactgatcaccaccgacggcttcctgcacccgaaccaagtgctgaaggagcgtggtctgatgaagaaaaagggtttcccggaaagctacgatatgcaccgtctggtgaaatttgttagcgacctgaagagcggtgtgccgaacgttaccgcgccggtgtacagccacctgatctatgatgttattccggacggcgataaaaccgtggttcagccggacatcctgattctggagggtctgaacgtgctgcaaagcggcatggactatccgcacgatccgcaccacgtgtttgttagcgacttcgtggattttagcatctacgttgacgcgccggaggatctgctgcagacctggtacattaaccgtttcctgaaatttcgtgagggtgcgttcaccgacccggatagctactttcacaactatgcgaaactgaccaaggaagaggcgatcaaaaccgcgatgaccatttggaaggagatgaactggctgaacctgaagcaaaacattctgccgacccgtgaacgtgcgagcctgattctgaccaaaagcatcaaccacgcggtggaggaagttcgtctgcgtaag

SEQ ID NO: 86 - protein, 316 aa, Artificial Sequence
  Pantothenate Kinase from Escherichia coli variant
MSIKEQTLMTPYLQLDRNQWAALRDSNPMTLSEDEIARLKGINEDLSLEEVAEIYLPLSRLLNFYISSNLRRQAVLEQFLGTNGQRIPYIISIAGSVAVGKSTTARVLQALLSRWPEHRRVELITTDGFLHPNQVLKERGLMKKKGFPESYDMHRLVKFVSDLKSGVPNVTAPVYSHLIYDVIPDGDKTVVQPDILILEGLNVLQSGMDYPHDPHHVFVSDFVDFSIYVDAPEDLLQTWYINRFLKFREGAFTDPDSYFHNYAKLTKEEAIKTAMTIWKEMNWLNLKQNILPTRERASLILTKSINHAVEEVRLRK

SEQ ID NO: 87 - DNA, 948 bp, Artificial Sequence
  Pantothenate Kinase from Escherichia coli variant
atgagcatcaaagagcagaccctgatgaccccgtacctgcagctggaccgtaaccaatgggcggcgctgcgtgatagtaacccgatgaccctgagcgaggacgaaatcgcgcgtctgaagggtattaacgaggatctgagcctggaggaagtggcggaaatctacctgccgctgagccgtctgctgaacttctatattagcagcaacctgcgtcgtcaggcggttctggaacaatttctgggtaccaacggccagcgtatcccgtatatcattagcattgcgggtagcgtggcggttggcaaaagcaccaccgcgcgtgtgctgcaggcgctgctgagccgttggccggagcaccgtcgtgttgaactgatcaccaccgacggcttcctgcacccgaaccaagtgctgaaggagcgtggtctgatgaagaaaaagggtttcccggaaagctacgatatgcaccgtctggtgaaatttgttagcgacctgaagagcggtgtgccgaacgttaccgcgccggtgtacagccacctgatctatgatgttattccggacggcgataaaaccgtggttcagccggacatcctgattctggagggtctgaacgtgctgcaaagcggcatggactatccgcacgatccgcaccacgtgtttgttagcgacttcgtggattttagcatctacgttgacgcgccggaggatctgctgcagacctggtacattaaccgtttcctgaaatttcgtgagggtgcgttcaccgacccggatagctactttcacaactatgcgaaactgaccaaggaagaggcgatcaaaaccgcgatgaccatttggaaggagatgaacctgctgaacctgaagcaaaacattctgccgacccgtgaacgtgcgagcctgattctgaccaaaagcgcgaaccacgcggtggaggaagttcgtctgcgtaag

SEQ ID NO: 88 - protein, 316 aa, Artificial Sequence
  Pantothenate Kinase from Escherichia coli variant
MSIKEQTLMTPYLQLDRNQWAALRDSNPMTLSEDEIARLKGINEDLSLEEVAEIYLPLSRLLNFYISSNLRRQAVLEQFLGTNGQRIPYIISIAGSVAVGKSTTARVLQALLSRWPEHRRVELITTDGFLHPNQVLKERGLMKKKGFPESYDMHRLVKFVSDLKSGVPNVTAPVYSHLIYDVIPDGDKTVVQPDILILEGLNVLQSGMDYPHDPHHVFVSDFVDFSIYVDAPEDLLQTWYINRFLKFREGAFTDPDSYFHNYAKLTKEEAIKTAMTIWKEMNLLNLKQNILPTRERASLILTKSANHAVEEVRLRK

SEQ ID NO: 89 - DNA, 948 bp, Artificial Sequence
  Pantothenate Kinase from Escherichia coli variant
atgagcatcaaagagcagaccctgatgaccccgtacctgcagttcgaccgtaaccaaatggcggcgctggcggatagcgttccgatgacgctgagcgaggacgaaatcgcgcgtctgaagggtattaacgaggatctgagcctggaggaagtggcggaaatctacctgccgctgagccgtctgctgaacttctatattagcagcaacctgcgtcgtcaggcggttctggaacaatttctgggtaccaacggccagcgtatcccgtatatcattagcattgcgggtagcgtggcggttggcaaaagcaccaccgcgcgtgtgctgcaggcgctgctgagccgttggccggagcaccgtcgtgttgaactgatcaccaccgacggcttcctgcacccgaaccaggtgctgaaggagcgtggtctgatgaagaaaaagggtttcccggaaagctacgatatgcaccgtctggtgaaatttgttagcgacctgaagagcggtgtgccgaacgttaccgcgccggtgtacagccacctgatctatgatgttattccggacggcgataaaaccgtggttcagccggacatcctgatcctggagggtctgaacgtgctgcaaagcggcatggactatccgcacgatccgcaccacgtgtttgttagcgacttcgtggattttagcatctacgttgacgcgccggaggatctgctgcagacctggtacattaaccgtttcctgaaatttcgtgagggtgcgttcaccgacccggatagctactttcacaactatgcgaaactgaccaaggaagaggcgatcaaaaccgcgatgaccatttggaaggagatgaactggctgaacctgaagcaaaacattctgccgacccgtgaacgtgcgagcctgattctgaccaaaagcgcgaaccacgcggtggaggaagttcgtctgcgtaag

SEQ ID NO: 90 - protein, 316 aa, Artificial Sequence
  Pantothenate Kinase from Escherichia coli variant
MSIKEQTLMTPYLQFDRNQMAALADSVPMTLSEDEIARLKGINEDLSLEEVAEIYLPLSRLLNFYISSNLRRQAVLEQFLGTNGQRIPYIISIAGSVAVGKSTTARVLQALLSRWPEHRRVELITTDGFLHPNQVLKERGLMKKKGFPESYDMHRLVKFVSDLKSGVPNVTAPVYSHLIYDVIPDGDKTVVQPDILILEGLNVLQSGMDYPHDPHHVFVSDFVDFSIYVDAPEDLLQTWYINRFLKFREGAFTDPDSYFHNYAKLTKEEAIKTAMTIWKEMNWLNLKQNILPTRERASLILTKSANHAVEEVRLRK

SEQ ID NO: 91 - DNA, 948 bp, Artificial Sequence
  Pantothenate Kinase from Escherichia coli variant
atgagcatcaaagagcagaccctgatgaccccgtacctgcagtttgaccgtaaccaatgggcggcgctgcgtgatagtaacccgatgaccctgagcgaggacgaaatcgcgcgtctgaagggtattaacgaggatctgagcctggaggaagtggcggaaatctacctgccgctgagccgtctgctgaacttctatattagcagcaacctgcgtcgtcaggcggttctggaagcgtttctgggtaccaacggccagcgtatcccgtatatcattagcattgcgggtagcgtggcggttggcaaaagcaccaccgcgcgtgtgctgcaggcgctgctgagccgttggcctgagcaccgtcgtgttgaactgatcaccaccgacggcttcctgcacccgaaccaagtgctgaaggagcgtggtctgatgaagaaaaagggtttcccggaaagctacgatatgcaccgtctggtgaaatttgttagcgacctgaagagcggtgtgccgaacgttaccgcgccggtgtacagccacctgatctatgatgttattccggacggcgataaaaccgtggttcagccggacatcctgattctggagggtctgaacgtgctgcaaagcggcatggactatccgcacgatccgcaccacgtgtttgttagcgacttcgtggattttagcatctacgttgacgcgccggaggatctgctgcagacctggtacattaaccgtttcctgaaatttcgtgagggtgcgttcaccgacccggatagctactttcacaactatgcgaaactgaccaaggaagaggcgatcaaaaccgcgatgaccatttggaaggagatgaactggctgaacctgaagcaaaacattctgccgacccgtgaacgtgcgagcctgattctgaccaaaagcgcgaaccacgcggtggaggaagttcgtctgcgtaag

SEQ ID NO: 92 - protein, 316 aa, Artificial Sequence
  Pantothenate Kinase from Escherichia coli variant
MSIKEQTLMTPYLQFDRNQWAALRDSNPMTLSEDEIARLKGINEDLSLEEVAEIYLPLSRLLNFYISSNLRRQAVLEAFLGTNGQRIPYIISIAGSVAVGKSTTARVLQALLSRWPEHRRVELITTDGFLHPNQVLKERGLMKKKGFPESYDMHRLVKFVSDLKSGVPNVTAPVYSHLIYDVIPDGDKTVVQPDILILEGLNVLQSGMDYPHDPHHVFVSDFVDFSIYVDAPEDLLQTWYINRFLKFREGAFTDPDSYFHNYAKLTKEEAIKTAMTIWKEMNWLNLKQNILPTRERASLILTKSANHAVEEVRLRK

SEQ ID NO: 93 - DNA, 948 bp, Artificial Sequence
  Pantothenate Kinase from Escherichia coli variant
atgagcatcaaagagcagaccctgatgaccccgtacctgcagctggaccgtaaccaatgggcggcgctgcgtgatctggtgccgatgaccctgagcgaggacgaaatcgcgcgtctgaagggtattaacgaggatctgagcctggaggaagtggcggaaatctacctgccgctgagccgtctgctgaacttctatattagcagcaacctgcgtcgtcaggcggttctggaacaatttctgggtaccaacggccagcgtatcccgtatatcattagcattgcgggtagcgtggcggttggcaaaagcaccaccgcgcgtgtgctgcaggcgctgctgagccgttggccggagcaccgtcgtgttgaactgatcaccaccgacggcttcctgcacccgaaccaagtgctgaaggagcgtggtctgatgaagaaaaagggtttcccggaaagctacgatatgcaccgtctggtgaaatttgttagcgacctgaagagcggtgtgccgaacgttaccgcgccggtgtacagccacctgatctatgatgttattccggacggcgataaaaccgtggttcagccggacatcctgattctggagggtctgaacgtgctgcaaagcggcatggactatccgcacgatccgcaccacgtgtttgttagcgacttcgtggattttagcatctacgttgacgcgccggaggatctgctgcagacctggtacattaaccgtttcctgaaatttcgtgagggtgcgttcaccgacccggatagctactttcacaactatgcgaaactgaccaaggaagaggcgatcaaaaccgcgatgaccatttggaaggagatgaaccacctgaacctgaagcaaaacattctgccgacccgtgaacgtgcgagcctgattctgaccaaaagcgcgaaccacgcggtggaggaagttcgtctgcgtaag

SEQ ID NO: 94 - protein, 316 aa, Artificial Sequence
  Pantothenate Kinase from Escherichia coli variant
MSIKEQTLMTPYLQLDRNQWAALRDLVPMTLSEDEIARLKGINEDLSLEEVAEIYLPLSRLLNFYISSNLRRQAVLEQFLGTNGQRIPYIISIAGSVAVGKSTTARVLQALLSRWPEHRRVELITTDGFLHPNQVLKERGLMKKKGFPESYDMHRLVKFVSDLKSGVPNVTAPVYSHLIYDVIPDGDKTVVQPDILILEGLNVLQSGMDYPHDPHHVFVSDFVDFSIYVDAPEDLLQTWYINRFLKFREGAFTDPDSYFHNYAKLTKEEAIKTAMTIWKEMNHLNLKQNILPTRERASLILTKSANHAVEEVRLRK

SEQ ID NO: 95 - DNA, 948 bp, Artificial Sequence
  Pantothenate Kinase from Escherichia coli variant
atgagcatcaaagagcagaccctgatgaccccgtacgatcaattcgaccgtaaccaatgggcgaccctgcgtgatagcgttccgatgaccctgagcgaggacgaaatcgcgcgtctgaagggtattaacgaggatctgagcctggaggaagtggcggaaatctacctgccgctgagccgtctgctgaacttctatattagcagcaacctgcgtcgtcaggcggttctggaacaatttctgggtaccaacggccagcgtatcccgtatatcattagcattgcgggtagcgtggcggttggcaaaagcaccaccgcgcgtgtgctgcaggcgctgctgagccgttggccggagcaccgtcgtgttgaactgatcaccaccgacggcttcctgcacccgaaccaagtgctgaaggagcgtggtctgatgaagaaaaagggtttcccggaaagctacgatatgcaccgtctggtgaaatttgttagcgacctgaagagcggtgtgccgaacgttaccgcgccggtgtacagccacctgatctatgatgttattccggacggcgataaaaccgtggttcagccggacatcctgattctggagggtctgaacgtgctgcaaagcggcatggactatccgcacgatccgcaccacgtgttcgttagcgacttcgtggattttagcatctacgttgacgcgccggaggatctgctgcagacctggtacattaaccgtttcctgaaatttcgtgagggtgcgttcaccgacccggatagctactttcacaactatgcgaaactgaccaaggaagaggcgatcaaaaccgcgatgaccatctggaaggagatgaactggctgaacctgaagcaaaacattctgccgacccgtgaacgtgcgagcctgattctgaccaaaagcgcgaaccacgcggtggaggaagttcgtctgcgtaag

SEQ ID NO: 96 - protein, 316 aa, Artificial Sequence
  Pantothenate Kinase from Escherichia coli variant
MSIKEQTLMTPYDQFDRNQWATLRDSVPMTLSEDEIARLKGINEDLSLEEVAEIYLPLSRLLNFYISSNLRRQAVLEQFLGTNGQRIPYIISIAGSVAVGKSTTARVLQALLSRWPEHRRVELITTDGFLHPNQVLKERGLMKKKGFPESYDMHRLVKFVSDLKSGVPNVTAPVYSHLIYDVIPDGDKTVVQPDILILEGLNVLQSGMDYPHDPHHVFVSDFVDFSIYVDAPEDLLQTWYINRFLKFREGAFTDPDSYFHNYAKLTKEEAIKTAMTIWKEMNWLNLKQNILPTRERASLILTKSANHAVEEVRLRK

SEQ ID NO: 97 - DNA, 948 bp, Artificial Sequence
  Pantothenate Kinase from Escherichia coli variant
atgagcatcaaagagcagaccctgatgaccccgtacgatgaattcgaccgtaaccaatgggcgaccctgcgtgatagcgttccgatgaccctgagcgaggacgaaatcgcgcgtctgaagggtattaacgaggatctgagcctggaggaagtggcggaaatctacctgccgctgagccgtctgctgaacttctatattagcagcaacctgcgtcgtcaggcggttctggaacaatttctgggtaccaacggccagcgtatcccgtatatcattagcattgcgggtagcgtggcggttggcaaaagcaccaccgcggcagtgctgcaggcgctgctgagccgttggccggagcaccgtcgtgttgaactgatcaccaccgacggcttcctgcacccgaaccaagtgctgaaggagcgtggtctgatgaagaaaaagggtttcccggaaagctacgatatgcaccgtctggtgaaatttgttagcgacctgaagagcggtgtgccgaacgttaccgcgccggtgtacagccacctgatctatgatgttattccggacggcgataaaaccgtggttcagccagacatcctgattctggagggtctgaacgtgctgcaaagcggcatggactatccgcacgatccgcaccacgtgttcgttagcgacttcgtggattttagcatctacgttgacgcgccggaggatctgctgcagacctggtacattaaccgtttcctgaaaatgcgtgagggtgcgttcaccgacccggatagctactttcacaactatgcgaaactgaccaaggaagaggcgattaaaaccgcgatgaccatttggaaggagatgaactggctgaacctgaagcaaaacattctgccgacccgtgaacgtgcgagcctgattctgaccaaaagcgcgaaccacgcggtggaggaagttcgtctgcgtaag

SEQ ID NO: 98 - protein, 316 aa, Artificial Sequence
  Pantothenate Kinase from Escherichia coli variant
MSIKEQTLMTPYDEFDRNQWATLRDSVPMTLSEDEIARLKGINEDLSLEEVAEIYLPLSRLLNFYISSNLRRQAVLEQFLGTNGQRIPYIISIAGSVAVGKSTTAAVLQALLSRWPEHRRVELITTDGFLHPNQVLKERGLMKKKGFPESYDMHRLVKFVSDLKSGVPNVTAPVYSHLIYDVIPDGDKTVVQPDILILEGLNVLQSGMDYPHDPHHVFVSDFVDFSIYVDAPEDLLQTWYINRFLKMREGAFTDPDSYFHNYAKLTKEEAIKTAMTIWKEMNWLNLKQNILPTRERASLILTKSANHAVEEVRLRK

SEQ ID NO: 99 - DNA, 948 bp, Artificial Sequence
  Pantothenate Kinase from Escherichia coli variant
atgagcatcaaagagcagaccctgatgaccccgtacctgcagttcgaccgtaaccaatgggcggcgctgcgtgatagcgttccgatgacgctgagcgaggacgaaatcgcgcgtctgaagggtattaacgaggatctgagcctggaggaagtggcggaaatctacctgccgctgagccgtctgctgaacttctatattagcagcaacctgcgtcgtcaggcggaactggaacaatttctgggtaccaacggccagcgtatcccgtatatcattagcattgcgggtagcgtggcggttggcaaaagcaccaccgcgcgtgtgctgcaggcgctgctgagccgttggccggagcaccgtcgtgttgaactgatcaccaccgacggcttcctgcacccgaaccaggtgctgaaggagcgtggtctgatgaagaaaaagggtttcccggaaagctacgatatgcaccgtctggtgaaatttgttagcgacctgaagagcggtgtgccgaacgttaccgcgccggtgtacagccacctgatctatgatgttattccggacggcgataaaaccgtggttcagccggacatcctgatcctggagggtctgaacgtgctgcaaagcggcatggactatccgcacgatccgcaccacgtgtttgttagcgacttcgtggattttagcatctacgttgacgcgccggaggatctgctgcagacctggtacattaaccgtttcctgaaatttcgtgagggtgcgttcaccgacccggatagctactttcacaactatgcgaaactgaccaaggaagaggcgatcaaaaccgcgatgaccatttggaaggagatgaactggctgaacctgaagcaaaacattctgccgacccgtgaacgtgcgagcctgattctgaccaaaagcgcgaaccacgcggtggaggaagttcgtctgcgtaag

SEQ ID NO: 100 - protein, 316 aa, Artificial Sequence
  Pantothenate Kinase from Escherichia coli variant
MSIKEQTLMTPYLQFDRNQWAALRDSVPMTLSEDEIARLKGINEDLSLEEVAEIYLPLSRLLNFYISSNLRRQAELEQFLGTNGQRIPYIISIAGSVAVGKSTTARVLQALLSRWPEHRRVELITTDGFLHPNQVLKERGLMKKKGFPESYDMHRLVKFVSDLKSGVPNVTAPVYSHLIYDVIPDGDKTVVQPDILILEGLNVLQSGMDYPHDPHHVFVSDFVDFSIYVDAPEDLLQTWYINRFLKFREGAFTDPDSYFHNYAKLTKEEAIKTAMTIWKEMNWLNLKQNILPTRERASLILTKSANHAVEEVRLRK

SEQ ID NO: 101 - DNA, 948 bp, Artificial Sequence
  Pantothenate Kinase from Escherichia coli variant
atgagcatcaaagagcagaccctgatgaccccgtacctgcagttcgaccgtaaccagtgggcggctctgcgtgattcggttccgtcgaccctgagcgaggacgaaatcgcgcgtctgaagggtattaacgaggatctgagcctggaggaagtggcggaaatctacctgccgctgagccgtctgctgaacttctatattagcagcaacctgcgtcgtcaggcggttctggaacaatttctgggtaccaacggccagcgtatcccgtatatcattagcattgcgggtagcgtggcggttggcaaaagcaccaccgcgcgtgtgctgcaggcgctgctgagccgttggccggagcaccgtcgtgttgaactgatcaccaccgacggcttcctgcacccgaaccaagtgctgaaggagcgtggtctgatgaagaaaaagggtttcccggaaagctacgatatgcaccgtctggtgaaatttgttagcgacctgaagagcggtgtgccgaacgttaccgcgccggtgtacagccacctgatctatgatgttattccggacggcgataaaaccgtggttcagccggacatcctgattctggagggtctgaacgtgctgcaaagcggcatggactatccgcacgatccgcaccacgtgtttgttagcgacttcgtggattttagcatctacgttgacgcgccggaggatctgctgcagacctggtacattaaccgtttcctgaaatttcgtgagggtgcgttcaccgacccggatagctactttcacaactatgcgaaactgaccaaggaagaggcgatcaaaaccgcgatgaccatttggaaggagatgaactggctgaacctgaagcaaaacattctgccgacccgtgaacgtgcgagcctgattctgaccaaaagcgcgaaccacgcggtggaggaagttcgtctgcgtaag

SEQ ID NO: 102 - protein, 316 aa, Artificial Sequence
  Pantothenate Kinase from Escherichia coli variant
MSIKEQTLMTPYLQFDRNQWAALRDSVPSTLSEDEIARLKGINEDLSLEEVAEIYLPLSRLLNFYISSNLRRQAVLEQFLGTNGQRIPYIISIAGSVAVGKSTTARVLQALLSRWPEHRRVELITTDGFLHPNQVLKERGLMKKKGFPESYDMHRLVKFVSDLKSGVPNVTAPVYSHLIYDVIPDGDKTVVQPDILILEGLNVLQSGMDYPHDPHHVFVSDFVDFSIYVDAPEDLLQTWYINRFLKFREGAFTDPDSYFHNYAKLTKEEAIKTAMTIWKEMNWLNLKQNILPTRERASLILTKSANHAVEEVRLRK

SEQ ID NO: 103 - DNA, 948 bp, Artificial Sequence
  Pantothenate Kinase from Escherichia coli variant
atgagcatcaaagagcagaccctgatgaccccgtacctgcagttcgaccgtaaccaatgggcggcgctggcggatagcgttccgatgcgcctgagcgaggacgaaatcgcgcgtctgaagggtattaacgaggatctgagcctggaggaagtggcggaaatctacctgccgctgagccgtctgctgaacttctatattagcagcaacctgcgtcgtcaggcggttctggaacaatttctgggtaccaacggccagcgtatcccgtatatcattagcattgcgggtagcgtggcggttggcaaaagcaccaccgcgcgtgtgctgcaggcgctgctgagccgttggccggagcaccgtcgtgttgaactgatcaccaccgacggcttcctgcacccgaaccaagtgctgaaggagcgtggtctgatgaagaaaaagggtttcccggaaagctacgatatgcaccgtctggtgaaatttgttagcgacctgaagagcggtgtgccgaacgttaccgcgccggtgtacagccacctgatctatgatgttattccggacggcgataaaaccgtggttcagccggacatcctgatcctggagggtctgaacgtgctgcaaagcggcatggactatccgcacgatccgcaccacgtgtttgttagcgacttcgtggattttagcatctacgttgacgcgccggaggatctgctgcagacctggtacattaaccgtttcctgaaatttcgtgagggtgcgttcaccgacccggatagctactttcacaactatgcgaaactgaccaaggaagaggcgatcaaaaccgcgatgaccatttggaaggagatgaactggctgaacctgaagcaaaacattctgccgacccgtgaacgtgcgagcctgattctgaccaaaagcgcgaaccacgcggtggaggaagttcgtctgcgtaag

SEQ ID NO: 104 - protein, 316 aa, Artificial Sequence
  Pantothenate Kinase from Escherichia coli variant
MSIKEQTLMTPYLQFDRNQWAALADSVPMRLSEDEIARLKGINEDLSLEEVAEIYLPLSRLLNFYISSNLRRQAVLEQFLGTNGQRIPYIISIAGSVAVGKSTTARVLQALLSRWPEHRRVELITTDGFLHPNQVLKERGLMKKKGFPESYDMHRLVKFVSDLKSGVPNVTAPVYSHLIYDVIPDGDKTVVQPDILILEGLNVLQSGMDYPHDPHHVFVSDFVDFSIYVDAPEDLLQTWYINRFLKFREGAFTDPDSYFHNYAKLTKEEAIKTAMTIWKEMNWLNLKQNILPTRERASLILTKSANHAVEEVRLRK

SEQ ID NO: 105 - DNA, 948 bp, Artificial Sequence
  Pantothenate Kinase from Escherichia coli variant
atgagcatcaaagagcagaccctgatgaccccgtacctgcagttcgaccgtaaccaatgggcggcgctggcggatagcgttccgatgacgctgagcgaggacgaaatcgcgcgtctgaagggtattaacgaggatctgagcctggaggaagtggcggaaatctacctgccgctgagccgtctgctgaacttctatattagcagcaacctgcgtcgtcaggcggttctggaacaatttctgggtaccaacggccagcgtatcccgtatatcattagcattgcgggtagcgtggcggttggcaaaagcaccaccgcgcgtgtgctgcaggcgctgctgagccgttggccggagcaccgtcgtgttgaactgatcaccaccgacggcttcctgcacccgaaccaagtgctgaaggagcgtggtctgatgaagaaaaagggtttcccggaaagctacgatatgcaccgtctggtgaaatttgttagcgacctgaagagcggtgtgccgaacgttaccgcgccggtgtacagccacctgatctatgatgttattccggacggcgataaaaccgtggttcagccggacatcctgattctggagggtctgaacgtgctgcaaagcggcatggactatccgcacgatccgcaccacgtgtttgttagcgacttcgtggattttagcatctacgttgacgcgccggaggatctgctgcagacctggtacattaaccgtttcctgaaatttcgtgagggtgcgttcaccgacccggatagctactttcacaactatgcgaaactgaccaaggaagaggcgatcaaaaccgcgatgaccatttggaaggagatgaactggctgaacctgaagcaaaacattctgccgacccgtgaacgtgcgagcctgattctgaccaaaagcgcgaaccacgcggtggaggaagttcgtctgcgtaag

SEQ ID NO: 106 - protein, 316 aa, Artificial Sequence
  Pantothenate Kinase from Escherichia coli variant
MSIKEQTLMTPYLQFDRNQWAALADSVPMTLSEDEIARLKGINEDLSLEEVAEIYLPLSRLLNFYISSNLRRQAVLEQFLGTNGQRIPYIISIAGSVAVGKSTTARVLQALLSRWPEHRRVELITTDGFLHPNQVLKERGLMKKKGFPESYDMHRLVKFVSDLKSGVPNVTAPVYSHLIYDVIPDGDKTVVQPDILILEGLNVLQSGMDYPHDPHHVFVSDFVDFSIYVDAPEDLLQTWYINRFLKFREGAFTDPDSYFHNYAKLTKEEAIKTAMTIWKEMNWLNLKQNILPTRERASLILTKSANHAVEEVRLRK

SEQ ID NO: 107 - DNA, 948 bp, Artificial Sequence
  Pantothenate Kinase from Escherichia coli variant
atgagcatcaaagagcagaccctgatgaccccgtacctgcagttcgaccgtaaccaatgggcggcgctgcgtgatctggtgccgatgaccctgagcgaggacgaaatcgcgcgtctgaagggtattaacgaggatctgagcctggaggaagtggcggaaatctacctgccgctgagccgtctgctgaacttctatattagcagcaacctgcgtcgtcaggcggttctggaacaatttctgggtaccaacggccagcgtatcccgtatatcattagcattgcgggtagcgtggcggttggcaaaagcaccaccgcgcgtgtgctgcaggcgctgctgagccgttggccggagcaccgtcgtgttgaactgatcaccaccgacggcttcctgcacccgaaccaagtgctgaaggagcgtggtctgatgaagaaaaagggtttcccggaaagctacgatatgcaccgtctggtgaaatttgttagcgacctgaagagcggtgtgccgaacgttaccgcgccggtgtacagccacctgatctatgatgttattccggacggcgataaaaccgtggttcagccggacatcctgattctggagggtctgaacgtgctgcaaagcggcatggactatccgcacgatccgcaccacgtgtttgttagcgacttcgtggattttagcatctacgttgacgcgccggaggatctgctgcagacctggtacattaaccgtttcctgaaatttcgtgagggtgcgttcaccgacccggatagctactttcacaactatgcgaaactgaccaaggaagaggcgatcaaaaccgcgatgaccatttggaaggagatgaactggctgaacctgaagcaaaacattctgccgacccgtgaacgtgcgagcctgattctgaccaaaagcgcgaaccacgcggtggaggaagttcgtctgcgtaag

SEQ ID NO: 108 - protein, 316 aa, Artificial Sequence
  Pantothenate Kinase from Escherichia coli variant
MSIKEQTLMTPYLQFDRNQWAALRDLVPMTLSEDEIARLKGINEDLSLEEVAEIYLPLSRLLNFYISSNLRRQAVLEQFLGTNGQRIPYIISIAGSVAVGKSTTARVLQALLSRWPEHRRVELITTDGFLHPNQVLKERGLMKKKGFPESYDMHRLVKFVSDLKSGVPNVTAPVYSHLIYDVIPDGDKTVVQPDILILEGLNVLQSGMDYPHDPHHVFVSDFVDFSIYVDAPEDLLQTWYINRFLKFREGAFTDPDSYFHNYAKLTKEEAIKTAMTIWKEMNWLNLKQNILPTRERASLILTKSANHAVEEVRLRK

SEQ ID NO: 109 - DNA, 948 bp, Artificial Sequence
  Pantothenate Kinase from Escherichia coli variant
atgagcatcaaagagcagaccctgatgaccccgtacgatgaattcgaccgtaaccaatgggcggccctgcgtgatagcgttccgatgaccctgagcgaggacgaaatcgcgcgtctgaagggtattaacgaggatctgagcctggaggaagtggcggaaatctacctgccgctgagccgtctgctgaacttctatattagcagcaacctgcgtcgtcaggcggttctggaacaatttctgggtaccaacggccagcgtatcccgtatatcattagcattgcgggtagcgtggcggttggcaaaagcaccaccgcgcgtgtgctgcaggcgctgctgagccgttggccggagcaccgtcgtgttgaactgatcaccaccgacggcttcctgcacccgaaccaagtgctgaaggagcgtggtctgatgaagaaaaagggtttcccggaaagctacgatatgcaccgtctggtgaaatttgttagcgacctgaagagcggtgtgccgaacgttaccgcgccggtgtacagccacctgatctatgatgttattccggacggcgataaaaccgtggttcagccggacatcctgattctggagggtctgaacgtgctgcaaagcggcatggactatccgcacgatccgcaccacgtggaggttagcgacttcgtggattttagcatctacgttgacgcgccggaggatctgctgcagacctggtacattaaccgtttcctgaaaatgcgtgagggtgcgttcaccgacccggatagctactttcacaactatgcgaaactgaccaaggaagaggcgatcaaaaccgcgatgaccatttggaaggagatgaactggctgaacctgaagcaaaacattctgccgacccgtgaacgtgcgagcctgattctgaccaaaagcactaaccacgcggtggaggaagttcgtctgcgtaag

SEQ ID NO: 110 - protein, 316 aa, Artificial Sequence
  Pantothenate Kinase from Escherichia coli variant
MSIKEQTLMTPYDEFDRNQWAALRDSVPMTLSEDEIARLKGINEDLSLEEVAEIYLPLSRLLNFYISSNLRRQAVLEQFLGTNGQRIPYIISIAGSVAVGKSTTARVLQALLSRWPEHRRVELITTDGFLHPNQVLKERGLMKKKGFPESYDMHRLVKFVSDLKSGVPNVTAPVYSHLIYDVIPDGDKTVVQPDILILEGLNVLQSGMDYPHDPHHVEVSDFVDFSIYVDAPEDLLQTWYINRFLKMREGAFTDPDSYFHNYAKLTKEEAIKTAMTIWKEMNWLNLKQNILPTRERASLILTKSTNHAVEEVRLRK

SEQ ID NO: 111 - DNA, 948 bp, Artificial Sequence
  Pantothenate Kinase from Escherichia coli variant
atgagcatcaaagagcagaccctgatgaccccgtacctgcagctggaccgtaaccaatgggcggcgctgcgtgatagcgttccgatgaccctgagcgaggacgaaattgcgcgtctgaagggtattaacgaggatctgagcctggaggaagtggcggaaatctacctgccgctgagccgtctgctgaacttctatattagcagcaacctgcgtcgtcaggcggttctggaacaatttctgggtaccaacggccagcgtatcccgtatatcattagcattgcgggtagcgtggcggttggcaaaagcaccaccgcgcgtgtgctgcaggcgctgctgagccgttggccggagcaccgtcgtgttgaactgatcaccaccgacggcttcctgcacccgaaccaagtgctgaaggagcgtggtctgatgaagaaaaagggtttcccggaaagctacgatatgcaccgtctggtgaaatttgttagcgacctgaagagcggtgtgccgaacgttaccgcgccggtgtacagccacctgatctatgatgttattccggacggcgataaaaccgtggttcagccggacatcctgattctggagggtctgaacgtgctgcaaagcggcatggactatccgcacgatccgcaccacgtgtttgttagcgacttcgtggattttagcatctacgttgacgcgccggaggatctgctgcagacctggtacattaaccgtttcctgaaatttcgtgagggtgcgttcaccgacccggatagctactttcacaactatgcgaaactgaccaaggaagaggcgatcaaaaccgcgatgaccatttggaaggagatgaacctgctgaacctgaagcaaaacattctgccgacccgtgaacgtgcgagcctgattctgaccaaaagcgcgaaccacgcggtggaggaagttcgtctgcgtaag

SEQ ID NO: 112 - protein, 316 aa, Artificial Sequence
  Pantothenate Kinase from Escherichia coli variant
MSIKEQTLMTPYLQLDRNQWAALRDSVPMTLSEDEIARLKGINEDLSLEEVAEIYLPLSRLLNFYISSNLRRQAVLEQFLGTNGQRIPYIISIAGSVAVGKSTTARVLQALLSRWPEHRRVELITTDGFLHPNQVLKERGLMKKKGFPESYDMHRLVKFVSDLKSGVPNVTAPVYSHLIYDVIPDGDKTVVQPDILILEGLNVLQSGMDYPHDPHHVFVSDFVDFSIYVDAPEDLLQTWYINRFLKFREGAFTDPDSYFHNYAKLTKEEAIKTAMTIWKEMNLLNLKQNILPTRERASLILTKSANHAVEEVRLRK

SEQ ID NO: 113 - DNA, 948 bp, Artificial Sequence
  Pantothenate Kinase from Escherichia coli variant
atgagcatcaaagagcagaccctgatgaccccgtacctgcagttcgaccgtaaccagtgggcggctctgcgtgatccggttccgtcgaccctgagcgaggacgaaatcgcgcgtctgaagggtattaacgaggatctgagcctggaggaagtggcggaaatctacctgccgctgagccgtctgctgaacttctatattagcagcaacctgcgtcgtcaggcggttctggaacaatttctgggtaccaacggccagcgtatcccgtatatcattagcattgcgggtagcgtggcggttggcaaaagcaccaccgcgcgtgtgctgcaggcgctgctgagccgttggccggagcaccgtcgtgttgaactgatcaccaccgacggcttcctgcacccgaaccaagtgctgaaggagcgtggtctgatgaagaaaaagggtttcccggaaagctacgatatgcaccgtctggtgaaatttgttagcgacctgaagagcggtgtgccgaacgttaccgcgccggtgtacagccacctgatctatgatgttattccggacggcgataaaaccgtggttcagccggacatcctgattctggagggtctgaacgtgctgcaaagcggcatggactatccgcacgatccgcaccacgtgtttgttagcgacttcgtggattttagcatctacgttgacgcgccggaggatctgctgcagacctggtacattaaccgtttcctgaaatttcgtgagggtgcgttcaccgacccggatagctactttcacaactatgcgaaactgaccaaggaagaggcgatcaaaaccgcgatgaccatttggaaggagatgaactggctgaacctgaagcaaaacattctgccgacccgtgaacgtgcgagcctgattctgaccaaaagcgcgaaccacgcggtggaggaagttcgtctgcgtaag

SEQ ID NO: 114 - protein, 316 aa, Artificial Sequence
  Pantothenate Kinase from Escherichia coli variant
MSIKEQTLMTPYLQFDRNQWAALRDPVPSTLSEDEIARLKGINEDLSLEEVAEIYLPLSRLLNFYISSNLRRQAVLEQFLGTNGQRIPYIISIAGSVAVGKSTTARVLQALLSRWPEHRRVELITTDGFLHPNQVLKERGLMKKKGFPESYDMHRLVKFVSDLKSGVPNVTAPVYSHLIYDVIPDGDKTVVQPDILILEGLNVLQSGMDYPHDPHHVFVSDFVDFSIYVDAPEDLLQTWYINRFLKFREGAFTDPDSYFHNYAKLTKEEAIKTAMTIWKEMNWLNLKQNILPTRERASLILTKSANHAVEEVRLRK

SEQ ID NO: 115 - DNA, 948 bp, Artificial Sequence
  Pantothenate Kinase from Escherichia coli variant
atgagcatcaaagagcagaccctgatgaccccgtacgatcaattcgaccgtaaccaatgggcggccctgcgtgatagcgttccgatgaccctgagcgaggacgaaatcgcgcgtctgaagggtattaacgaggatctgagcctggaggaagtggcggaaatctacctgccgctgagccgtctgctgaacttctatattagcagcaacctgcgtcgtcaggcggttctggaacaatttctgggtaccaacggccagcgtatcccgtatatcattagcattgcgggtagcgtggcggttggcaaaagcaccaccgcgcgtgtgctgcaggcgctgctgagccgttggccggagcaccgtcgtgttgaactgatcaccaccgacggcttcctgcacccgaaccaagtgctgaaggagcgtggtctgatgaagaaaaagggtttcccggaaagctacgatatgcaccgtctggtgaaatttgttagcgacctgaagagcggtgtgccgaacgttaccgcgccggtgtacagccacctgatctatgatgttattccggacggcgataaaaccgtggttcagccggacatcctgattctggagggtctgaacgtgctgcaaagcggcatggactatccgcacgatccgcaccacgtgtttgttagcgacttcgtggattttagcatctacgttgacgcgccggaggatctgctgcagacctggtacattaaccgtttcctgaaatttcgtgagggtgcgttcaccgacccggatagctactttcacaactatgcgaaactgaccaaggaagaggcgatcaaaaccgcgatgaccatttggaaggagatgaactggctgaacctgaagcaaaacattctgccgacccgtgaacgtgcgagcctgattctgaccaaaagcgcgaaccacgcggtggaggaagttcgtctgcgtaag

SEQ ID NO: 116 - protein, 316 aa, Artificial Sequence
  Pantothenate Kinase from Escherichia coli variant
MSIKEQTLMTPYDQFDRNQWAALRDSVPMTLSEDEIARLKGINEDLSLEEVAEIYLPLSRLLNFYISSNLRRQAVLEQFLGTNGQRIPYIISIAGSVAVGKSTTARVLQALLSRWPEHRRVELITTDGFLHPNQVLKERGLMKKKGFPESYDMHRLVKFVSDLKSGVPNVTAPVYSHLIYDVIPDGDKTVVQPDILILEGLNVLQSGMDYPHDPHHVFVSDFVDFSIYVDAPEDLLQTWYINRFLKFREGAFTDPDSYFHNYAKLTKEEAIKTAMTIWKEMNWLNLKQNILPTRERASLILTKSANHAVEEVRLRK

SEQ ID NO: 117 - DNA, 948 bp, Artificial Sequence
  Pantothenate Kinase from Escherichia coli variant
atgagcatcaaagagcagaccctgatgaccccgtacctgcagttcgaccgtaaccaatgggcggcgctgagcgatagcgttccgatgacgctgagcgaggacgaaatcgcgcgtctgaagggtattaacgaggatctgagcctggaggaagtggcggaaatctacctgccgctgagccgtctgctgaacttctatattagcagcaacctgcgtcgtcaggcggaactggaacaatttctgggtaccaacggccagcatatcccgtatatcattagcattgcgggtagcgtggcggttggcaaaagcaccaccgcgcgtgtgctgcaggcgctgctgagccgttggccggagcaccgtcgtgttgaactgatcaccaccgacggcttcctgcacccgaacctggtgctgaaggagcgtggtctgatgaagaaaaagggtttcccggaaagctacgatatgcaccgtctggtgaaatttgttagcgacctgaagagcggtgtgccgaacgttaccgcgccggtgtacagccacctgatctatgatgttattccggacggcgataaaaccgtggttcagccggacatcctgattctggagggtctgaacgtgctgcaaagcggcatggactatccgcacgatccgcaccacgtgtttgttagcgacttcgtggattttagcatctacgttgacgcgccggaggatctgctgcagacctggtacattaaccgtttcctgaaatttcgtgagggtgcgttcaccgacccggatagctactttcacaactatgcgaaactgaccaaggaagaggcgatcaaaaccgcgatgaccatttggaaggagatgaactggctgaacctgaagcaaaacattctgccgacccgtgaacgtgcgagcctgattctgaccaaaagcgcgaaccacgcggtggaggaagttcgtctgcgtaag

SEQ ID NO: 118 - protein, 316 aa, Artificial Sequence
  Pantothenate Kinase from Escherichia coli variant
MSIKEQTLMTPYLQFDRNQWAALSDSVPMTLSEDEIARLKGINEDLSLEEVAEIYLPLSRLLNFYISSNLRRQAELEQFLGTNGQHIPYIISIAGSVAVGKSTTARVLQALLSRWPEHRRVELITTDGFLHPNLVLKERGLMKKKGFPESYDMHRLVKFVSDLKSGVPNVTAPVYSHLIYDVIPDGDKTVVQPDILILEGLNVLQSGMDYPHDPHHVFVSDFVDFSIYVDAPEDLLQTWYINRFLKFREGAFTDPDSYFHNYAKLTKEEAIKTAMTIWKEMNWLNLKQNILPTRERASLILTKSANHAVEEVRLRK

SEQ ID NO: 119 - DNA, 948 bp, Artificial Sequence
  Pantothenate Kinase from Escherichia coli variant
atgagcatcaaagagcagaccctgatgaccccgtacctgcaattcgaccgtaaccaatgggcgggcctgcgtgatagcgttccgatgaccctgagcgaggacgaaatcgcgcgtctgaagggtattaacgaggatctgagcctggaggaagtggcggaaatctacctgccgctgagccgtctgctgaacttctatattagcagcaacctgcgtcgtcaggcggttctggaacaatttctgggtaccaacggccagcgtatcccgtatatcattagcattgcgggtagcgtggcggttggcaaaagcaccaccgcgcgtgtgctgcaggcgctgctgagccgttggccggagcaccgtcgtgttgaactgatcaccaccgacggcttcctgcacccgaaccaagtgctgaaggagcgtggtctgatgaagaaaaagggtttcccggaaagctacgatatgcaccgtctggtgaaatttgttagcgacctgaagagcggtgtgccgaacgttaccgcgccggtgtacagccacctgatctatgatgttattccggacggcgataaaaccgtggttcagccggacatcctgattctggagggtctgaacgtgctgcaaagcggcatggactatccgcacgatccgcaccacgtggaggttagcgacttcgtggattttagcatctacgttgacgccccggaggatctgctgcagacctggtacattaaccgtttcctgaaatttcgtgagggtgcgttcaccgacccggatagctactttcacaactatgcgaaactgaccaaggaagaggcgagtaaaaccgcgatgaccatttggaaggagatgaactggctgaacctgaagcaaaacattctgccgacccgtgaacgtgcgagcctgattctgaccaaaagcgcgaaccacgcggtggaggaagttcgtctgcgtaag

SEQ ID NO: 120 - protein, 316 aa, Artificial Sequence
  Pantothenate Kinase from Escherichia coli variant
MSIKEQTLMTPYLQFDRNQWAGLRDSVPMTLSEDEIARLKGINEDLSLEEVAEIYLPLSRLLNFYISSNLRRQAVLEQFLGTNGQRIPYIISIAGSVAVGKSTTARVLQALLSRWPEHRRVELITTDGFLHPNQVLKERGLMKKKGFPESYDMHRLVKFVSDLKSGVPNVTAPVYSHLIYDVIPDGDKTVVQPDILILEGLNVLQSGMDYPHDPHHVEVSDFVDFSIYVDAPEDLLQTWYINRFLKFREGAFTDPDSYFHNYAKLTKEEASKTAMTIWKEMNWLNLKQNILPTRERASLILTKSANHAVEEVRLRK

SEQ ID NO: 121 - DNA, 948 bp, Artificial Sequence
  Pantothenate Kinase from Escherichia coli variant
atgagcatcaaagagcagaccctgatgaccccgtacctgcagctggaccgtaaccaatgggcggcgctgcgtgatagtaacccgatgaccctgagcgaggacgaaatcgcgcgtctgaagggtattaacgaggatctgagcctggaggaagtggcggaaatctacctgccgctgagccgtctgctgaacttctatattagcagcaacctgcgtcgtcaggcggttctggaacagtttctgggtaccaacggccagcgtatcccgtatatcattagcattgcgggtagcgtggcggttggcaaaagcaccaccgcgcgtgtgctgcaggcgctgctgagccgttggccggagcatcctcgtgttgaactgatcaccaccgacggcttcctgcacccgaaccaagtgctgaaggagcgtggtctgatgaagaaaaagggtttcccggaaagctacgatatgcaccgtctgatgaaatttgttaaagacctgaagagcggtgtgccgaatgttaccgcgccggtgtacagccacctgatctatgatgttattccggacggcgataaaaccgtggttcagccggacatcctgattctggagggtctgaacgtgctgcaaagcggcatggactatccgcacgatccgcaccacgtgtttgttagcgacttcgtggattttagcatctacgttgacgcgccggaggatctgctgcagacctggtacattaaccgtttcctgaaatttcgtgagggtgcgttcaccgacccggatagctactttcacaattatgcgaaactgaccaaggaagaggcgatcaaaaccgcgatgaccatttggaaggagatgaaccacctgaacctgaagcaaaacattctgccgacccgtgaacgtgcgagcctgattctgaccaaaagcgcaaaccacgcggtggaggaagttcgtctgcgtaag

SEQ ID NO: 122 - protein, 316 aa, Artificial Sequence
  Pantothenate Kinase from Escherichia coli variant
MSIKEQTLMTPYLQLDRNQWAALRDSNPMTLSEDEIARLKGINEDLSLEEVAEIYLPLSRLLNFYISSNLRRQAVLEQFLGTNGQRIPYIISIAGSVAVGKSTTARVLQALLSRWPEHPRVELITTDGFLHPNQVLKERGLMKKKGFPESYDMHRLMKFVKDLKSGVPNVTAPVYSHLIYDVIPDGDKTVVQPDILILEGLNVLQSGMDYPHDPHHVFVSDFVDFSIYVDAPEDLLQTWYINRFLKFREGAFTDPDSYFHNYAKLTKEEAIKTAMTIWKEMNHLNLKQNILPTRERASLILTKSANHAVEEVRLRK

SEQ ID NO: 123 - DNA, 948 bp, Artificial Sequence
  Pantothenate Kinase from Escherichia coli variant
atgagcatcaaagagcagaccctgatgaccccgtacctgcagctggaccgtaaccaatgggcggcgctgcgtgatagtaacccgatgaccctgagcgaggacgaaatcgcgcgtctgaagtgtattaacgaggatctgagcctggaggaagtggcggaaatctacctgccgctgagccgtctgctgaacttctatattagcagcaacctgcgtcgtcaggcggttctggaacagtttctgggtaccaacggccagcgtatcccgtatatcattagcattgcgggtagcgtggcggttggcaaaagcaccaccgcgcgtgtgctgcaggcgctgctgagccgttggccggagcatcctcgtgttgaactgatcaccaccgacggcttcctgcacccgaaccaagtgctgaaggagcgtggtctgatgaagaaaaagggtttcccggaaagctacgatatgcaccgtctggtgaaatttgttcgtgacctgaagagcggtgtgccgcaagttaccgcgccggtgtacagccacctgatctatgatgttattccggacggcgataaaaccgtggttcagccggacatcctgattctggagggtctgaacgtgctgcaaagcggcatggactatccgcacgatccgcaccacgtgtttgttagcgacttcgtggattttagcatctacgttgacgcgccggaggatctgctgcagacctggtacattaaccgtttcctgaaatttcgtgagggtgcgttcaccgacccggatagctactttcacgggtatgcgaaactgaccaaggaagaggcgatcaaaaccgcgatgaccatttggaaggagatgaaccacctgaacctgaagcaaaacattctgccgacccgtgaacgtgcgagtctgattctgaccaaaagcgcaaaccacgttgtggaggaagttcgtctgcgtaag

SEQ ID NO: 124 - protein, 316 aa, Artificial Sequence
  Pantothenate Kinase from Escherichia coli variant
MSIKEQTLMTPYLQLDRNQWAALRDSNPMTLSEDEIARLKCINEDLSLEEVAEIYLPLSRLLNFYISSNLRRQAVLEQFLGTNGQRIPYIISIAGSVAVGKSTTARVLQALLSRWPEHPRVELITTDGFLHPNQVLKERGLMKKKGFPESYDMHRLVKFVRDLKSGVPQVTAPVYSHLIYDVIPDGDKTVVQPDILILEGLNVLQSGMDYPHDPHHVFVSDFVDFSIYVDAPEDLLQTWYINRFLKFREGAFTDPDSYFHGYAKLTKEEAIKTAMTIWKEMNHLNLKQNILPTRERASLILTKSANHVVEEVRLRK

SEQ ID NO: 125 - DNA, 948 bp, Artificial Sequence
  Pantothenate Kinase from Escherichia coli variant
atgagcatcaaagagcagaccctgatgaccccgtacctgcagctggaccgtaaccaatgggcggcgctgcgtgatagtaacccgatgaccctgagcgaggacgaaatcgcgcgtctgaagggtattaaccctgatctgagcctggaggaagtggcggaaatctacctgccgctgagccgtctgctgaacttctatattagcagcaacctgcgtcgtcaggcggttcaggaacagtttctgggtaccaacggccagcgtatcccgtatatcattagcattgcgggtagcgtggcggttggcaaaagcaccaccgcgcgtgtgctgcaggcgctgctgagccgttggccggagcatcctcgtgttgaactgatcaccaccgacggcttcctgcacccgaaccaagtgctgaaggagcgtggtctgatgaagaaaaagggtttcccggaaagctacgatatgcaccgtctgatgaaatttgttaaagacctgaagagcggtgtgccgaatgttaccgcgccggtgtacagccacctgatctatgatgttattccggacggcgataaaaccgtggttcagccggacatcctgattctggagggtctgaacgtgctgcaaagcggcatggactatccgcacgatccgcaccacgtgtttgttagcgacttcgtggattttagcatctacgttgacgcgccggaggatctgctgcagacctggtacattaaccgtttcctgaaatttcgtgagggtgcgttcaccgacccggatagctactttcacaactatgcgaaactgaccaaggaagaggcgatcaaaaccgcgatgaccatttggaaggagatgaaccacctgaacctgaagcaaaacattctgccgacccgtgaacgtgcgagcctgattctgaccaaaagcgcaaaccacgcggtggaggaagttcgtctgcgtaag

SEQ ID NO: 126 - protein, 316 aa, Artificial Sequence
  Pantothenate Kinase from Escherichia coli variant
MSIKEQTLMTPYLQLDRNQWAALRDSNPMTLSEDEIARLKGINPDLSLEEVAEIYLPLSRLLNFYISSNLRRQAVQEQFLGTNGQRIPYIISIAGSVAVGKSTTARVLQALLSRWPEHPRVELITTDGFLHPNQVLKERGLMKKKGFPESYDMHRLMKFVKDLKSGVPNVTAPVYSHLIYDVIPDGDKTVVQPDILILEGLNVLQSGMDYPHDPHHVFVSDFVDFSIYVDAPEDLLQTWYINRFLKFREGAFTDPDSYFHNYAKLTKEEAIKTAMTIWKEMNHLNLKQNILPTRERASLILTKSANHAVEEVRLRK

SEQ ID NO: 127 - DNA, 948 bp, Artificial Sequence
  Pantothenate Kinase from Escherichia coli variant
atgagcatcaaagagcagaccctgatgaccccgtacctgcagctggaccgtaaccaatgggcggcgctgcgtgatagtaacccgatgaccctgagcgaggacgaaatcgcgcgtctgaagggtattaacgaggatctgagcctggaggaagtggcggaaatctacctgccgctgagccgtctgctgaacttctatattagcagcaacctgcgtcgtcaggcggttctggaacagtttctgggtaccaacggccagcgtatcccgtatatcattagcattgcgggtagcgtggcggttggcaaaagcaccaccgcgcgtgtgctgcaggcgctgctgagccgttggccggagcatcctcgtgttgaactgatcaccaccgacggcttcctgcacccgaaccaagtgctgaaggagcgtggtctgatgaagaaaaagggtttcccggaaagctacgatatgcaccgtctggtgaaatttgttagcgacctgaagagcggtgtgccgaatgttaccgcgccggtgtacagccacctgatctatgatgttattccggacggcgataaaaccgtggttcagccggacatcctgattctggagggtctgaacgtgctgcaaagcggcatggactatccgcacgatccgcaccacgtgtttgttagcgacttcgtggattttagcatctacgttgacgcgccggaggatctgctgcagacctggtacattaaccgtttcctgaaatttcgtgagggtgcgttcaccgacccggatagctactttcacgggtatgcgaaactgaccaaggaagaggcgatcaaaaccgcgatgaccatttggaaggagatgaaccacctgaacctgaagcaaaacattctgccgacccgtgaacgtgcgcgtctgattctgaccaaaagcgcaaaccacatcgtggaggaagttcgtctgcgtaag

SEQ ID NO: 128 - protein, 316 aa, Artificial Sequence
  Pantothenate Kinase from Escherichia coli variant
MSIKEQTLMTPYLQLDRNQWAALRDSNPMTLSEDEIARLKGINEDLSLEEVAEIYLPLSRLLNFYISSNLRRQAVLEQFLGTNGQRIPYIISIAGSVAVGKSTTARVLQALLSRWPEHPRVELITTDGFLHPNQVLKERGLMKKKGFPESYDMHRLVKFVSDLKSGVPNVTAPVYSHLIYDVIPDGDKTVVQPDILILEGLNVLQSGMDYPHDPHHVFVSDFVDFSIYVDAPEDLLQTWYINRFLKFREGAFTDPDSYFHGYAKLTKEEAIKTAMTIWKEMNHLNLKQNILPTRERARLILTKSANHIVEEVRLRK

SEQ ID NO: 129 - DNA, 948 bp, Artificial Sequence
  Pantothenate Kinase from Escherichia coli variant
atgagcatcaaagagcagaccctgatgaccccgtacctgcagctggaccgtaaccaatgggcggcgctgcgtgatagtaacccgatgaccctgagcgaggacgaaatcgcgcgtctgaagtgtattaacgaggatctgagcctggaggaagtggcggaatggtacctgccgctgagccgtctgctgaacttctatattagcagcaacctgcgtcgtcaggcggttctggaacagtttctgggtaccaacggccagcgtatcccgtatatcattagcattgcgggtagcgtggcggttggcaaaagcaccaccgcgcgtgtgctgcaggcgctgctgagccgttggccggagcatcctcgtgttgaactgatcaccaccgacggcttcctgcacccgaaccaagtgctgaaggagcgtggtctgatgaagaaaaagggtttcccggaaagctacgatatgcaccgtctgatgaaatttgttagtgacctgaagagcggtgtgccgcaagttaccgcgccggtgtacagccacctgatctatgatgttattccggacggcgataaaaccgtggttcagccggacatcctgattctggagggtctgaacgtgctgcaaagcggcatggactatccgcacgatccgcaccacgtgtttgttagcgacttcgtggattttagcatctacgttgacgcgccggaggatctgctgcagacctggtacattaaccgtttcctgaaatttcgtgagggtgcgttcaccgacccggatagctactttcacgggtatgcgaaactgaccaaggaagaggcgatcaaaaccgcgatgaccatttggaaggagatgaaccacctgaacctgaagcaaaacattctgccgacccgtgaacgtgcgagcctgattctgaccaaaagcgcaaaccacgcggtggaggaagttcgtctgcgtaag

SEQ ID NO: 130 - protein, 316 aa, Artificial Sequence
  Pantothenate Kinase from Escherichia coli variant
MSIKEQTLMTPYLQLDRNQWAALRDSNPMTLSEDEIARLKCINEDLSLEEVAEWYLPLSRLLNFYISSNLRRQAVLEQFLGTNGQRIPYIISIAGSVAVGKSTTARVLQALLSRWPEHPRVELITTDGFLHPNQVLKERGLMKKKGFPESYDMHRLMKFVSDLKSGVPQVTAPVYSHLIYDVIPDGDKTVVQPDILILEGLNVLQSGMDYPHDPHHVFVSDFVDFSIYVDAPEDLLQTWYINRFLKFREGAFTDPDSYFHGYAKLTKEEAIKTAMTIWKEMNHLNLKQNILPTRERASLILTKSANHAVEEVRLRK

SEQ ID NO: 131 - DNA, 948 bp, Artificial Sequence
  Pantothenate Kinase from Escherichia coli variant
atgagcatcaaagagcagaccctgatgaccccgtacctgcagctggaccgtaaccaatgggcggcgctgcgtgatagtaacccgatgaccctgagcgaggacgaaatcgcgcgtctgaagggtattaacgaggatctgagcctggaggaagtggcggaagtctacctgccgctgagccgtctgctgaacttctatattagcagcaacctgcgtcgtcaggcggttctggaacagtttctgggtaccaacggccagcgtatcccgtatatcattagcattgcgggtagcgtggcggttggcaaaagcaccaccgcgcgtgtgctgcaggcgctgctgagccgttggccggagcatcgtcgtgttgaactgatcaccaccgacggcttcctgcacccgaaccaagtgctgaaggagcgtggtctgatgaagaaaaagggtttcccggaaagctacgatatgcaccgtctgatgaaatttgttaaagacctgaagagcggtgtgccgaacgttaccgcgccggtgtacagccacctgatctatgatgttattccggacggcgataaaaccgtggttcagccggacatcctgattctggagggtctgaacgtgctgcaaagcggcatggactatccgcacgatccgcaccacgtgtttgttagcgacttcgtggattttagcatctacgttgacgcgccggaggatctgctgcagacctggtacattaaccgtttcctgaaatttcgtgagggtgcgttcaccgacccggatagctactttcacgggtatgcgaaactgaccaaggaagaggcgatcaaaaccgcgatgaccatttggaaggagatgaaccacctgaacctgaagcaaaacattctgccgacccgtgaacgtgcgagcctgattctgaccaaaagcgcaaaccacatcgtggaggaagttcgtctgcgtaag

SEQ ID NO: 132 - protein, 316 aa, Artificial Sequence
  Pantothenate Kinase from Escherichia coli variant
MSIKEQTLMTPYLQLDRNQWAALRDSNPMTLSEDEIARLKGINEDLSLEEVAEVYLPLSRLLNFYISSNLRRQAVLEQFLGTNGQRIPYIISIAGSVAVGKSTTARVLQALLSRWPEHRRVELITTDGFLHPNQVLKERGLMKKKGFPESYDMHRLMKFVKDLKSGVPNVTAPVYSHLIYDVIPDGDKTVVQPDILILEGLNVLQSGMDYPHDPHHVFVSDFVDFSIYVDAPEDLLQTWYINRFLKFREGAFTDPDSYFHGYAKLTKEEAIKTAMTIWKEMNHLNLKQNILPTRERASLILTKSANHIVEEVRLRK

SEQ ID NO: 133 - DNA, 948 bp, Artificial Sequence
  Pantothenate Kinase from Escherichia coli variant
atgagcatcaaagagcagaccctgatgaccccgtacctgcaactggaccgtaacgcgtgggcggggctgcgtgatagtaacccgatgaccctgagcgaggacgaaatcgcgcgtctgaagggtattaacgaggatctgagcctggaggaagtggcggaagtctacctgccgctgagccgtctgctgaacttctatattagcagcaacctgcgtcgtcaggcggttctggaacagtttctgggtaccaacggccagcgtatcccgtatatcattagcattgcgggtagcgtggcggttggcaaaagcaccaccgcgcgtgtgctgcaggcgctgctgagccgttggccggagcatcgtcgtgttgaactgatcaccaccgacggcttcctgcacccgaaccaagtgctgaaggagcgtggtctgatgaagaaaaagggtttcccggaaagctacgatatgcaccgtctgatgaaatttgttagtgacctgaagagcggtgtgccgcaagttaccgcgccggtgtacagccacctgatctatgatgttattccggacggcgataaaaccgtggttcagccggacatcctgattctggagggtctgaacgtgctgcaaagcggcatggactatccgcacgatccgcaccacgtgtttgttagcgacttcgtggattttagcatctacgttgacgcgccggaggatctgctgcagacctggtacattaaccgtttcctgaaatttcgtgagggtgcgttcaccgacccggatagctactttcacaactatgcgaaactgaccaaggaagaggcgatcaaaaccgcgatgaccatttggaaggagatgaaccacctgaacctgaagcaaaacattctgccgacccgtgaacgtgcgagcctgattctgaccaaaagcgcaaaccacgctgtggaggaagttcgtctgcgtaag

SEQ ID NO: 134 - protein, 316 aa, Artificial Sequence
  Pantothenate Kinase from Escherichia coli variant
MSIKEQTLMTPYLQLDRNAWAGLRDSNPMTLSEDEIARLKGINEDLSLEEVAEVYLPLSRLLNFYISSNLRRQAVLEQFLGTNGQRIPYIISIAGSVAVGKSTTARVLQALLSRWPEHRRVELITTDGFLHPNQVLKERGLMKKKGFPESYDMHRLMKFVSDLKSGVPQVTAPVYSHLIYDVIPDGDKTVVQPDILILEGLNVLQSGMDYPHDPHHVFVSDFVDFSIYVDAPEDLLQTWYINRFLKFREGAFTDPDSYFHNYAKLTKEEAIKTAMTIWKEMNHLNLKQNILPTRERASLILTKSANHAVEEVRLRK

SEQ ID NO: 135 - DNA, 948 bp, Artificial Sequence
  Pantothenate Kinase from Escherichia coli variant
atgagcatcaaagagcagaccctgatgaccccgtacctgcagctggaccgtaaccaatgggcggcgctgcgtgatagtaacccgatgaccctgagcgaggacgaaatcgcgcgtctgaagggtattaaccctgatctgagcctggaggaagtggcggaagtctacctgccgctgagccgtctgctgaacttctatattagcagcaacctgcgtcgtcaggcggttctggaacagtttctgggtaccaacggccagcgtatcccgtatatcattagcattgcgggtagcgtggcggttggcaaaagcaccaccgcgcgtgtgctgcaggcgctgctgagccgttggccggagcatcctcgtgttgaactgatcaccaccgacggcttcctgcacccgaaccaagtgctgaaggagcgtggtctgatgaagaaaaagggtttcccggaaagctacgatatgcaccgtctgatgaaatttgttcgtgacctgaagagcggtgtgccgaatgttaccgcgccggtgtacagccacctgatctatgatgttattccggacggcgataaaaccgtggttcagccggacatcctgattctggagggtctgaacgtgctgcaaagcggcatggactatccgcacgatccgcaccacgtgtttgttagcgacttcgtggattttagcatctacgttgacgcgccggaggatctgctgcagacctggtacattaaccgtttcctgaaatttcgtgagggtgcgttcaccgacccggatagctactttcacccgtatgcgaaactgaccaaggaagaggcgatcaaaaccgcgatgaccatttggaaggagatgaaccacctgaacctgaagcaaaacattctgccgacccgtgaacgtgcgcgtctgattctgaccaaaagcgcaaaccacgctgtggaggaagttcgtctgcgtaag

SEQ ID NO: 136 - protein, 316 aa, Artificial Sequence
  Pantothenate Kinase from Escherichia coli variant
MSIKEQTLMTPYLQLDRNQWAALRDSNPMTLSEDEIARLKGINPDLSLEEVAEVYLPLSRLLNFYISSNLRRQAVLEQFLGTNGQRIPYIISIAGSVAVGKSTTARVLQALLSRWPEHPRVELITTDGFLHPNQVLKERGLMKKKGFPESYDMHRLMKFVRDLKSGVPNVTAPVYSHLIYDVIPDGDKTVVQPDILILEGLNVLQSGMDYPHDPHHVFVSDFVDFSIYVDAPEDLLQTWYINRFLKFREGAFTDPDSYFHPYAKLTKEEAIKTAMTIWKEMNHLNLKQNILPTRERARLILTKSANHAVEEVRLRK

SEQ ID NO: 137 - DNA, 948 bp, Artificial Sequence
  Pantothenate Kinase from Escherichia coli variant
atgagcatcaaagagcagaccctgatgaccccgtacctgcagctggaccgtaaccaatgggcggcgctgcgtgatagtaacccgatgaccctgagcgaggacgaaatcgcgcgtctgaagcggattaacgaggatctgagcctggaggaagtggcggaaatctacctgccgctgagccgtctgctgaacttctatattagcagcaacctgcgtcgtcaggcggttctggaacagtttctgggtaccaacggccagcgtatcccgtatatcattagcattgcgggtagcgtggcggttggcaaaagcaccaccgcgcgtgtgctgcaggcgctgctgagccgttggccggagcatcgtcgtgttgaactgatcaccaccgacggcttcctgcacccgaaccaagtgctgaaggagcgtggtctgatgaagaaaaagggtttcccggaaagctacgatatgcaccgtctggtgaaatttgttagcgacctgaagagcggtgtgccgaacgttaccgcgccggtgtacagccacctgatctatgatgttattccggacggcgataaaaccgtggttcagccggacatcctgattctggagggtctgaacgtgctgcaaagcggcatggactatccgcacgatccgcaccacgtgtttgttagcgacttcgtggattttagcatctacgttgacgcgccggaggatctgctgcagacctggtacattaaccgtttcctgaaatttcgtgagggtgcgttcaccgacccggatagctactttcacaactatgcgaaactgaccaaggaagaggcgatcaaaaccgcgatgaccatttggaaggagatgaaccacctgaacctgaagcaaaacattctgccgacccgtgaacgtgcgagcctgattctgaccaaaagcgcaaaccacgcggtggaggaagttcgtctgcgtaag

SEQ ID NO: 138 - protein, 316 aa, Artificial Sequence
  Pantothenate Kinase from Escherichia coli variant
MSIKEQTLMTPYLQLDRNQWAALRDSNPMTLSEDEIARLKRINEDLSLEEVAEIYLPLSRLLNFYISSNLRRQAVLEQFLGTNGQRIPYIISIAGSVAVGKSTTARVLQALLSRWPEHRRVELITTDGFLHPNQVLKERGLMKKKGFPESYDMHRLVKFVSDLKSGVPNVTAPVYSHLIYDVIPDGDKTVVQPDILILEGLNVLQSGMDYPHDPHHVFVSDFVDFSIYVDAPEDLLQTWYINRFLKFREGAFTDPDSYFHNYAKLTKEEAIKTAMTIWKEMNHLNLKQNILPTRERASLILTKSANHAVEEVRLRK

SEQ ID NO: 139 - DNA, 948 bp, Artificial Sequence
  Pantothenate Kinase from Escherichia coli variant
atgagcatcaaagagcagaccctgatgaccccgtacctgcagctggaccgtaaccaatgggcggcgctgcgtgatagtaacccgatgaccctgagcgaggacgaaatcgcgcgtctgaagtgtattaaccaggatctgagcctggaggaagtggcggaaatctacctgccgctgagccgtctgctgaacttctatattagcagcaacctgcgtcgtcaggcggttctggaacagtttctgggtaccaacggccagcgtatcccgtatatcattagcattgcgggtagcgtggcggttggcaaaagcaccaccgcgcgtgtgctgcaggcgctgctgagccgttggccggagcaccgtcgtgttgaactgatcaccaccgacggcttcctgcacccgaaccaagtgctgaaggagcgtggtctgatgaagaaaaagggtttcccggaaagctacgatatgcaccgtctggtgaaatttgttagtgacctgaagagcggtgtgccgcaagttaccgcgccggtgtacagccacctgatctatgatgttattccggacggcgataaaaccgtggttcagccggacatcctgattctggagggtctgaacgtgctgcaaagcggcatggactatccgcacgatccgcaccacgtgtttgttagcgacttcgtggattttagcatctacgttgacgcgccggaggatctgctgcagacctggtacattaaccgtttcctgaaatttcgtgagggtgcgttcaccgacccggatagctactttcacccgtatgcgaaactgaccaaggaagaggcgatcaaaaccgcgatgaccatttggaaggagatgaaccacctgaacctgaagcaaaacattctgccgacccgtgaacgtgcgcgtctgattctgaccaaaagcgcaaaccacgttgtggaggaagttcgtctgcgtaag

SEQ ID NO: 140 - protein, 316 aa, Artificial Sequence
  Pantothenate Kinase from Escherichia coli variant
MSIKEQTLMTPYLQLDRNQWAALRDSNPMTLSEDEIARLKCINQDLSLEEVAEIYLPLSRLLNFYISSNLRRQAVLEQFLGTNGQRIPYIISIAGSVAVGKSTTARVLQALLSRWPEHRRVELITTDGFLHPNQVLKERGLMKKKGFPESYDMHRLVKFVSDLKSGVPQVTAPVYSHLIYDVIPDGDKTVVQPDILILEGLNVLQSGMDYPHDPHHVFVSDFVDFSIYVDAPEDLLQTWYINRFLKFREGAFTDPDSYFHPYAKLTKEEAIKTAMTIWKEMNHLNLKQNILPTRERARLILTKSANHVVEEVRLRK

SEQ ID NO: 141 - DNA, 948 bp, Artificial Sequence
  Pantothenate Kinase from Escherichia coli variant
atgagcatcaaagagcagaccctgatgaccccgtacctgcagctggaccgtaaccaatgggcggcgctgcgtgatagtaacccgatgaccctgagcgaggacgaaatcgcgcgtctgaagggtattaacgaggatctgagcctggaggaagtggcggaaatctacctgccgctgagccgtctgctgaacttctatattagcagcaacctgcgtcgtcaggcggttctggaacagtttctgggtaccaacggccagcgtatcccgtatatcattagcattgcgggtagcgtggcggttggcaaaagcaccaccgcgcgtgtgctgcaggcgctgctgagccgttggccggagcaccgtcgtgttgaactgatcaccaccgacggcttcctgcacccgaaccaagtgctgaaggagcgtggtctgatgaagaaaaagggtttcccggaaagctacgatatgcaccgtctgatgaaatttgttagtgacctgaagagcggtgtgccgaatgttaccgcgccggtgtacagccacctgatctatgatgttattccggacggcgataaaaccgtggttcagccggacatcctgattctggagggtctgaacgtgctgcaaagcggcatggactatccgcacgatccgcaccacgtgtttgttagcgacttcgtggattttagcatctacgttgacgcgccggaggatctgctgcagacctggtacattaaccgtttcctgaaatttcgtgagggtgcgttcaccgacccggatagctactttcacaattatgcgaaactgaccaaggaagaggcgatcaaaaccgcgatgaccatttggaaggagatgaaccacctgaacctgaagcaaaacattctgccgacccgtgaacgtgcgagcctgattctgaccaaaagcgcaaaccacgcggtggaggaagttcgtctgcgtaag

SEQ ID NO: 142 - protein, 316 aa, Artificial Sequence
  Pantothenate Kinase from Escherichia coli variant
MSIKEQTLMTPYLQLDRNQWAALRDSNPMTLSEDEIARLKGINEDLSLEEVAEIYLPLSRLLNFYISSNLRRQAVLEQFLGTNGQRIPYIISIAGSVAVGKSTTARVLQALLSRWPEHRRVELITTDGFLHPNQVLKERGLMKKKGFPESYDMHRLMKFVSDLKSGVPNVTAPVYSHLIYDVIPDGDKTVVQPDILILEGLNVLQSGMDYPHDPHHVFVSDFVDFSIYVDAPEDLLQTWYINRFLKFREGAFTDPDSYFHNYAKLTKEEAIKTAMTIWKEMNHLNLKQNILPTRERASLILTKSANHAVEEVRLRK

SEQ ID NO: 143 - DNA, 948 bp, Artificial Sequence
  Pantothenate Kinase from Escherichia coli variant
atgagcatcaaagagcagaccctgatgaccccgtacctgcagctggaccgtaaccaatgggcggcgctgcgtgatagtaacccgatgaccctgagcgaggacgaaatcgcgcgtctgaagtgtattaaccaggatctgagcctggaggaagtggcggaagtctacctgccgctgagccgtctgctgaacttctatattagcagcaacctgcgtcgtcaggcggttctggaacagtttctgggtaccaacggccagcgtatcccgtatatcattagcattgcgggtagcgtggcggttggcaaaagcaccaccgcgcgtgtgctgcaggcgctgctgagccgttggccggagcatcctaaggttgaactgatcaccaccgacggcttcctgcacccgaaccaagtgctgaaggagcgtggtctgatgaagaaaaagggtttcccggaaagctacgatatgcaccgtctgatgaaatttgttagtgacctgaagagcggtgtgccgaatgttaccgcgccggtgtacagccacctgatctatgatgttattccggacggcgataaaaccgtggttcagccggacatcctgattctggagggtctgaacgtgctgcaaagcggcatggactatccgcacgatccgcaccacgtgtttgttagcgacttcgtggattttagcatctacgttgacgcgccggaggatctgctgcagacctggtacattaaccgtttcctgaaatttcgtgagggtgcgttcaccgacccggatagctactttcacgggtatgcgaaactgaccaaggaagaggcgatcaaaaccgcgatgaccatttggaaggagatgaaccacctgaacctgaagcaaaacattctgccgacccgtgaacgtgcgcgtctgattctgaccaaaagcgcaaaccacgttgtggaggaagttcgtctgcgtaag

SEQ ID NO: 144 - protein, 316 aa, Artificial Sequence
  Pantothenate Kinase from Escherichia coli variant
MSIKEQTLMTPYLQLDRNQWAALRDSNPMTLSEDEIARLKCINQDLSLEEVAEVYLPLSRLLNFYISSNLRRQAVLEQFLGTNGQRIPYIISIAGSVAVGKSTTARVLQALLSRWPEHPKVELITTDGFLHPNQVLKERGLMKKKGFPESYDMHRLMKFVSDLKSGVPNVTAPVYSHLIYDVIPDGDKTVVQPDILILEGLNVLQSGMDYPHDPHHVFVSDFVDFSIYVDAPEDLLQTWYINRFLKFREGAFTDPDSYFHGYAKLTKEEAIKTAMTIWKEMNHLNLKQNILPTRERARLILTKSANHVVEEVRLRK

SEQ ID NO: 145 - DNA, 948 bp, Artificial Sequence
  Pantothenate Kinase from Escherichia coli variant
atgagcatcaaagagcagaccctgatgaccccgtacctgcagctggaccgtaaccaatgggcggcgctgcgtgatagtaacccgatgaccctgagcgaggacgaaatcgcgcgtctgaagggtattaaccaggatctgagcctggaggaagtggcggaatggtacctgccgctgagccgtctgctgaacttctatattagcagcaacctgcgtcgtcaggcggttctggaacagtttctgggtaccaacggccagcgtatcccgtatatcattagcattgcgggtagcgtggcggttggcaaaagcaccaccgcgcgtgtgctgcaggcgctgctgagccgttggccggagcatcctcgtgttgaactgatcaccaccgacggcttcctgcacccgaaccaagtgctgaaggagcgtggtctgatgaagaaaaagggtttcccggaaagctacgatatgcaccgtctggtgaaatttgttagtgacctgaagagcggtgtgccgcaagttaccgcgccggtgtacagccacctgatctatgatgttattccggacggcgataaaaccgtggttcagccggacatcctgattctggagggtctgaacgtgctgcaaagcggcatggactatccgcacgatccgcaccacgtgtttgttagcgacttcgtggattttagcatctacgttgacgcgccggaggatctgctgcagacctggtacattaaccgtttcctgaaatttcgtgagggtgcgttcaccgacccggatagctactttcacaactatgcgaaactgaccaaggaagaggcgatcaaaaccgcgatgaccatttggaaggagatgaaccacctgaacctgaagcaaaacattctgccgacccgtgaacgtgcgagcctgattctgaccaaaagcgcaaaccacgcggtggaggaagttcgtctgcgtaag

SEQ ID NO: 146 - protein, 316 aa, Artificial Sequence
  Pantothenate Kinase from Escherichia coli variant
MSIKEQTLMTPYLQLDRNQWAALRDSNPMTLSEDEIARLKGINQDLSLEEVAEWYLPLSRLLNFYISSNLRRQAVLEQFLGTNGQRIPYIISIAGSVAVGKSTTARVLQALLSRWPEHPRVELITTDGFLHPNQVLKERGLMKKKGFPESYDMHRLVKFVSDLKSGVPQVTAPVYSHLIYDVIPDGDKTVVQPDILILEGLNVLQSGMDYPHDPHHVFVSDFVDFSIYVDAPEDLLQTWYINRFLKFREGAFTDPDSYFHNYAKLTKEEAIKTAMTIWKEMNHLNLKQNILPTRERASLILTKSANHAVEEVRLRK

SEQ ID NO: 147 - DNA, 948 bp, Artificial Sequence
  Pantothenate Kinase from Escherichia coli variant
atgagcatcaaagagcagaccctgatgaccccgtacctgcagctggaccgtaaccaatgggcggcgctgcgtgatagtaacccgatgaccctgagcgaggacgaaatcgcgcgtctgaagggtattaacgaggatctgagcctggaggaagtggcggaatggtacctgccgctgagccgtctgctgaacttctatattagcagcaacctgcgtcgtcaggcggttctggaacagtttctgggtaccaacggccagcgtatcccgtatatcattagcattgcgggtagcgtggcggttggcaaaagcaccaccgcgcgtgtgctgcaggcgctgctgagccgttggccggagcatgcccgtgttgaactgatcaccaccgacggcttcctgcacccgaaccaagtgctgaaggagcgtggtctgatgaagaaaaagggtttcccggaaagctacgatatgcaccgtctgatgaaatttgttaaagacctgaagagcggtgtgccgcaagttaccgcgccggtgtacagccacctgatctatgatgttattccggacggcgataaaaccgtggttcagccggacatcctgattctggagggtctgaacgtgctgcaaagcggcatggactatccgcacgatccgcaccacgtgtttgttagcgacttcgtggattttagcatctacgttgacgcgccggaggatctgctgcagacctggtacattaaccgtttcctgaaatttcgtgagggtgcgttcaccgacccggatagctactttcacaactatgcgaaactgaccaaggaagaggcgatcaaaaccgcgatgaccatttggaaggagatgaaccacctgaacctgaagcaaaacattctgccgacccgtgaacgtgcgagcctgattctgaccaaaagcgcaaaccacgcggtggaggaagttcgtctgcgtaag

SEQ ID NO: 148 - protein, 316 aa, Artificial Sequence
  Pantothenate Kinase from Escherichia coli variant
MSIKEQTLMTPYLQLDRNQWAALRDSNPMTLSEDEIARLKGINEDLSLEEVAEWYLPLSRLLNFYISSNLRRQAVLEQFLGTNGQRIPYIISIAGSVAVGKSTTARVLQALLSRWPEHARVELITTDGFLHPNQVLKERGLMKKKGFPESYDMHRLMKFVKDLKSGVPQVTAPVYSHLIYDVIPDGDKTVVQPDILILEGLNVLQSGMDYPHDPHHVFVSDFVDFSIYVDAPEDLLQTWYINRFLKFREGAFTDPDSYFHNYAKLTKEEAIKTAMTIWKEMNHLNLKQNILPTRERASLILTKSANHAVEEVRLRK

SEQ ID NO: 149 - DNA, 948 bp, Artificial Sequence
  Pantothenate Kinase from Escherichia coli variant
atgagcatcaaagagcagaccctgatgaccccgtacctgcagctggaccgtaaccaatgggcggcgctgcgtgatagtaacccgatgaccctgagcgaggacgaaatcgcgcgtctgaagggtattaacgaggatctgagcctggaggaagtggcggaaatctacctgccgctgagccgtctgctgaacttctatattagcagcaacctgcgtcgtcaggcggttctggaacagtttctgggtaccaacggccagcgtatcccgtatatcattagcattgcgggtagcgtggcggttggcaaaagcaccaccgcgcgtgtgctgcaggcgctgctgagccgttggccggagcaccgtcgtgttgaactgatcaccaccgacggcttcctgcacccgaaccaagtgctgaaggagcgtggtctgatgaagaaaaagggtttcccggaaagctacgatatgcaccgtctgatgaaatttgttagtgacctgaagagcggtgtgccgaacgttaccgcgccggtgtacagccacctgatctatgatgttattccggacggcgataaaaccgtggttcagccggacatcctgattctggagggtctgaacgtgctgcaaagcggcatggactatccgcacgatccgcaccacgtgtttgttagcgacttcgtggattttagcatctacgttgacgcgccggaggatctgctgcagacctggtacattaaccgtttcctgaaatttcgtgagggtgcgttcaccgacccggatagctactttcacaactatgcgaaactgaccaaggaagaggcgatcaaaaccgcgatgaccatttggaaggagatgaaccacctgaacctgaagcaaaacattctgccgacccgtgaacgtgcgagcctgattctgaccaaaagcgcaaaccacgttgtggaggaagttcgtctgcgtaag

SEQ ID NO: 150 - protein, 316 aa, Artificial Sequence
  Pantothenate Kinase from Escherichia coli variant
MSIKEQTLMTPYLQLDRNQWAALRDSNPMTLSEDEIARLKGINEDLSLEEVAEIYLPLSRLLNFYISSNLRRQAVLEQFLGTNGQRIPYIISIAGSVAVGKSTTARVLQALLSRWPEHRRVELITTDGFLHPNQVLKERGLMKKKGFPESYDMHRLMKFVSDLKSGVPNVTAPVYSHLIYDVIPDGDKTVVQPDILILEGLNVLQSGMDYPHDPHHVFVSDFVDFSIYVDAPEDLLQTWYINRFLKFREGAFTDPDSYFHNYAKLTKEEAIKTAMTIWKEMNHLNLKQNILPTRERASLILTKSANHVVEEVRLRK

SEQ ID NO: 151 - DNA, 948 bp, Artificial Sequence
  Pantothenate Kinase from Escherichia coli variant
atgagcatcaaagagcagaccctgatgaccccgtacctgcagctggaccgtaaccaatgggcggcgctgcgtgatagtaacccgatgaccctgagcgaggacgaaatcgcgcgtctgaagggtattaaccaggatctgagcctggaggaagtggcggaagtctacctgccgctgagccgtctgctgaacttctatattagcagcaacctgcgtcgtcaggcggttctggaacagtttctgggtaccaacggccagcgtatcccgtatatcattagcattgcgggtagcgtggcggttggcaaaagcaccaccgcgcgtgtgctgcaggcgctgctgagccgttggccggagcataaaaaggttgaactgatcaccaccgacggcttcctgcacccgaaccaagtgctgaaggagcgtggtctgatgaagaaaaagggtttcccggaaagctacgatatgcaccgtctgatgaaatttgttcgtgacctgaagagcggtgtgccgaatgttaccgcgccggtgtacagccacctgatctatgatgttattccggacggcgataaaaccgtggttcagccggacatcctgattctggagggtctgaacgtgctgcaaagcggcatggactatccgcacgatccgcaccacgtgtttgttagcgacttcgtggattttagcatctacgttgacgcgccggaggatctgctgcagacctggtacattaaccgtttcctgaaatttcgtgagggtgcgttcaccgacccggatagctactttcacgggtatgcgaaactgaccaaggaagaggcgatcaaaaccgcgatgaccatttggaaggagatgaaccacctgaacctgaagcaaaacattctgccgacccgtgaacgtgcgagcctgattctgaccaaaagcgcaaaccacgcggtggaggaagttcgtctgcgtaag

SEQ ID NO: 152 - protein, 316 aa, Artificial Sequence
  Pantothenate Kinase from Escherichia coli variant
MSIKEQTLMTPYLQLDRNQWAALRDSNPMTLSEDEIARLKGINQDLSLEEVAEVYLPLSRLLNFYISSNLRRQAVLEQFLGTNGQRIPYIISIAGSVAVGKSTTARVLQALLSRWPEHKKVELITTDGFLHPNQVLKERGLMKKKGFPESYDMHRLMKFVRDLKSGVPNVTAPVYSHLIYDVIPDGDKTVVQPDILILEGLNVLQSGMDYPHDPHHVFVSDFVDFSIYVDAPEDLLQTWYINRFLKFREGAFTDPDSYFHGYAKLTKEEAIKTAMTIWKEMNHLNLKQNILPTRERASLILTKSANHAVEEVRLRK

SEQ ID NO: 153 - DNA, 948 bp, Artificial Sequence
  Pantothenate Kinase from Escherichia coli variant
atgagcatcaaagagcagaccctgatgaccccgtacctgcagctggaccgtaaccaatgggcggcgctgcgtgatagtaacccgatgaccctgagcgaggacgaaatcgcgcgtctgaagggtattaaccaggatctgagcctggaggaagtggcggaaatctacctgccgctgagccgtctgctgaacttctatattagcagcaacctgcgtcgtcaggcggttctggaacagtttctgggtaccaacggccagcgtatcccgtatatcattagcattgcgggtagcgtggcggttggcaaaagcaccaccgcgcgtgtgctgcaggcgctgctgagccgttggccggagcatcctcgtgttgaactgatcaccaccgacggcttcctgcacccgaaccaagtgctgaaggagcgtggtctgatgaagaaaaagggtttcccggaaagctacgatatgcaccgtctggtgaaatttgttcgtgacctgaagagcggtgtgccgaatgttaccgcgccggtgtacagccacctgatctatgatgttattccggacggcgataaaaccgtggttcagccggacatcctgattctggagggtctgaacgtgctgcaaagcggcatggactatccgcacgatccgcaccacgtgtttgttagcgacttcgtggattttagcatctacgttgacgcgccggaggatctgctgcagacctggtacattaaccgtttcctgaaatttcgtgagggtgcgttcaccgacccggatagctactttcacccgtatgcgaaactgaccaaggaagaggcgatcaaaaccgcgatgaccatttggaaggagatgaaccacctgaacctgaagcaaaacattctgccgacccgtgaacgtgcgcgtctgattctgaccaaaagcgcaaaccacgcggtggaggaagttcgtctgcgtaag

SEQ ID NO: 154 - protein, 316 aa, Artificial Sequence
  Pantothenate Kinase from Escherichia coli variant
MSIKEQTLMTPYLQLDRNQWAALRDSNPMTLSEDEIARLKGINQDLSLEEVAEIYLPLSRLLNFYISSNLRRQAVLEQFLGTNGQRIPYIISIAGSVAVGKSTTARVLQALLSRWPEHPRVELITTDGFLHPNQVLKERGLMKKKGFPESYDMHRLVKFVRDLKSGVPNVTAPVYSHLIYDVIPDGDKTVVQPDILILEGLNVLQSGMDYPHDPHHVFVSDFVDFSIYVDAPEDLLQTWYINRFLKFREGAFTDPDSYFHPYAKLTKEEAIKTAMTIWKEMNHLNLKQNILPTRERARLILTKSANHAVEEVRLRK

SEQ ID NO: 155 - DNA, 948 bp, Artificial Sequence
  Pantothenate Kinase from Escherichia coli variant
atgagcatcaaagagcagaccctgatgaccccgtacctgcagctggaccgtaaccaatgggcggcgctgcgtgatagtaacccgatgaccctgagcgaggacgaaatcgcgcgtctgaagtgtattaaccaggatctgagcctggaggaagtggcggaagtctacctgccgctgagccgtctgctgaacttctatattagcagcaacctgcgtcgtcaggcggttctggaacagtttctgggtaccaacggccagcgtatcccgtatatcattagcattgcgggtagcgtggcggttggcaaaagcaccaccgcgcgtgtgctgcaggcgctgctgagccgttggccggagcatgccaaggttgaactgatcaccaccgacggcttcctgcacccgaaccaagtgctgaaggagcgtggtctgatgaagaaaaagggtttcccggaaagctacgatatgcaccgtctgatgaaatttgttagtgacctgaagagcggtgtgccgcaagttaccgcgccggtgtacagccacctgatctatgatgttattccggacggcgataaaaccgtggttcagccggacatcctgattctggagggtctgaacgtgctgcaaagcggcatggactatccgcacgatccgcaccacgtgtttgttagcgacttcgtggattttagcatctacgttgacgcgccggaggatctgctgcagacctggtacattaaccgtttcctgaaatttcgtgagggtgcgttcaccgacccggatagctactttcacccgtatgcgaaactgaccaaggaagaggcgatcaaaaccgcgatgaccatttggaaggagatgaaccacctgaacctgaagcaaaacattctgccgacccgtgaacgtgcgagcctgattctgaccaaaagcgcaaaccacgctgtggaggaagttcgtctgcgtaag

SEQ ID NO: 156 - protein, 316 aa, Artificial Sequence
  Pantothenate Kinase from Escherichia coli variant
MSIKEQTLMTPYLQLDRNQWAALRDSNPMTLSEDEIARLKCINQDLSLEEVAEVYLPLSRLLNFYISSNLRRQAVLEQFLGTNGQRIPYIISIAGSVAVGKSTTARVLQALLSRWPEHAKVELITTDGFLHPNQVLKERGLMKKKGFPESYDMHRLMKFVSDLKSGVPQVTAPVYSHLIYDVIPDGDKTVVQPDILILEGLNVLQSGMDYPHDPHHVFVSDFVDFSIYVDAPEDLLQTWYINRFLKFREGAFTDPDSYFHPYAKLTKEEAIKTAMTIWKEMNHLNLKQNILPTRERASLILTKSANHAVEEVRLRK

SEQ ID NO: 157 - DNA, 948 bp, Artificial Sequence
  Pantothenate Kinase from Escherichia coli variant
atgagcatcaaagagcagaccctgatgaccccgtacctggaactggaccgtaacacgtgggcggcgctgcgtgatagtaacccgatgaccctgagcgaggacgaaatcgcgcgtctgaagtgtattaacgaggatctgagcctggaggaagtggcggaaatctacctgccgctgagccgtctgctgaacttctatattagcagcaacctgcgtcgtcaggcggttctggaacagtttctgggtaccaacggccagcgtatcccgtatatcattagcattgcgggtagcgtggcggttggcaaaagcaccaccgcgcgtgtgctgcaggcgctgctgagccgttggccggagcatcgtcgtgttgaactgatcaccaccgacggcttcctgcacccgaaccaagtgctgaaggagcgtggtctgatgaagaaaaagggtttcccggaaagctacgatatgcaccgtctgatgaaatttgttaaagacctgaagagcggtgtgccgaatgttaccgcgccggtgtacagccacctgatctatgatgttattccggacggcgataaaaccgtggttcagccggacatcctgattctggagggtctgaacgtgctgcaaagcggcatggactatccgcacgatccgcaccacgtgtttgttagcgacttcgtggattttagcatctacgttgacgcgccggaggatctgctgcagacctggtacattaaccgtttcctgaaatttcgtgagggtgcgttcaccgacccggatagctactttcacccgtatgcgaaactgaccaaggaagaggcgatcaaaaccgcgatgaccatttggaaggagatgaaccacctgaacctgaagcaaaacattctgccgacccgtgaacgtgcgagcctgattctgaccaaaagcgcaaaccacgcggtggaggaagttcgtctgcgtaag

SEQ ID NO: 158 - protein, 316 aa, Artificial Sequence
  Pantothenate Kinase from Escherichia coli variant
MSIKEQTLMTPYLELDRNTWAALRDSNPMTLSEDEIARLKCINEDLSLEEVAEIYLPLSRLLNFYISSNLRRQAVLEQFLGTNGQRIPYIISIAGSVAVGKSTTARVLQALLSRWPEHRRVELITTDGFLHPNQVLKERGLMKKKGFPESYDMHRLMKFVKDLKSGVPNVTAPVYSHLIYDVIPDGDKTVVQPDILILEGLNVLQSGMDYPHDPHHVFVSDFVDFSIYVDAPEDLLQTWYINRFLKFREGAFTDPDSYFHPYAKLTKEEAIKTAMTIWKEMNHLNLKQNILPTRERASLILTKSANHAVEEVRLRK

SEQ ID NO: 159 - DNA, 948 bp, Artificial Sequence
  Pantothenate Kinase from Escherichia coli variant
atgagcatcaaagagcagaccctgatgaccccgtacctgcagctggaccgtaaccaatgggcggggctgcgtgatagtaacccgatgaccctgagcgaggacgaaatcgcgcgtctgaagggtattaacgaggatctgagcctggaggaagtggcggaaatctacctgccgctgagccgtctgctgaacttctatattagcagcaacctgcgtcgtcaggcggttctggaacagtttctgggtaccaacggccagcgtatcccgtatatcattagcattgcgggtagcgtggcggttggcaaaagcaccaccgcggctgtgctgcaggcgctgctgagccgttggccggagcatcgtcgtgttgaactgatcaccaccgacggcttcctgcacccgaaccaagtgctgaaggagcgtggtctgatgaagaaaaagggtttcccggaaagctacgatatgcaccgtctggtgaaatttgttagcgacctgaagagcggtgtgccgaacgttaccgcgccggtgtacagccacctgatctatgatgttattccggacggcgataaaaccgtggttcagccggacatcctgattctggagggtctgaacgtgctgcaaagcggcatggactatccgcacgatccgcaccacgtggaagttagcgacttcgtggattttagcatctacgttgacgcgccggaggatctgctgcagacctggtacattaaccgtttcctgaaatttcgtgagggtgcgttcaccgacccggatagctactttcacaactatgcgaaactgaccaaggaagaggcgatcaaaaccgcgatgaccatctggaaggagatgaaccacctgaacctgaagcaaaacattctgccgacccgtgaacgtgcgagcctgattctgaccaaaagcgcaaaccacgcggtggaggaagttcgtctgcgtaag

SEQ ID NO: 160 - protein, 316 aa, Artificial Sequence
  Pantothenate Kinase from Escherichia coli variant
MSIKEQTLMTPYLQLDRNQWAGLRDSNPMTLSEDEIARLKGINEDLSLEEVAEIYLPLSRLLNFYISSNLRRQAVLEQFLGTNGQRIPYIISIAGSVAVGKSTTAAVLQALLSRWPEHRRVELITTDGFLHPNQVLKERGLMKKKGFPESYDMHRLVKFVSDLKSGVPNVTAPVYSHLIYDVIPDGDKTVVQPDILILEGLNVLQSGMDYPHDPHHVEVSDFVDFSIYVDAPEDLLQTWYINRFLKFREGAFTDPDSYFHNYAKLTKEEAIKTAMTIWKEMNHLNLKQNILPTRERASLILTKSANHAVEEVRLRK

SEQ ID NO: 161 - DNA, 948 bp, Artificial Sequence
  Pantothenate Kinase from Escherichia coli variant
atgagcatcaaagagcagaccctgatgaccccgtacctgcagctggaccgtaaccaatgggcggcgctgcgtgatagtaacccgatgaccctgagcgaggacgaaatcgcgcgtctgaagggtattaaccctgatctgagcctggaggaagtggcggaaatctacctgccgctgagccgtctgctgaacttctatattagcagcaacctgcgtcgtcaggcggttctggaacagtttctgggtaccaacggccagcgtatcccgtatatcattagcattgcgggtagcgtggcggttggcaaaagcaccaccgcgcgtgtgctgcaggcgctgctgagccgttggccggagcaccgtcgtgttgaactgatcaccaccgacggcttcctgcacccgaaccaagtgctgaaggagcgtggtctgatgaagaaaaagggtttcccggaaagctacgatatgcaccgtctgatgaaatttgttagtgacctgaagagcggtgtgccgaacgttaccgcgccggtgtacagccacctgatctatgatgttattccggacggcgataaaaccgtggttcagccggacatcctgattctggagggtctgaacgtgctgcaaagcggcatggactatccgcacgatccgcaccacgtgtttgttagcgacttcgtggattttagcatctacgttgacgcgccggaggatctgctgcagacctggtacattaaccgtttcctgaaatttcgtgagggtgcgttcaccgacccggatagctactttcacaactatgcgaaactgaccaaggaagaggcgatcaaaaccgcgatgaccatttggaaggagatgaaccacctgaacctgaagcaaaacattctgccgacccgtgaacgtgcgcgtctgattctgaccaaaagcgcaaaccacgcggtggaggaagttcgtctgcgtaag

SEQ ID NO: 162 - protein, 316 aa, Artificial Sequence
  Pantothenate Kinase from Escherichia coli variant
MSIKEQTLMTPYLQLDRNQWAALRDSNPMTLSEDEIARLKGINPDLSLEEVAEIYLPLSRLLNFYISSNLRRQAVLEQFLGTNGQRIPYIISIAGSVAVGKSTTARVLQALLSRWPEHRRVELITTDGFLHPNQVLKERGLMKKKGFPESYDMHRLMKFVSDLKSGVPNVTAPVYSHLIYDVIPDGDKTVVQPDILILEGLNVLQSGMDYPHDPHHVFVSDFVDFSIYVDAPEDLLQTWYINRFLKFREGAFTDPDSYFHNYAKLTKEEAIKTAMTIWKEMNHLNLKQNILPTRERARLILTKSANHAVEEVRLRK

SEQ ID NO: 163 - DNA, 948 bp, Artificial Sequence
  Pantothenate Kinase from Escherichia coli variant
atgagcatcaaagagcagaccctgatgaccccgtacctgcagctggaccgtaaccaatgggcggcgctgcgtgatagtaacccgatgaccctgagcgaggacgaaatcgcgcgtctgaagggtattaacgaggatctgagcctggaggaagtggcggaaatctacctgccgctgagccgtctgctgaacttctatattagcagcaacctgcgtcgtcaggcggttctggaacagtttctgggtaccaacggccagcgtatcccgtatatcattagcattgcgggtagcgtggcggttggcaaaagcaccaccgcgcgtgtgctgcaggcgctgctgagccgttggccggagcaccgtcgtgttgaactgatcaccaccgacggcttcctgcacccgaaccaagtgctgaaggagcgtggtctgatgaagaaaaagggtttcccggaaagctacgatatgcaccgtctgatgaaatttgttagtgacctgaagagcggtgtgccgcaagttaccgcgccggtgtacagccacctgatctatgatgttattccggacggcgataaaaccgtggttcagccggacatcctgattctggagggtctgaacgtgctgcaaagcggcatggactatccgcacgatccgcaccacgtgtttgttagcgacttcgtggattttagcatctacgttgacgcgccggaggatctgctgcagacctggtacattaaccgtttcctgaaatttcgtgagggtgcgttcaccgacccggatagctactttcacccgtatgcgaaactgaccaaggaagaggcgatcaaaaccgcgatgaccatttggaaggagatgaaccacctgaacctgaagcaaaacattctgccgacccgtgaacgtgcgcgtctgattctgaccaaaagcgcaaaccacatcgtggaggaagttcgtctgcgtaag

SEQ ID NO: 164 - protein, 316 aa, Artificial Sequence
  Pantothenate Kinase from Escherichia coli variant
MSIKEQTLMTPYLQLDRNQWAALRDSNPMTLSEDEIARLKGINEDLSLEEVAEIYLPLSRLLNFYISSNLRRQAVLEQFLGTNGQRIPYIISIAGSVAVGKSTTARVLQALLSRWPEHRRVELITTDGFLHPNQVLKERGLMKKKGFPESYDMHRLMKFVSDLKSGVPQVTAPVYSHLIYDVIPDGDKTVVQPDILILEGLNVLQSGMDYPHDPHHVFVSDFVDFSIYVDAPEDLLQTWYINRFLKFREGAFTDPDSYFHPYAKLTKEEAIKTAMTIWKEMNHLNLKQNILPTRERARLILTKSANHIVEEVRLRK

SEQ ID NO: 165 - DNA, 948 bp, Artificial Sequence
  Pantothenate Kinase from Escherichia coli variant
atgagcatcaaagagcagaccctgatgaccccgtacctgcagctggaccgtaaccaatgggcggcgctgcgtgatagtaacccgatgaccctgagcgaggacgaaatcgcgcgtctgaagggtattaacgaggatctgagcctggaggaagtggcggaaatctacctgccgctgagccgtctgctgaacttctatattagcagcaacctgcgtcgtcaggcggttctggaacagtttctgggtaccaacggccagcgtatcccgtatatcattagcattgcgggtagcgtggcggttggcaaaagcaccaccgcgcgtgtgctgcaggcgctgctgagccgttggccggagcaccgtcgtgttgaactgatcaccaccgacggcttcctgcacccgaaccaagtgctgaaggagcgtggtctgatgaagaaaaagggtttcccggaaagctacgatatgcaccgtctgatgaaatttgttcgtgacctgaagagcggtgtgccgaacgttaccgcgccggtgtacagccacctgatctatgatgttattccggacggcgataaaaccgtggttcagccggacatcctgattctggagggtctgaacgtgctgcaaagcggcatggactatccgcacgatccgcaccacgtgtttgttagcgacttcgtggattttagcatctacgttgacgcgccggaggatctgctgcagacctggtacattaaccgtttcctgaaatttcgtgagggtgcgttcaccgacccggatagctactttcacaactatgcgaaactgaccaaggaagaggcgatcaaaaccgcgatgaccatttggaaggagatgaaccacctgaacctgaagcaaaacattctgccgacccgtgaacgtgcgagtctgattctgaccaaaagcgcaaaccacgttgtggaggaagttcgtctgcgtaag

SEQ ID NO: 166 - protein, 316 aa, Artificial Sequence
  Pantothenate Kinase from Escherichia coli variant
MSIKEQTLMTPYLQLDRNQWAALRDSNPMTLSEDEIARLKGINEDLSLEEVAEIYLPLSRLLNFYISSNLRRQAVLEQFLGTNGQRIPYIISIAGSVAVGKSTTARVLQALLSRWPEHRRVELITTDGFLHPNQVLKERGLMKKKGFPESYDMHRLMKFVRDLKSGVPNVTAPVYSHLIYDVIPDGDKTVVQPDILILEGLNVLQSGMDYPHDPHHVFVSDFVDFSIYVDAPEDLLQTWYINRFLKFREGAFTDPDSYFHNYAKLTKEEAIKTAMTIWKEMNHLNLKQNILPTRERASLILTKSANHVVEEVRLRK

SEQ ID NO: 167 - DNA, 948 bp, Artificial Sequence
  Pantothenate Kinase from Escherichia coli variant
atgagcatcaaagagcagaccctgatgaccccgtacctgcagctggaccgtaaccaatgggcggcgctgcgtgatagtaacccgatgaccctgagcgaggacgaaatcgcgcgtctgaagggtattaacgaggatctgagcctggaggaagtggcggaaatctacctgccgctgagccgtctgctgaacttctatattagcagcaacctgcgtcgtcaggcggttctggaacagtttctgggtaccaacggccagcgtatcccgtatatcattagcattgcgggtagcgtggcggttggcaaaagcaccaccgcgcgtgtgctgcaggcgctgctgagccgttggccggagcataaacgtgttgaactgatcaccaccgacggcttcctgcacccgaaccaagtgctgaaggagcgtggtctgatgaagaaaaagggtttcccggaaagctacgatatgcaccgtctgatgaaatttgttcgtgacctgaagagcggtgtgccgcaagttaccgcgccggtgtacagccacctgatctatgatgttattccggacggcgataaaaccgtggttcagccggacatcctgattctggagggtctgaacgtgctgcaaagcggcatggactatccgcacgatccgcaccacgtgtttgttagcgacttcgtggattttagcatctacgttgacgcgccggaggatctgctgcagacctggtacattaaccgtttcctgaaatttcgtgagggtgcgttcaccgacccggatagctactttcacccgtatgcgaaactgaccaaggaagaggcgatcaaaaccgcgatgaccatttggaaggagatgaaccacctgaacctgaagcaaaacattctgccgacccgtgaacgtgcgagcctgattctgaccaaaagcgcaaaccacgcggtggaggaagttcgtctgcgtaag

SEQ ID NO: 168 - protein, 316 aa, Artificial Sequence
  Pantothenate Kinase from Escherichia coli variant
MSIKEQTLMTPYLQLDRNQWAALRDSNPMTLSEDEIARLKGINEDLSLEEVAEIYLPLSRLLNFYISSNLRRQAVLEQFLGTNGQRIPYIISIAGSVAVGKSTTARVLQALLSRWPEHKRVELITTDGFLHPNQVLKERGLMKKKGFPESYDMHRLMKFVRDLKSGVPQVTAPVYSHLIYDVIPDGDKTVVQPDILILEGLNVLQSGMDYPHDPHHVFVSDFVDFSIYVDAPEDLLQTWYINRFLKFREGAFTDPDSYFHPYAKLTKEEAIKTAMTIWKEMNHLNLKQNILPTRERASLILTKSANHAVEEVRLRK

SEQ ID NO: 169 - DNA, 948 bp, Artificial Sequence
  Pantothenate Kinase from Escherichia coli variant
atgagcatcaaagagcagaccctgatgaccccgtacctgcagctggaccgtaaccaatgggcggcgctgcgtgatagtaacccgatgaccctgagcgaggacgaaatcgcgcgtctgaagtgtattaaccaggatctgagcctggaggaagtggcggaagtctacctgccgctgagccgtctgctgaacttctatattagcagcaacctgcgtcgtcaggcggttctggaacagtttctgggtaccaacggccagcgtatcccgtatatcattagcattgcgggtagcgtggcggttggcaaaagcaccaccgcgcgtgtgctgcaggcgctgctgagccgttggccggagcatcctaaggttgaactgatcaccaccgacggcttcctgcacccgaaccaagtgctgaaggagcgtggtctgatgaagaaaaagggtttcccggaaagctacgatatgcaccgtctggtgaaatttgttaaagacctgaagagcggtgtgccgcaagttaccgcgccggtgtacagccacctgatctatgatgttattccggacggcgataaaaccgtggttcagccggacatcctgattctggagggtctgaacgtgctgcaaagcggcatggactatccgcacgatccgcaccacgtgtttgttagcgacttcgtggattttagcatctacgttgacgcgccggaggatctgctgcagacctggtacattaaccgtttcctgaaatttcgtgagggtgcgttcaccgacccggatagctactttcacgggtatgcgaaactgaccaaggaagaggcgatcaaaaccgcgatgaccatttggaaggagatgaaccacctgaacctgaagcaaaacattctgccgacccgtgaacgtgcgcgtctgattctgaccaaaagcgcaaaccacgctgtggaggaagttcgtctgcgtaag

SEQ ID NO: 170 - protein, 316 aa, Artificial Sequence
  Pantothenate Kinase from Escherichia coli variant
MSIKEQTLMTPYLQLDRNQWAALRDSNPMTLSEDEIARLKCINQDLSLEEVAEVYLPLSRLLNFYISSNLRRQAVLEQFLGTNGQRIPYIISIAGSVAVGKSTTARVLQALLSRWPEHPKVELITTDGFLHPNQVLKERGLMKKKGFPESYDMHRLVKFVKDLKSGVPQVTAPVYSHLIYDVIPDGDKTVVQPDILILEGLNVLQSGMDYPHDPHHVFVSDFVDFSIYVDAPEDLLQTWYINRFLKFREGAFTDPDSYFHGYAKLTKEEAIKTAMTIWKEMNHLNLKQNILPTRERARLILTKSANHAVEEVRLRK

SEQ ID NO: 171 - DNA, 948 bp, Artificial Sequence
  Pantothenate Kinase from Escherichia coli variant
atgagcatcaaagagcagaccctgatgaccccgtacctgcagctggaccgtaaccaatgggcggcgctgcgtgatagtaacccgatgaccctgagcgaggacgaaatcgcgcgtctgaagtgtattaacgaggatctgagcctggaggaagtggcggaaatctacctgccgctgagccgtctgctgaacttctatattagcagcaacctgcgtcgtcaggcggttctggaacagtttctgggtaccaacggccagcgtatcccgtatatcattagcattgcgggtagcgtggcggttggcaaaagcaccaccgcgcgtgtgctgcaggcgctgctgagccgttggccggagcatcctcgtgttgaactgatcaccaccgacggcttcctgcacccgaaccaagtgctgaaggagcgtggtctgatgaagaaaaagggtttcccggaaagctacgatatgcaccgtctggtgaaatttgttcgtgacctgaagagcggtgtgccgaacgttaccgcgccggtgtacagccacctgatctatgatgttattccggacggcgataaaaccgtggttcagccggacatcctgattctggagggtctgaacgtgctgcaaagcggcatggactatccgcacgatccgcaccacgtgtttgttagcgacttcgtggattttagcatctacgttgacgcgccggaggatctgctgcagacctggtacattaaccgtttcctgaaatttcgtgagggtgcgttcaccgacccggatagctactttcacaattatgcgaaactgaccaaggaagaggcgatcaaaaccgcgatgaccatttggaaggagatgaaccacctgaacctgaagcaaaacattctgccgacccgtgaacgtgcgagtctgattctgaccaaaagcgcaaaccacgttgtggaggaagttcgtctgcgtaag

SEQ ID NO: 172 - protein, 316 aa, Artificial Sequence
  Pantothenate Kinase from Escherichia coli variant
MSIKEQTLMTPYLQLDRNQWAALRDSNPMTLSEDEIARLKCINEDLSLEEVAEIYLPLSRLLNFYISSNLRRQAVLEQFLGTNGQRIPYIISIAGSVAVGKSTTARVLQALLSRWPEHPRVELITTDGFLHPNQVLKERGLMKKKGFPESYDMHRLVKFVRDLKSGVPNVTAPVYSHLIYDVIPDGDKTVVQPDILILEGLNVLQSGMDYPHDPHHVFVSDFVDFSIYVDAPEDLLQTWYINRFLKFREGAFTDPDSYFHNYAKLTKEEAIKTAMTIWKEMNHLNLKQNILPTRERASLILTKSANHVVEEVRLRK

SEQ ID NO: 173 - DNA, 948 bp, Artificial Sequence
  Pantothenate Kinase from Escherichia coli variant
atgagcatcaaagagcagaccctgatgaccccgtacctgcagctggaccgtaaccaatgggcggcgctgcgtgatagtaacccgatgaccctgagcgaggacgaaatcgcgcgtctgaagggtattaaccaggatctgagcctggaggaagtggcggaaatctacctgccgctgagccgtctgctgaacttctatattagcagcaacctgcgtcgtcaggcggttctggaacagtttctgggtaccaacggccagcgtatcccgtatatcattagcattgcgggtagcgtggcggttggcaaaagcaccaccgcgcgtgtgctgcaggcgctgctgagccgttggccggagcatcgtcgtgttgaactgatcaccaccgacggcttcctgcacccgaaccaagtgctgaaggagcgtggtctgatgaagaaaaagggtttcccggaaagctacgatatgcaccgtctggtgaaatttgttagcgacctgaagagcggtgtgccgaatgttaccgcgccggtgtacagccacctgatctatgatgttattccggacggcgataaaaccgtggttcagccggacatcctgattctggagggtctgaacgtgctgcaaagcggcatggactatccgcacgatccgcaccacgtgtttgttagcgacttcgtggattttagcatctacgttgacgcgccggaggatctgctgcagacctggtacattaaccgtttcctgaaatttcgtgagggtgcgttcaccgacccggatagctactttcacccgtatgcgaaactgaccaaggaagaggcgatcaaaaccgcgatgaccatttggaaggagatgaaccacctgaacctgaagcaaaacattctgccgacccgtgaacgtgcgagcctgattctgaccaaaagcgcaaaccacgttgtggaggaagttcgtctgcgtaag

SEQ ID NO: 174 - protein, 316 aa, Artificial Sequence
  Pantothenate Kinase from Escherichia coli variant
MSIKEQTLMTPYLQLDRNQWAALRDSNPMTLSEDEIARLKGINQDLSLEEVAEIYLPLSRLLNFYISSNLRRQAVLEQFLGTNGQRIPYIISIAGSVAVGKSTTARVLQALLSRWPEHRRVELITTDGFLHPNQVLKERGLMKKKGFPESYDMHRLVKFVSDLKSGVPNVTAPVYSHLIYDVIPDGDKTVVQPDILILEGLNVLQSGMDYPHDPHHVFVSDFVDFSIYVDAPEDLLQTWYINRFLKFREGAFTDPDSYFHPYAKLTKEEAIKTAMTIWKEMNHLNLKQNILPTRERASLILTKSANHVVEEVRLRK

SEQ ID NO: 175 - DNA, 948 bp, Artificial Sequence
  Pantothenate Kinase from Escherichia coli variant
atgagcatcaaagagcagaccctgatgaccccgtacctgcagctggaccgtaaccaatgggcggcgctgcgtgatagtaacccgatgaccctgagcgaggacgaaatcgcgcgtctgaagggtattaaccctgatctgagcctggaggaagtggcggaatggtacctgccgctgagccgtctgctgaacttctatattagcagcaacctgcgtcgtcaggcggttctggaacagtttctgggtaccaacggccagcgtatcccgtatatcattagcattgcgggtagcgtggcggttggcaaaagcaccaccgcgcgtgtgctgcaggcgctgctgagccgttggccggagcatgccaaggttgaactgatcaccaccgacggcttcctgcacccgaaccaagtgctgaaggagcgtggtctgatgaagaaaaagggtttcccggaaagctacgatatgcaccgtctggtgaaatttgttagcgacctgaagagcggtgtgccgcaagttaccgcgccggtgtacagccacctgatctatgatgttattccggacggcgataaaaccgtggttcagccggacatcctgattctggagggtctgaacgtgctgcaaagcggcatggactatccgcacgatccgcaccacgtgtttgttagcgacttcgtggattttagcatctacgttgacgcgccggaggatctgctgcagacctggtacattaaccgtttcctgaaatttcgtgagggtgcgttcaccgacccggatagctactttcacgggtatgcgaaactgaccaaggaagaggcgatcaaaaccgcgatgaccatttggaaggagatgaaccacctgaacctgaagcaaaacattctgccgacccgtgaacgtgcgagcctgattctgaccaaaagcgcaaaccacgcggtggaggaagttcgtctgcgtaag

SEQ ID NO: 176 - protein, 316 aa, Artificial Sequence
  Pantothenate Kinase from Escherichia coli variant
MSIKEQTLMTPYLQLDRNQWAALRDSNPMTLSEDEIARLKGINPDLSLEEVAEWYLPLSRLLNFYISSNLRRQAVLEQFLGTNGQRIPYIISIAGSVAVGKSTTARVLQALLSRWPEHAKVELITTDGFLHPNQVLKERGLMKKKGFPESYDMHRLVKFVSDLKSGVPQVTAPVYSHLIYDVIPDGDKTVVQPDILILEGLNVLQSGMDYPHDPHHVFVSDFVDFSIYVDAPEDLLQTWYINRFLKFREGAFTDPDSYFHGYAKLTKEEAIKTAMTIWKEMNHLNLKQNILPTRERASLILTKSANHAVEEVRLRK

SEQ ID NO: 177 - DNA, 948 bp, Artificial Sequence
  Pantothenate Kinase from Escherichia coli variant
atgagcatcaaagagcagaccctgatgaccccgtacctgcagctggaccgtaaccaatgggcggcgctgcgtgatagtaacccgatgaccctgagcgaggacgaaatcgcgcgtctgaagggtattaacgaggatctgagcctggaggaagtggcggaaatctacctgccgctgagccgtctgctgaacttctatattagcagcaacctgcgtcgtcaggcggttctggaacagtttctgggtaccaacggccagcgtatcccgtatatcattagcattgcgggtagcgtggcggttggcaaaagcaccaccgcgcgtgtgctgcaggcgctgctgagccgttggccggagcatcgtcgtgttgaactgatcaccaccgacggcttcctgcacccgaaccaagtgctgaaggagcgtggtctgatgaagaaaaagggtttcccggaaagctacgatatgcaccgtctggtgaaatttgttagcgacctgaagagcggtgtgccgaacgttaccgcgccggtgtacagccacctgatctatgatgttattccggacggcgataaaaccgtggttcagccggacatcctgattctggagggtctgaacgtgctgcaaagcggcatggactatccgcacgatccgcaccacgtgtttgttagcgacttcgtggattttagcatctacgttgacgcgccggaggatctgctgcagacctggtacattaaccgtttcctgaaatttcgtgagggtgcgttcaccgacccggatagctactttcacaactatgcgaaactgaccaaggaagaggcgatcaaaaccgcgatgaccatttggaaggagatgaaccacctgaacctgaagcaaaacattctgccgacccgtgaacgtgcgagcctgattctgaccaaaagcgcaaaccacgcggtgtcggaagttcgtctgcgtaag

SEQ ID NO: 178 - protein, 316 aa, Artificial Sequence
  Pantothenate Kinase from Escherichia coli variant
MSIKEQTLMTPYLQLDRNQWAALRDSNPMTLSEDEIARLKGINEDLSLEEVAEIYLPLSRLLNFYISSNLRRQAVLEQFLGTNGQRIPYIISIAGSVAVGKSTTARVLQALLSRWPEHRRVELITTDGFLHPNQVLKERGLMKKKGFPESYDMHRLVKFVSDLKSGVPNVTAPVYSHLIYDVIPDGDKTVVQPDILILEGLNVLQSGMDYPHDPHHVFVSDFVDFSIYVDAPEDLLQTWYINRFLKFREGAFTDPDSYFHNYAKLTKEEAIKTAMTIWKEMNHLNLKQNILPTRERASLILTKSANHAVSEVRLRK

SEQ ID NO: 179 - DNA, 948 bp, Artificial Sequence
  Pantothenate Kinase from Escherichia coli variant
atgagcatcaaagagcagaccctgatgaccccgtacctgcagctggaccgtaaccaatgggcggcgctgcgtgatagtaacccgatgaccctgagcgaggacgaaatcgcgcgtctgaagtgtattaaccaggatctgagcctggaggaagtggcggaaatctacctgccgctgagccgtctgctgaacttctatattagcagcaacctgcgtcgtcaggcggttctggaacagtttctgggtaccaacggccagcgtatcccgtatatcattagcattgcgggtagcgtggcggttggcaaaagcaccaccgcgcgtgtgctgcaggcgctgctgagccgttggccggagcaccgtcgtgttgaactgatcaccaccgacggcttcctgcacccgaaccaagtgctgaaggagcgtggtctgatgaagaaaaagggtttcccggaaagctacgatatgcaccgtctggtgaaatttgttagcgacctgaagagcggtgtgccgcaagttaccgcgccggtgtacagccacctgatctatgatgttattccggacggcgataaaaccgtggttcagccggacatcctgattctggagggtctgaacgtgctgcaaagcggcatggactatccgcacgatccgcaccacgtgtttgttagcgacttcgtggattttagcatctacgttgacgcgccggaggatctgctgcagacctggtacattaaccgtttcctgaaatttcgtgagggtgcgttcaccgacccggatagctactttcacccgtatgcgaaactgaccaaggaagaggcgatcaaaaccgcgatgaccatttggaaggagatgaaccacctgaacctgaagcaaaacattctgccgacccgtgaacgtgcgagcctgattctgaccaaaagcgcaaaccacgttgtggaggaagttcgtctgcgtaag

SEQ ID NO: 180 - protein, 316 aa, Artificial Sequence
  Pantothenate Kinase from Escherichia coli variant
MSIKEQTLMTPYLQLDRNQWAALRDSNPMTLSEDEIARLKCINQDLSLEEVAEIYLPLSRLLNFYISSNLRRQAVLEQFLGTNGQRIPYIISIAGSVAVGKSTTARVLQALLSRWPEHRRVELITTDGFLHPNQVLKERGLMKKKGFPESYDMHRLVKFVSDLKSGVPQVTAPVYSHLIYDVIPDGDKTVVQPDILILEGLNVLQSGMDYPHDPHHVFVSDFVDFSIYVDAPEDLLQTWYINRFLKFREGAFTDPDSYFHPYAKLTKEEAIKTAMTIWKEMNHLNLKQNILPTRERASLILTKSANHVVEEVRLRK

SEQ ID NO: 181 - DNA, 948 bp, Artificial Sequence
  Pantothenate Kinase from Escherichia coli variant
atgagcatcaaagagcagaccctgatgaccccgtacctgcagctggaccgtaaccaatgggcggcgctgcgtgatagtaacccgatgaccctgagcgaggacgaaatcgcgcgtctgaagtgtattaaccctgatctgagcctggaggaagtggcggaatggtacctgccgctgagccgtctgctgaacttctatattagcagcaacctgcgtcgtcaggcggttctggaacagtttctgggtaccaacggccagcgtatcccgtatatcattagcattgcgggtagcgtggcggttggcaaaagcaccaccgcgcgtgtgctgcaggcgctgctgagccgttggccggagcatcctcgtgttgaactgatcaccaccgacggcttcctgcacccgaaccaagtgctgaaggagcgtggtctgatgaagaaaaagggtttcccggaaagctacgatatgcaccgtctggtgaaatttgttagcgacctgaagagcggtgtgccgaatgttaccgcgccggtgtacagccacctgatctatgatgttattccggacggcgataaaaccgtggttcagccggacatcctgattctggagggtctgaacgtgctgcaaagcggcatggactatccgcacgatccgcaccacgtgtttgttagcgacttcgtggattttagcatctacgttgacgcgccggaggatctgctgcagacctggtacattaaccgtttcctgaaatttcgtgagggtgcgttcaccgacccggatagctactttcacaactatgcgaaactgaccaaggaagaggcgatcaaaaccgcgatgaccatttggaaggagatgaaccacctgaacctgaagcaaaacattctgccgacccgtgaacgtgcgcgtctgattctgaccaaaagcacaaaccacgcggtggaggaagttcgtctgcgtaag

SEQ ID NO: 182 - protein, 316 aa, Artificial Sequence
  Pantothenate Kinase from Escherichia coli variant
MSIKEQTLMTPYLQLDRNQWAALRDSNPMTLSEDEIARLKCINPDLSLEEVAEWYLPLSRLLNFYISSNLRRQAVLEQFLGTNGQRIPYIISIAGSVAVGKSTTARVLQALLSRWPEHPRVELITTDGFLHPNQVLKERGLMKKKGFPESYDMHRLVKFVSDLKSGVPNVTAPVYSHLIYDVIPDGDKTVVQPDILILEGLNVLQSGMDYPHDPHHVFVSDFVDFSIYVDAPEDLLQTWYINRFLKFREGAFTDPDSYFHNYAKLTKEEAIKTAMTIWKEMNHLNLKQNILPTRERARLILTKSTNHAVEEVRLRK

SEQ ID NO: 183 - DNA, 948 bp, Artificial Sequence
  Pantothenate Kinase from Escherichia coli variant
atgagcatcaaagagcagaccctgatgaccccgtacctgcagctggaccgtaaccaatgggcggcgctgcgtgatagtaacccgatgaccctgagcgaggacgaaatcgcgcgtctgaagggtattaacgaggatctgagcctggaggaagtggcggaaatctacctgccgctgagccgtctgctgaacttctatattagcagcaacctgcgtcgtcaggcggttctggaacagtttctgggtaccaacggccagcgtatcccgtatatcattagcattgcgggtagcgtggcggttggcaaaagcaccaccgcgcgtgtgctgcaggcgctgctgagccgttggccggagcatcaacgtgttgaactgatcaccaccgacggcttcctgcacccgaaccaagtgctgaaggagcgtggtctgatgaagaaaaagggtttcccggaaagctacgatatgcaccgtctggtgaaatttgttagtgacctgaagagcggtgtgccgcaagttaccgcgccggtgtacagccacctgatctatgatgttattccggacggcgataaaaccgtggttcagccggacatcctgattctggagggtctgaacgtgctgcaaagcggcatggactatccgcacgatccgcaccacgtgtttgttagcgacttcgtggattttagcatctacgttgacgcgccggaggatctgctgcagacctggtacattaaccgtttcctgaaatttcgtgagggtgcgttcaccgacccggatagctactttcacgggtatgcgaaactgaccaaggaagaggcgatcaaaaccgcgatgaccatttggaaggagatgaaccacctgaacctgaagcaaaacattctgccgacccgtgaacgtgcgagcctgattctgaccaaaagcgcaaaccacgctgtggaggaagttcgtctgcgtaag

SEQ ID NO: 184 - protein, 316 aa, Artificial Sequence
  Pantothenate Kinase from Escherichia coli variant
MSIKEQTLMTPYLQLDRNQWAALRDSNPMTLSEDEIARLKGINEDLSLEEVAEIYLPLSRLLNFYISSNLRRQAVLEQFLGTNGQRIPYIISIAGSVAVGKSTTARVLQALLSRWPEHQRVELITTDGFLHPNQVLKERGLMKKKGFPESYDMHRLVKFVSDLKSGVPQVTAPVYSHLIYDVIPDGDKTVVQPDILILEGLNVLQSGMDYPHDPHHVFVSDFVDFSIYVDAPEDLLQTWYINRFLKFREGAFTDPDSYFHGYAKLTKEEAIKTAMTIWKEMNHLNLKQNILPTRERASLILTKSANHAVEEVRLRK

SEQ ID NO: 185 - DNA, 948 bp, Artificial Sequence
  Pantothenate Kinase from Escherichia coli variant
atgagcatcaaagagcagaccctgatgaccccgtacctgcagctggaccgtaaccaatgggcggcgctgcgtgatagtaacccgatgaccctgagcgaggacgaaatcgcgcgtctgaagggtattaaccaggatctgagcctggaggaagtggcggaaatctacctgccgctgagccgtctgctgaacttctatattagcagcaacctgcgtcgtcaggcggttctggaacagtttctgggtaccaacggccagcgtatcccgtatatcattagcattgcgggtagcgtggcggttggcaaaagcaccaccgcgcgtgtgctgcaggcgctgctgagccgttggccggagcatcgtcgtgttgaactgatcaccaccgacggcttcctgcacccgaaccaagtgctgaaggagcgtggtctgatgaagaaaaagggtttcccggaaagctacgatatgcaccgtctgatgaaatttgttaaagacctgaagagcggtgtgccgcaagttaccgcgccggtgtacagccacctgatctatgatgttattccggacggcgataaaaccgtggttcagccggacatcctgattctggagggtctgaacgtgctgcaaagcggcatggactatccgcacgatccgcaccacgtgtttgttagcgacttcgtggattttagcatctacgttgacgcgccggaggatctgctgcagacctggtacattaaccgtttcctgaaatttcgtgagggtgcgttcaccgacccggatagctactttcacaattatgcgaaactgaccaaggaagaggcgatcaaaaccgcgatgaccatttggaaggagatgaaccacctgaacctgaagcaaaacattctgccgacccgtgaacgtgcgagtctgattctgaccaaaagcgcaaaccacgctgtggaggaagttcgtctgcgtaag

SEQ ID NO: 186 - protein, 316 aa, Artificial Sequence
  Pantothenate Kinase from Escherichia coli variant
MSIKEQTLMTPYLQLDRNQWAALRDSNPMTLSEDEIARLKGINQDLSLEEVAEIYLPLSRLLNFYISSNLRRQAVLEQFLGTNGQRIPYIISIAGSVAVGKSTTARVLQALLSRWPEHRRVELITTDGFLHPNQVLKERGLMKKKGFPESYDMHRLMKFVKDLKSGVPQVTAPVYSHLIYDVIPDGDKTVVQPDILILEGLNVLQSGMDYPHDPHHVFVSDFVDFSIYVDAPEDLLQTWYINRFLKFREGAFTDPDSYFHNYAKLTKEEAIKTAMTIWKEMNHLNLKQNILPTRERASLILTKSANHAVEEVRLRK

SEQ ID NO: 187 - DNA, 948 bp, Artificial Sequence
  Pantothenate Kinase from Escherichia coli variant
atgagcatcaaagagcagaccctgatgaccccgtacctgcagctggaccgtaaccaatgggcggcgctgcgtgatagtaacccgatgaccctgagcgaggacgaaatcgcgcgtctgaagggtattaaccctgatctgagcctggaggaagtggcggaaatctacctgccgctgagccgtctgctgaacttctatattagcagcaacctgcgtcgtcaggcggttctggaacagtttctgggtaccaacggccagcgtatcccgtatatcattagcattgcgggtagcgtggcggttggcaaaagcaccaccgcgcgtgtgctgcaggcgctgctgagccgttggccggagcataaacgtgttgaactgatcaccaccgacggcttcctgcacccgaaccaagtgctgaaggagcgtggtctgatgaagaaaaagggtttcccggaaagctacgatatgcaccgtctgatgaaatttgttaaagacctgaagagcggtgtgccgaatgttaccgcgccggtgtacagccacctgatctatgatgttattccggacggcgataaaaccgtggttcagccggacatcctgattctggagggtctgaacgtgctgcaaagcggcatggactatccgcacgatccgcaccacgtgtttgttagcgacttcgtggattttagcatctacgttgacgcgccggaggatctgctgcagacctggtacattaaccgtttcctgaaatttcgtgagggtgcgttcaccgacccggatagctactttcacaactatgcgaaactgaccaaggaagaggcgatcaaaaccgcgatgaccatttggaaggagatgaaccacctgaacctgaagcaaaacattctgccgacccgtgaacgtgcgagtctgattctgaccaaaagcgcaaaccacgcggtggaggaagttcgtctgcgtaag

SEQ ID NO: 188 - protein, 316 aa, Artificial Sequence
  Pantothenate Kinase from Escherichia coli variant
MSIKEQTLMTPYLQLDRNQWAALRDSNPMTLSEDEIARLKGINPDLSLEEVAEIYLPLSRLLNFYISSNLRRQAVLEQFLGTNGQRIPYIISIAGSVAVGKSTTARVLQALLSRWPEHKRVELITTDGFLHPNQVLKERGLMKKKGFPESYDMHRLMKFVKDLKSGVPNVTAPVYSHLIYDVIPDGDKTVVQPDILILEGLNVLQSGMDYPHDPHHVFVSDFVDFSIYVDAPEDLLQTWYINRFLKFREGAFTDPDSYFHNYAKLTKEEAIKTAMTIWKEMNHLNLKQNILPTRERASLILTKSANHAVEEVRLRK

SEQ ID NO: 189 - DNA, 948 bp, Artificial Sequence
  Pantothenate Kinase from Escherichia coli variant
atgagcatcaaagagcagaccctgatgaccccgtacctgcagctggaccgtaaccaatgggcggcgctgcgtgatagtaacccgatgaccctgagcgaggacgaaatcgcgcgtctgaagggtattaaccaggatctgagcctggaggaagtggcggaaatctacctgccgctgagccgtctgctgaacttctatattagcagcaacctgcgtcgtcaggcggttctggaacagtttctgggtaccaacggccagcgtatcccgtatatcattagcattgcgggtagcgtggcggttggcaaaagcaccaccgcgcgtgtgctgcaggcgctgctgagccgttggccggagcatcgtcgtgttgaactgatcaccaccgacggcttcctgcacccgaaccaagtgctgaaggagcgtggtctgatgaagaaaaagggtttcccggaaagctacgatatgcaccgtctggtgaaatttgttagtgacctgaagagcggtgtgccgaatgttaccgcgccggtgtacagccacctgatctatgatgttattccggacggcgataaaaccgtggttcagccggacatcctgattctggagggtctgaacgtgctgcaaagcggcatggactatccgcacgatccgcaccacgtgtttgttagcgacttcgtggattttagcatctacgttgacgcgccggaggatctgctgcagacctggtacattaaccgtttcctgaaatttcgtgagggtgcgttcaccgacccggatagctactttcacgggtatgcgaaactgaccaaggaagaggcgatcaaaaccgcgatgaccatttggaaggagatgaaccacctgaacctgaagcaaaacattctgccgacccgtgaacgtgcgcgtctgattctgaccaaaagcgcaaaccacgttgtggaggaagttcgtctgcgtaag

SEQ ID NO: 190 - protein, 316 aa, Artificial Sequence
  Pantothenate Kinase from Escherichia coli variant
MSIKEQTLMTPYLQLDRNQWAALRDSNPMTLSEDEIARLKGINQDLSLEEVAEIYLPLSRLLNFYISSNLRRQAVLEQFLGTNGQRIPYIISIAGSVAVGKSTTARVLQALLSRWPEHRRVELITTDGFLHPNQVLKERGLMKKKGFPESYDMHRLVKFVSDLKSGVPNVTAPVYSHLIYDVIPDGDKTVVQPDILILEGLNVLQSGMDYPHDPHHVFVSDFVDFSIYVDAPEDLLQTWYINRFLKFREGAFTDPDSYFHGYAKLTKEEAIKTAMTIWKEMNHLNLKQNILPTRERARLILTKSANHVVEEVRLRK

SEQ ID NO: 191 - DNA, 948 bp, Artificial Sequence
  Pantothenate Kinase from Escherichia coli variant
atgagcatcaaagagcagaccctgatgaccccgtacctgcagctggaccgtaaccaatgggcggcgctgcgtgatagtaacccgatgaccctgagcgaggacgaaatcgcgcgtctgaagggtattaaccctgatctgagcctggaggaagtggcggaaatctacctgccgctgagccgtctgctgaacttctatattagcagcaacctgcgtcgtcaggcggttctggaacagtttctgggtaccaacggccagcgtatcccgtatatcattagcattgcgggtagcgtggcggttggcaaaagcaccaccgcgcgtgtgctgcaggcgctgctgagccgttggccggagcatcctaaggttgaactgatcaccaccgacggcttcctgcacccgaaccaagtgctgaaggagcgtggtctgatgaagaaaaagggtttcccggaaagctacgatatgcaccgtctggtgaaatttgttagtgacctgaagagcggtgtgccgaacgttaccgcgccggtgtacagccacctgatctatgatgttattccggacggcgataaaaccgtggttcagccggacatcctgattctggagggtctgaacgtgctgcaaagcggcatggactatccgcacgatccgcaccacgtgtttgttagcgacttcgtggattttagcatctacgttgacgcgccggaggatctgctgcagacctggtacattaaccgtttcctgaaatttcgtgagggtgcgttcaccgacccggatagctactttcacccgtatgcgaaactgaccaaggaagaggcgatcaaaaccgcgatgaccatttggaaggagatgaaccacctgaacctgaagcaaaacattctgccgacccgtgaacgtgcgagtctgattctgaccaaaagcgcaaaccacgcggtggaggaagttcgtctgcgtaag

SEQ ID NO: 192 - protein, 316 aa, Artificial Sequence
  Pantothenate Kinase from Escherichia coli variant
MSIKEQTLMTPYLQLDRNQWAALRDSNPMTLSEDEIARLKGINPDLSLEEVAEIYLPLSRLLNFYISSNLRRQAVLEQFLGTNGQRIPYIISIAGSVAVGKSTTARVLQALLSRWPEHPKVELITTDGFLHPNQVLKERGLMKKKGFPESYDMHRLVKFVSDLKSGVPNVTAPVYSHLIYDVIPDGDKTVVQPDILILEGLNVLQSGMDYPHDPHHVFVSDFVDFSIYVDAPEDLLQTWYINRFLKFREGAFTDPDSYFHPYAKLTKEEAIKTAMTIWKEMNHLNLKQNILPTRERASLILTKSANHAVEEVRLRK

SEQ ID NO: 193 - DNA, 948 bp, Artificial Sequence
  Pantothenate Kinase from Escherichia coli variant
atgagcatcaaagagcagaccctgatgaccccgtacctgcagctggaccgtaaccaatgggcggcgctgcgtgatagtaacccgatgaccctgagcgaggacgaaatcgcgcgtctgaagggtattaacgaggatctgagcctggaggaagtggcggaaatctacctgccgctgagccgtctgctgaacttctatattagcagcaacctgcgtcgtcaggcggttctggaacagtttctgggtaccaacggccagcgtatcccgtatatcattagcattgcgggtagcgtggcggttggcaaaagcaccaccgcgcgtgtgctgcaggcgctgctgagccgttggccggagcatcgtaaggttgaactgatcaccaccgacggcttcctgcacccgaaccaagtgctgaaggagcgtggtctgatgaagaaaaagggtttcccggaaagctacgatatgcaccgtctgatgaaatttgttagtgacctgaagagcggtgtgccgaatgttaccgcgccggtgtacagccacctgatctatgatgttattccggacggcgataaaaccgtggttcagccggacatcctgattctggagggtctgaacgtgctgcaaagcggcatggactatccgcacgatccgcaccacgtgtttgttagcgacttcgtggattttagcatctacgttgacgcgccggaggatctgctgcagacctggtacattaaccgtttcctgaaatttcgtgagggtgcgttcaccgacccggatagctactttcacccgtatgcgaaactgaccaaggaagaggcgatcaaaaccgcgatgaccatttggaaggagatgaaccacctgaacctgaagcaaaacattctgccgacccgtgaacgtgcgagcctgattctgaccaaaagcgcaaaccacgcggtggaggaagttcgtctgcgtaag

SEQ ID NO: 194 - protein, 316 aa, Artificial Sequence
  Pantothenate Kinase from Escherichia coli variant
MSIKEQTLMTPYLQLDRNQWAALRDSNPMTLSEDEIARLKGINEDLSLEEVAEIYLPLSRLLNFYISSNLRRQAVLEQFLGTNGQRIPYIISIAGSVAVGKSTTARVLQALLSRWPEHRKVELITTDGFLHPNQVLKERGLMKKKGFPESYDMHRLMKFVSDLKSGVPNVTAPVYSHLIYDVIPDGDKTVVQPDILILEGLNVLQSGMDYPHDPHHVFVSDFVDFSIYVDAPEDLLQTWYINRFLKFREGAFTDPDSYFHPYAKLTKEEAIKTAMTIWKEMNHLNLKQNILPTRERASLILTKSANHAVEEVRLRK

SEQ ID NO: 195 - DNA, 948 bp, Artificial Sequence
  Pantothenate Kinase from Escherichia coli variant
atgagcatcaaagagcagaccctgatgaccccgtacctgcagctggaccgtaaccaatgggcggcgctgcgtgatagtaacccgatgaccctgagcgaggacgaaatcgcgcgtctgaagggtattaacgaggatctgagcctggaggaagtggcggaaatctacctgccgctgagccgtctgctgaacttctatattagcagcaacctgcgtcgtcaggcggttctggaacagtttctgggtaccaacggccagcgtatcccgtatatcattagcattgcgggtagcgtggcggttggcaaaagcaccaccgcgcgtgtgctgcaggcgctgctgagccgttggccggagcatcgtcgtgttgaactgatcaccaccgacggcttcctgcacccgaaccaagtgctgaaggagcgtggtctgatgaagaaaaagggtttcccggaaagctacgatatgcaccgtctggtgaaatttgttagcgacctgaagagcggtgtgccgaacgttaccgcgccggtgtacagccacctgatctatgatgttattccggacggcgataaaaccgtggttcagccggacatcctgattctggagggtctgaacgtgctgcaaagcggcatggactatccgcacgatccgcaccacgtgtttgttagcgacttcgtggattttagcatctacgttgacgcgccggaggatctgctgcagacctggtacattaaccgtttcctgaaatttcgtgagggtgcgttcaccgacccggatagctactttcacaactatgcgaaactgaccaaggaagaggcgatcaaaaccgcgatgaccatttggaaggagatgaaccacctgaacctgaagcaaaacattctgccgacccgtgaacgtgcgagcctgattctggctaaaagcgcaaaccacgcggtggaggaagttcgtctgcgtaag

SEQ ID NO: 196 - protein, 316 aa, Artificial Sequence
  Pantothenate Kinase from Escherichia coli variant
MSIKEQTLMTPYLQLDRNQWAALRDSNPMTLSEDEIARLKGINEDLSLEEVAEIYLPLSRLLNFYISSNLRRQAVLEQFLGTNGQRIPYIISIAGSVAVGKSTTARVLQALLSRWPEHRRVELITTDGFLHPNQVLKERGLMKKKGFPESYDMHRLVKFVSDLKSGVPNVTAPVYSHLIYDVIPDGDKTVVQPDILILEGLNVLQSGMDYPHDPHHVFVSDFVDFSIYVDAPEDLLQTWYINRFLKFREGAFTDPDSYFHNYAKLTKEEAIKTAMTIWKEMNHLNLKQNILPTRERASLILAKSANHAVEEVRLRK

SEQ ID NO: 197 - DNA, 948 bp, Artificial Sequence
  Pantothenate Kinase from Escherichia coli variant
atgagcatcaaagagcagaccctgatgaccccgtacctgcagctggaccgtaaccaatgggcggcgctgcgtgatagtaacccgatgaccctgagcgaggacgaaatcgcgcgtctgaagggtattaaccaggatctgagcctggaggaagtggcggaagtctacctgccgctgagccgtctgctgaacttctatattagcagcaacctgcgtcgtcaggcggttctggaacagtttctgggtaccaacggccagcgtatcccgtatatcattagcattgcgggtagcgtggcggttggcaaaagcaccaccgcgcgtgtgctgcaggcgctgctgagccgttggccggagcatgccaaggttgaactgatcaccaccgacggcttcctgcacccgaaccaagtgctgaaggagcgtggtctgatgaagaaaaagggtttcccggaaagctacgatatgcaccgtctgatgaaatttgttcgtgacctgaagagcggtgtgccgcaagttaccgcgccggtgtacagccacctgatctatgatgttattccggacggcgataaaaccgtggttcagccggacatcctgattctggagggtctgaacgtgctgcaaagcggcatggactatccgcacgatccgcaccacgtgtttgttagcgacttcgtggattttagcatctacgttgacgcgccggaggatctgctgcagacctggtacattaaccgtttcctgaaatttcgtgagggtgcgttcaccgacccggatagctactttcacaactatgcgaaactgaccaaggaagaggcgatcaaaaccgcgatgaccatttggaaggagatgaaccacctgaacctgaagcaaaacattctgccgacccgtgaacgtgcgagtctgattctgaccaaaagcgcaaaccacgctgtggaggaagttcgtctgcgtaag

SEQ ID NO: 198 - protein, 316 aa, Artificial Sequence
  Pantothenate Kinase from Escherichia coli variant
MSIKEQTLMTPYLQLDRNQWAALRDSNPMTLSEDEIARLKGINQDLSLEEVAEVYLPLSRLLNFYISSNLRRQAVLEQFLGTNGQRIPYIISIAGSVAVGKSTTARVLQALLSRWPEHAKVELITTDGFLHPNQVLKERGLMKKKGFPESYDMHRLMKFVRDLKSGVPQVTAPVYSHLIYDVIPDGDKTVVQPDILILEGLNVLQSGMDYPHDPHHVFVSDFVDFSIYVDAPEDLLQTWYINRFLKFREGAFTDPDSYFHNYAKLTKEEAIKTAMTIWKEMNHLNLKQNILPTRERASLILTKSANHAVEEVRLRK

SEQ ID NO: 199 - DNA, 948 bp, Artificial Sequence
  Pantothenate Kinase from Escherichia coli variant
atgagcatcaaagagcagaccctgatgaccccgtacctgcagctggaccgtaaccaatgggcggcgctgcgtgatagtaacccgatgaccctgagcgaggacgaaatcgcgcgtctgaagggtattaacgaggatctgagcctggaggaagtggcggaaatctacctgccgctgagccgtctgctgaacttctatattagcagcaacctgcgtcgtcaggcggttctggaacagtttctgggtaccaacggccagcgtatcccgtatatcattagcattgcgggtagcgtggcggttggcaaaagcaccaccgcgcgtgtgctgcaggcgctgctgagccgttggccggagcaccgtcgtgttgaactgatcaccaccgacggcttcctgcacccgaaccaagtgctgaaggagcgtggtctgatgaagaaaaagggtttcccggaaagctacgatatgcaccgtctgatgaaatttgttcgtgacctgaagagcggtgtgccgcaagttaccgcgccggtgtacagccacctgatctatgatgttattccggacggcgataaaaccgtggttcagccggacatcctgattctggagggtctgaacgtgctgcaaagcggcatggactatccgcacgatccgcaccacgtgtttgttagcgacttcgtggattttagcatctacgttgacgcgccggaggatctgctgcagacctggtacattaaccgtttcctgaaatttcgtgagggtgcgttcaccgacccggatagctactttcacgggtatgcgaaactgaccaaggaagaggcgatcaaaaccgcgatgaccatttggaaggagatgaaccacctgaacctgaagcaaaacattctgccgacccgtgaacgtgcgagtctgattctgaccaaaagcgcaaaccacgctgtggaggaagttcgtctgcgtaag

SEQ ID NO: 200 - protein, 316 aa, Artificial Sequence
  Pantothenate Kinase from Escherichia coli variant
MSIKEQTLMTPYLQLDRNQWAALRDSNPMTLSEDEIARLKGINEDLSLEEVAEIYLPLSRLLNFYISSNLRRQAVLEQFLGTNGQRIPYIISIAGSVAVGKSTTARVLQALLSRWPEHRRVELITTDGFLHPNQVLKERGLMKKKGFPESYDMHRLMKFVRDLKSGVPQVTAPVYSHLIYDVIPDGDKTVVQPDILILEGLNVLQSGMDYPHDPHHVFVSDFVDFSIYVDAPEDLLQTWYINRFLKFREGAFTDPDSYFHGYAKLTKEEAIKTAMTIWKEMNHLNLKQNILPTRERASLILTKSANHAVEEVRLRK

SEQ ID NO: 201 - DNA, 948 bp, Artificial Sequence
  Pantothenate Kinase from Escherichia coli variant
atgagcatcaaagagcagaccctgatgaccccgtacctgcaactggaccgtaacacgtgggcggggctgcgtgatagtaacccgatgaccctgagcgaggacgaaatcgcgcgtctgaagtgtattaaccctgatctgagcctggaggaagtggcggaagtctacctgccgctgagccgtctgctgaacttctatattagcagcaacctgcgtcgtcaggcggttctggaacagtttctgggtaccaacggccagcgtatcccgtatatcattagcattgcgggtagcgtggcggttggcaaaagcaccaccgcgcgtgtgctgcaggcgctgctgagccgttggccggagcatgcccgtgttgaactgatcaccaccgacggcttcctgcacccgaaccaagtgctgaaggagcgtggtctgatgaagaaaaagggtttcccggaaagctacgatatgcaccgtctgatgaaatttgttagtgacctgaagagcggtgtgccgaatgttaccgcgccggtgtacagccacctgatctatgatgttattccggacggcgataaaaccgtggttcagccggacatcctgattctggagggtctgaacgtgctgcaaagcggcatggactatccgcacgatccgcaccacgtgtttgttagcgacttcgtggattttagcatctacgttgacgcgccggaggatctgctgcagacctggtacattaaccgtttcctgaaatttcgtgagggtgcgttcaccgacccggatagctactttcacgggtatgcgaaactgaccaaggaagaggcgatcaaaaccgcgatgaccatttggaaggagatgaaccacctgaacctgaagcaaaacattctgccgacccgtgaacgtgcgcgtctgattctgaccaaaagcgcaaaccacatcgtggaggaagttcgtctgcgtaag

SEQ ID NO: 202 - protein, 316 aa, Artificial Sequence
  Pantothenate Kinase from Escherichia coli variant
MSIKEQTLMTPYLQLDRNTWAGLRDSNPMTLSEDEIARLKCINPDLSLEEVAEVYLPLSRLLNFYISSNLRRQAVLEQFLGTNGQRIPYIISIAGSVAVGKSTTARVLQALLSRWPEHARVELITTDGFLHPNQVLKERGLMKKKGFPESYDMHRLMKFVSDLKSGVPNVTAPVYSHLIYDVIPDGDKTVVQPDILILEGLNVLQSGMDYPHDPHHVFVSDFVDFSIYVDAPEDLLQTWYINRFLKFREGAFTDPDSYFHGYAKLTKEEAIKTAMTIWKEMNHLNLKQNILPTRERARLILTKSANHIVEEVRLRK

SEQ ID NO: 203 - DNA, 948 bp, Artificial Sequence
  Pantothenate Kinase from Escherichia coli variant
atgagcatcaaagagcagaccctgatgaccccgtacctgcagctggaccgtaaccaatgggcggcgctgcgtgatagtaacccgatgaccctgagcgaggacgaaatcgcgcgtctgaagggtattaacgaggatctgagcctggaggaagtggcggaaatctacctgccgctgagccgtctgctgaacttctatattagcagcaacctgcgtcgtcaggcggttctggaacagtttctgggtaccaacggccagcgtatcccgtatatcattagcattgcgggtagcgtggcggttggcaaaagcaccaccgcgcgtgtgctgcaggcgctgctgagccgttggccggagcatcgtcgtgttgaactgatcaccaccgacggcttcctgcacccgaaccaagtgctgaaggagcgtggtctgatgaagaaaaagggtttcccggaaagctacgatatgcaccgtctggtgaaatttgttagcgacctgaagagcggtgtgccgaacgttaccgcgccggtgtacagccacctgatctatgatgttattccggacggcgataaaaccgtggttcagccggacatcctgattctggagggtctgaacgtgctgcaaagcggcatggactatccgcacgatccgcaccacgtgtttgttagcgacttcgtggattttagcatctacgttgacgcgccggaggatctgctgcagacctggtacattaaccgtttcctgaaatttcgtgagcgtgcgttcaccgacccggatagctactttcacaactatgcgaaactgaccaaggaagaggcgatcaaaaccgcgatgaccatttggaaggagatgaaccacctgaacctgaagcaaaacattctgccgacccgtgaacgtgcgagcctgattctgaccaaaagcgcaaaccacgcggtggaggaagttcgtctgcgtaag

SEQ ID NO: 204 - protein, 316 aa, Artificial Sequence
  Pantothenate Kinase from Escherichia coli variant
MSIKEQTLMTPYLQLDRNQWAALRDSNPMTLSEDEIARLKGINEDLSLEEVAEIYLPLSRLLNFYISSNLRRQAVLEQFLGTNGQRIPYIISIAGSVAVGKSTTARVLQALLSRWPEHRRVELITTDGFLHPNQVLKERGLMKKKGFPESYDMHRLVKFVSDLKSGVPNVTAPVYSHLIYDVIPDGDKTVVQPDILILEGLNVLQSGMDYPHDPHHVFVSDFVDFSIYVDAPEDLLQTWYINRFLKFRERAFTDPDSYFHNYAKLTKEEAIKTAMTIWKEMNHLNLKQNILPTRERASLILTKSANHAVEEVRLRK

SEQ ID NO: 205 - DNA, 948 bp, Artificial Sequence
  Pantothenate Kinase from Escherichia coli variant
atgagcatcaaagagcagaccctgatgaccccgtacctgcagctggaccgtaaccaatgggcggcgctgcgtgatagtaacccgatgaccctgagcgaggacgaaatcgcgcgtctgaagtgtattaaccctgatctgagcctggaggaagtggcggaaatctacctgccgctgagccgtctgctgaacttctatattagcagcaacctgcgtcgtcaggcggttctggaacagtttctgggtaccaacggccagcgtatcccgtatatcattagcattgcgggtagcgtggcggttggcaaaagcaccaccgcgcgtgtgctgcaggcgctgctgagccgttggccggagcaccgtcgtgttgaactgatcaccaccgacggcttcctgcacccgaaccaagtgctgaaggagcgtggtctgatgaagaaaaagggtttcccggaaagctacgatatgcaccgtctggtgaaatttgttcgtgacctgaagagcggtgtgccgcaagttaccgcgccggtgtacagccacctgatctatgatgttattccggacggcgataaaaccgtggttcagccggacatcctgattctggagggtctgaacgtgctgcaaagcggcatggactatccgcacgatccgcaccacgtgtttgttagcgacttcgtggattttagcatctacgttgacgcgccggaggatctgctgcagacctggtacattaaccgtttcctgaaatttcgtgagggtgcgttcaccgacccggatagctactttcacgggtatgcgaaactgaccaaggaagaggcgatcaaaaccgcgatgaccatttggaaggagatgaaccacctgaacctgaagcaaaacattctgccgacccgtgaacgtgcgagtctgattctgaccaaaagcgcaaaccacgcggtggaggaagttcgtctgcgtaag

SEQ ID NO: 206 - protein, 316 aa, Artificial Sequence
  Pantothenate Kinase from Escherichia coli variant
MSIKEQTLMTPYLQLDRNQWAALRDSNPMTLSEDEIARLKCINPDLSLEEVAEIYLPLSRLLNFYISSNLRRQAVLEQFLGTNGQRIPYIISIAGSVAVGKSTTARVLQALLSRWPEHRRVELITTDGFLHPNQVLKERGLMKKKGFPESYDMHRLVKFVRDLKSGVPQVTAPVYSHLIYDVIPDGDKTVVQPDILILEGLNVLQSGMDYPHDPHHVFVSDFVDFSIYVDAPEDLLQTWYINRFLKFREGAFTDPDSYFHGYAKLTKEEAIKTAMTIWKEMNHLNLKQNILPTRERASLILTKSANHAVEEVRLRK

SEQ ID NO: 207 - DNA, 948 bp, Artificial Sequence
  Pantothenate Kinase from Escherichia coli variant
atgagcatcaaagagcagaccctgatgaccccgtacctgcagctggaccgtaaccaatgggcggcgctgcgtgatagtaacccgatgaccctgagcgaggacgaaatcgcgcgtctgaagggtattaacgaggatctgagcctggaggaagtggcggaagtctacctgccgctgagccgtctgctgaacctgtatattagcagcaacctgcgtcgtcaggcggttctggaacagtttctgggtaccaacggccagcgtatcccgtatatcattagcattgcgggtagcgtggcggttggcaaaagcaccaccgcgcgtgtgctgcaggcgctgctgagccgttggccggagcatcgtcgtgttgaactgatcaccaccgacggcttcctgcacccgaaccaagtgctgaaggagcgtggtctgatgaagaaaaagggtttcccggaaagctacgatatgcaccgtctgatgaaatttgttaaagacctgaagagcggtgtgccgaacgttaccgcgccggtgtacagccacctgatctatgatgttattccggacggcgataaaaccgtggttcagccggacatcctgattctggagggtctgaacgtgctgcaaagcggcatggactatccgcacgatccgcaccacgtgtttgttagcgacttcgtggattttagcatctacgttgacgcgccggaggatctgctgcagacctggtacattaaccgtttcctgaaatttcgtgagggtgcgttcaccgacccggatagctactttcacgggtatgcgaaactgaccaaggaagaggcgatcaaaaccgcgatgaccatttggaaggagatgaaccacctgaacctgaagcaaaacattctgccgacccgtgaacgtgcgagcctgattctgaccaaaagcgcaaaccacatcgtggaggaagttcgtctgcgtaag

SEQ ID NO: 208 - protein, 316 aa, Artificial Sequence
  Pantothenate Kinase from Escherichia coli variant
MSIKEQTLMTPYLQLDRNQWAALRDSNPMTLSEDEIARLKGINEDLSLEEVAEVYLPLSRLLNLYISSNLRRQAVLEQFLGTNGQRIPYIISIAGSVAVGKSTTARVLQALLSRWPEHRRVELITTDGFLHPNQVLKERGLMKKKGFPESYDMHRLMKFVKDLKSGVPNVTAPVYSHLIYDVIPDGDKTVVQPDILILEGLNVLQSGMDYPHDPHHVFVSDFVDFSIYVDAPEDLLQTWYINRFLKFREGAFTDPDSYFHGYAKLTKEEAIKTAMTIWKEMNHLNLKQNILPTRERASLILTKSANHIVEEVRLRK

SEQ ID NO: 209 - DNA, 948 bp, Artificial Sequence
  Pantothenate Kinase from Escherichia coli variant
atgagcatcaaagagcagaccctgatgaccccgtacctgcagctggaccgtaaccaatgggcggcgctgcgtgatagtaacccgatgaccctgagcgaggacgaaatcgcgcgtctgaagggtattaacgaggatctgagcctggaggaagtggcggaagtctacctgccgctgagccgtctgctgaacttctatattagcagcaacctgcgtcgtcaggcggttctggaacagtttctgggtaccaacggccagcgtatcccgtatatcattagcattgcgggtagcgtggcggttggcaaaagcaccaccgcgcgtgtgctgcaggcgctgctgagccgttggccggagcatcgtcgtgttgaactgatcaccaccgacggcttcctgcacccgaaccaagtgctgaaggagcgtggtctgatgaagaaaaagggtttcccggaaagctacgatatgcaccgtctgatgaaatttgttaaagacctgaagagcggtgtgccgaacgttaccgcgccggtgtacagccacctgatcgaggatgttattccggacggcgataaaaccgtggttcagccggacatcctgattctggagggtctgaacgtgctgcaaagcggcatggactatccgcacgatccgcaccacgtgtttgttagcgacttcgtggattttagcatctacgttgacgcgccggaggatctgctgcagacctggtacattaaccgtttcctgaaatttcgtgagggtgcgttcaccgacccggatagctactttcacgggtatgcgaaactgaccaaggaagaggcgatcaaaaccgcgatgaccatttggaaggagatgaaccacctgaacctgaagcaaaacattctgccgacccgtgaacgtgcgagcctgattctgaccaaaagcgcaaaccacatcgtggaggaagttcgtctgcgtaag

SEQ ID NO: 210 - protein, 316 aa, Artificial Sequence
  Pantothenate Kinase from Escherichia coli variant
MSIKEQTLMTPYLQLDRNQWAALRDSNPMTLSEDEIARLKGINEDLSLEEVAEVYLPLSRLLNFYISSNLRRQAVLEQFLGTNGQRIPYIISIAGSVAVGKSTTARVLQALLSRWPEHRRVELITTDGFLHPNQVLKERGLMKKKGFPESYDMHRLMKFVKDLKSGVPNVTAPVYSHLIEDVIPDGDKTVVQPDILILEGLNVLQSGMDYPHDPHHVFVSDFVDFSIYVDAPEDLLQTWYINRFLKFREGAFTDPDSYFHGYAKLTKEEAIKTAMTIWKEMNHLNLKQNILPTRERASLILTKSANHIVEEVRLRK

SEQ ID NO: 211 - DNA, 948 bp, Artificial Sequence
  Pantothenate Kinase from Escherichia coli variant
atgagcatcaaagagcagaccctgatgaccccgtacctgcagctggaccgtaaccaatgggcggcgctgcgtgatagtaacccgatgaccctgagcgaggacgaaatcgcgcgtctgaagggtattaacgaggatctgagcctggaggaagtggcggaagtctacctgccgctgagccgtctgctgaacttctatattagcagcaacctgcgtcgtcaggcggttctggaacagtttctgggtaccaacggccagcgtatcccgtatatcattagcattgcgggtagcgtggcggttggcaaaagcaccaccgcgcgtgtgctgcaggcgctgctgagccgttggccggagcatcgtcgtgttgaatggatcaccaccgacggcttcctgcacccgaaccaagtgctgaaggagcgtggtctgatgaagaaaaagggtttcccggaaagctacgatatgcaccgtctgatgaaatttgttaaagacctgaagagcggtgtgccgaacgttaccgcgccggtgtacagccacctgatctatgatgttattccggacggcgataaaaccgtggttcagccggacatcctgattctggagggtctgaacgtgctgcaaagcggcatggactatccgcacgatccgcaccacgtgtttgttagcgacttcgtggattttagcatctacgttgacgcgccggaggatctgctgcagacctggtacattaaccgtttcctgaaatttcgtgagggtgcgttcaccgacccggatagctactttcacgggtatgcgaaactgaccaaggaagaggcgatcaaaaccgcgatgaccatttggaaggagatgaaccacctgaacctgaagcaaaacattctgccgacccgtgaacgtgcgagcctgattctgaccaaaagcgcaaaccacatcgtggaggaagttcgtctgcgtaag

SEQ ID NO: 212 - protein, 316 aa, Artificial Sequence
  Pantothenate Kinase from Escherichia coli variant
MSIKEQTLMTPYLQLDRNQWAALRDSNPMTLSEDEIARLKGINEDLSLEEVAEVYLPLSRLLNFYISSNLRRQAVLEQFLGTNGQRIPYIISIAGSVAVGKSTTARVLQALLSRWPEHRRVEWITTDGFLHPNQVLKERGLMKKKGFPESYDMHRLMKFVKDLKSGVPNVTAPVYSHLIYDVIPDGDKTVVQPDILILEGLNVLQSGMDYPHDPHHVFVSDFVDFSIYVDAPEDLLQTWYINRFLKFREGAFTDPDSYFHGYAKLTKEEAIKTAMTIWKEMNHLNLKQNILPTRERASLILTKSANHIVEEVRLRK

SEQ ID NO: 213 - DNA, 948 bp, Artificial Sequence
  Pantothenate Kinase from Escherichia coli variant
atgagcatcaaagagcagaccctgatgaccccgtacctgcagctggaccgtaaccaatgggcggcgctgcgtgatagtaacccgatgaccctgagcgaggacgaaatcgcgcgtctgaagggtattaacgaggatctgagcctggaggaagtggcggaagtctacctgccgctgagccgtctgctgaacttctatattagcagcaacctgcgtcgtcaggcggttctggaacagtttctgggtaccaacggccagcgtatcccgtatatcattagcattgcgggtagcgtggcggttggcaaaagcaccaccgcgcgtgtgctgcaggcgctgctgagccgttggccggagcatcgtcgtgttgaactgatcaccaccgacggcttcctgcacccgaaccgggtgctgaaggagcgtggtctgatgaagaaaaagggtttcccggaaagctacgatatgcaccgtctgatgaaatttgttaaagacctgaagagcggtgtgccgaacgttaccgcgccggtgtacagccacctgatctatgatgttattccggacggcgataaaaccgtggttcagccggacatcctgattctggagggtctgaacgtgctgcaaagcggcatggactatccgcacgatccgcaccacgtgtttgttagcgacttcgtggattttagcatctacgttgacgcgccggaggatctgctgcagacctggtacattaaccgtttcctgaaatttcgtgagggtgcgttcaccgacccggatagctactttcacgggtatgcgaaactgaccaaggaagaggcgatcaaaaccgcgatgaccatttggaaggagatgaaccacctgaacctgaagcaaaacattctgccgacccgtgaacgtgcgagcctgattctgaccaaaagcgcaaaccacatcgtggaggaagttcgtctgcgtaag

SEQ ID NO: 214 - protein, 316 aa, Artificial Sequence
  Pantothenate Kinase from Escherichia coli variant
MSIKEQTLMTPYLQLDRNQWAALRDSNPMTLSEDEIARLKGINEDLSLEEVAEVYLPLSRLLNFYISSNLRRQAVLEQFLGTNGQRIPYIISIAGSVAVGKSTTARVLQALLSRWPEHRRVELITTDGFLHPNRVLKERGLMKKKGFPESYDMHRLMKFVKDLKSGVPNVTAPVYSHLIYDVIPDGDKTVVQPDILILEGLNVLQSGMDYPHDPHHVFVSDFVDFSIYVDAPEDLLQTWYINRFLKFREGAFTDPDSYFHGYAKLTKEEAIKTAMTIWKEMNHLNLKQNILPTRERASLILTKSANHIVEEVRLRK

SEQ ID NO: 215 - DNA, 948 bp, Artificial Sequence; identical to SEQ ID NO: 211
  Pantothenate Kinase from Escherichia coli variant

SEQ ID NO: 216 - protein, 316 aa, Artificial Sequence; identical to SEQ ID NO: 212
  Pantothenate Kinase from Escherichia coli variant

SEQ ID NO: 217 - DNA, 948 bp, Artificial Sequence
  Pantothenate Kinase from Escherichia coli variant
atgagcatcaaagagcagaccctgatgaccccgtacctgcagctggaccgtaaccaatgggcggcgctgcgtgatagtaacccgatgaccctgagcgaggacgaaatcgcgcgtctgaagggtattaacgaggatctgagcctggaggaagtggcggaagtctacctgccgctgagccgtctgctgaacttctatattagcagcaacctgcgtcgtcaggcggttctggaacagtttctgggtaccaacggccagcgtatcccgtatatcattagcattgcgggtagcgtggcggttggcaaaagcaccaccgcgcgtgtgctgcaggcgctgctgagccgttggccggagcatcgtcgtgttgaactgatctcgaccgacggcttcctgcacccgaaccaagtgctgaaggagcgtggtctgatgaagaaaaagggtttcccggaaagctacgatatgcaccgtctgatgaaatttgttaaagacctgaagagcggtgtgccgaacgttaccgcgccggtgtacagccacctgatctatgatgttattccggacggcgataaaaccgtggttcagccggacatcctgattctggagggtctgaacgtgctgcaaagcggcatggactatccgcacgatccgcaccacgtgtttgttagcgacttcgtggattttagcatctacgttgacgcgccggaggatctgctgcagacctggtacattaaccgtttcctgaaatttcgtgagggtgcgttcaccgacccggatagctactttcacgggtatgcgaaactgaccaaggaagaggcgatcaaaaccgcgatgaccatttggaaggagatgaaccacctgaacctgaagcaaaacattctgccgacccgtgaacgtgcgagcctgattctgaccaaaagcgcaaaccacatcgtggaggaagttcgtctgcgtaag

SEQ ID NO: 218 - protein, 316 aa, Artificial Sequence
  Pantothenate Kinase from Escherichia coli variant
MSIKEQTLMTPYLQLDRNQWAALRDSNPMTLSEDEIARLKGINEDLSLEEVAEVYLPLSRLLNFYISSNLRRQAVLEQFLGTNGQRIPYIISIAGSVAVGKSTTARVLQALLSRWPEHRRVELISTDGFLHPNQVLKERGLMKKKGFPESYDMHRLMKFVKDLKSGVPNVTAPVYSHLIYDVIPDGDKTVVQPDILILEGLNVLQSGMDYPHDPHHVFVSDFVDFSIYVDAPEDLLQTWYINRFLKFREGAFTDPDSYFHGYAKLTKEEAIKTAMTIWKEMNHLNLKQNILPTRERASLILTKSANHIVEEVRLRK

SEQ ID NO: 219 - DNA, 948 bp, Artificial Sequence
  Pantothenate Kinase from Escherichia coli variant
atgagcatcaaagagcagaccctgatgaccccgtacctgcagctggaccgtaaccaatgggcggcgctgcgtgatagtaacccgatgaccctgagcgaggacgaaatcgcgcgtctgaagggtattaacgaggatctgagcctggaggaagtggcggaagtctacctgccgctgagccgtctgctgaacttctatattagcagcaacctgcgtcgtcaggcggttctggaacagtttctgggtaccaacggccagcgtatcccgtatatcattagcattgcgggtagcgtggcggttggcaaaagcaccaccgcgcgtgtgctgcaggcgctgctgagccgttggccggagcatcgtcgtgttgaactgatcggtaccgacggcttcctgcacccgaaccaagtgctgaaggagcgtggtctgatgaagaaaaagggtttcccggaaagctacgatatgcaccgtctgatgaaatttgttaaagacctgaagagcggtgtgccgaacgttaccgcgccggtgtacagccacctgatctatgatgttattccggacggcgataaaaccgtggttcagccggacatcctgattctggagggtctgaacgtgctgcaaagcggcatggactatccgcacgatccgcaccacgtgtttgttagcgacttcgtggattttagcatctacgttgacgcgccggaggatctgctgcagacctggtacattaaccgtttcctgaaatttcgtgagggtgcgttcaccgacccggatagctactttcacgggtatgcgaaactgaccaaggaagaggcgatcaaaaccgcgatgaccatttggaaggagatgaaccacctgaacctgaagcaaaacattctgccgacccgtgaacgtgcgagcctgattctgaccaaaagcgcaaaccacatcgtggaggaagttcgtctgcgtaag

SEQ ID NO: 220 - protein, 316 aa, Artificial Sequence
  Pantothenate Kinase from Escherichia coli variant
MSIKEQTLMTPYLQLDRNQWAALRDSNPMTLSEDEIARLKGINEDLSLEEVAEVYLPLSRLLNFYISSNLRRQAVLEQFLGTNGQRIPYIISIAGSVAVGKSTTARVLQALLSRWPEHRRVELIGTDGFLHPNQVLKERGLMKKKGFPESYDMHRLMKFVKDLKSGVPNVTAPVYSHLIYDVIPDGDKTVVQPDILILEGLNVLQSGMDYPHDPHHVFVSDFVDFSIYVDAPEDLLQTWYINRFLKFREGAFTDPDSYFHGYAKLTKEEAIKTAMTIWKEMNHLNLKQNILPTRERASLILTKSANHIVEEVRLRK

SEQ ID NO: 221 - DNA, 948 bp, Artificial Sequence
  Pantothenate Kinase from Escherichia coli variant
atgagcatcaaagagcagaccctgatgaccccgtacctgcagctggaccgtaaccaatgggcggcgctgcgtgatagtaacccgatgaccctgagcgaggacgaaatcgcgcgtctgaagggtattaacgaggatctgagcctggaggaagtggcggaagtctacctgccgctgagccgtctgctgaacttctatattagcagcaacctgcgtcgtcaggcggttctggaacagtttctgggtaccaacggccagcgtatcccgtatatcattagcattgcgggtagcgtggcggttggcaaaagcaccaccgcgcgtgtgctgcaggcgctgctgagccgttggccggagcatcgtcgtgttgaacatatcaccaccgacggcttcctgcacccgaaccaagtgctgaaggagcgtggtctgatgaagaaaaagggtttcccggaaagctacgatatgcaccgtctgatgaaatttgttaaagacctgaagagcggtgtgccgaacgttaccgcgccggtgtacagccacctgatctatgatgttattccggacggcgataaaaccgtggttcagccggacatcctgattctggagggtctgaacgtgctgcaaagcggcatggactatccgcacgatccgcaccacgtgtttgttagcgacttcgtggattttagcatctacgttgacgcgccggaggatctgctgcagacctggtacattaaccgtttcctgaaatttcgtgagggtgcgttcaccgacccggatagctactttcacgggtatgcgaaactgaccaaggaagaggcgatcaaaaccgcgatgaccatttggaaggagatgaaccacctgaacctgaagcaaaacattctgccgacccgtgaacgtgcgagcctgattctgaccaaaagcgcaaaccacatcgtggaggaagttcgtctgcgtaag

SEQ ID NO: 222 - protein, 316 aa, Artificial Sequence
  Pantothenate Kinase from Escherichia coli variant
MSIKEQTLMTPYLQLDRNQWAALRDSNPMTLSEDEIARLKGINEDLSLEEVAEVYLPLSRLLNFYISSNLRRQAVLEQFLGTNGQRIPYIISIAGSVAVGKSTTARVLQALLSRWPEHRRVEHITTDGFLHPNQVLKERGLMKKKGFPESYDMHRLMKFVKDLKSGVPNVTAPVYSHLIYDVIPDGDKTVVQPDILILEGLNVLQSGMDYPHDPHHVFVSDFVDFSIYVDAPEDLLQTWYINRFLKFREGAFTDPDSYFHGYAKLTKEEAIKTAMTIWKEMNHLNLKQNILPTRERASLILTKSANHIVEEVRLRK

SEQ ID NO: 223 - DNA, 948 bp, Artificial Sequence
  Pantothenate Kinase from Escherichia coli variant
atgagcatcaaagagcagaccctgatgaccccgtacctgcagctggaccgtaaccaatgggcggcgctgcgtgatagtaacccgatgaccctgagcgaggacgaaatcgcgcgtctgaagggtattaacgaggatctgagcctggaggaagtggcggaagtctacctgccgctgagccgtctgctgaacttctatattagcagcaacctgcagcgtcaggcggttctggaacagtttctgggtaccaacggccagcgtatcccgtatatcattagcattgcgggtagcgtggcggttggcaaaagcaccaccgcgcgtgtgctgcaggcgctgctgagccgttggccggagcatcgtcgtgttgaactgatcaccaccgacggcttcctgcacccgaaccaagtgctgaaggagcgtggtctgatgaagaaaaagggtttcccggaaagctacgatatgcaccgtctgatgaaatttgttaaagacctgaagagcggtgtgccgaacgttaccgcgccggtgtacagccacctgatctatgatgttattccggacggcgataaaaccgtggttcagccggacatcctgattctggagggtctgaacgtgctgcaaagcggcatggactatccgcacgatccgcaccacgtgtttgttagcgacttcgtggattttagcatctacgttgacgcgccggaggatctgctgcagacctggtacattaaccgtttcctgaaatttcgtgagggtgcgttcaccgacccggatagctactttcacgggtatgcgaaactgaccaaggaagaggcgatcaaaaccgcgatgaccatttggaaggagatgaaccacctgaacctgaagcaaaacattctgccgacccgtgaacgtgcgagcctgattctgaccaaaagcgcaaaccacatcgtggaggaagttcgtctgcgtaag

SEQ ID NO: 224 - protein, 316 aa, Artificial Sequence
  Pantothenate Kinase from Escherichia coli variant
MSIKEQTLMTPYLQLDRNQWAALRDSNPMTLSEDEIARLKGINEDLSLEEVAEVYLPLSRLLNFYISSNLQRQAVLEQFLGTNGQRIPYIISIAGSVAVGKSTTARVLQALLSRWPEHRRVELITTDGFLHPNQVLKERGLMKKKGFPESYDMHRLMKFVKDLKSGVPNVTAPVYSHLIYDVIPDGDKTVVQPDILILEGLNVLQSGMDYPHDPHHVFVSDFVDFSIYVDAPEDLLQTWYINRFLKFREGAFTDPDSYFHGYAKLTKEEAIKTAMTIWKEMNHLNLKQNILPTRERASLILTKSANHIVEEVRLRK

SEQ ID NO: 225 - DNA, 948 bp, Artificial Sequence
  Pantothenate Kinase from Escherichia coli variant
atgagcatcaaagagcagaccctgatgaccccgtacctgcagctggaccgtaaccaatgggcggcgctggctgatagtaacccgatgaccctgagcgaggacgaaatcgcgcgtctgaagggtattaacgaggatctgagcatggaggaagtggcggaagtctacctgccgctgagccgtctgctgaacttctatattagcagcaacctgcgtcgtcaggcggttctggaacagtttctgggtaccaacggccagcgtatcccgtatatcattagcattgcgggtagcgtggcggttggcaaaagcaccaccgcgcgtgtgctgcaggcgctgctgagccgttggccggagcatcgtcgtgttgaactgatcaccaccgacggcttcctgcacccgaaccaagtgctgaaggagcgtggtctgatgaagaaaaagggtttcccggaaagctacgatatgcaccgtctgatgaaatttgttaaagacctgaagagcggtgtgccgaacgttaccgcgccggtgtacagccacctgatctatgatgttattccggacggcgataaaaccgtggttcagccggacatcctgattctggagggtctgaacgtgctgcaaagcggcatggactatccgcacgatccgcaccacgtgtttgttagcgacttcgtggattttagcatctacgttgacgcgccggaggatctgctgcagacctggtacattaaccgtttcctgaaatttcgtgagggtgcgttcaccgacccggatagctactttcacgggtatgcgaaactgaccaaggaagaggcgatcaaaaccgcgatgaccatttggaaggagatgaaccacctgaacctgaagcaaaacattctgccgacccgtgaacgtgcgagcctgattctgaccaaaagcgcaaaccacatcgtggaggaagttcgtctgcgtaag

SEQ ID NO: 226 - protein, 316 aa, Artificial Sequence
  Pantothenate Kinase from Escherichia coli variant
MSIKEQTLMTPYLQLDRNQWAALADSNPMTLSEDEIARLKGINEDLSMEEVAEVYLPLSRLLNFYISSNLRRQAVLEQFLGTNGQRIPYIISIAGSVAVGKSTTARVLQALLSRWPEHRRVELITTDGFLHPNQVLKERGLMKKKGFPESYDMHRLMKFVKDLKSGVPNVTAPVYSHLIYDVIPDGDKTVVQPDILILEGLNVLQSGMDYPHDPHHVFVSDFVDFSIYVDAPEDLLQTWYINRFLKFREGAFTDPDSYFHGYAKLTKEEAIKTAMTIWKEMNHLNLKQNILPTRERASLILTKSANHIVEEVRLRK

SEQ ID NO: 227 - DNA, 948 bp, Artificial Sequence
  Pantothenate Kinase from Escherichia coli variant
atgagcatcaaagagcagaccctgatgaccccgtacctgcagctggaccgtaaccaatgggcggcgctgcgtgatagtaacccgatgaccctgagcgaggacgaaatcgcgcgtctgaagggtattaacgaggatctgagcctggaggaagtggcggaagtctacctgccgctgagccgtctgctgaacttctatattagcagcaacctgcgtcgtcaggcggttctggaacagtttctgggtaccaacggccagcgtatcccgtatatcattggtattgcgggtagcgtggcggttggcaaaagcaccaccgcgcgtgtgctgcaggcgctgctgagccgttggccggagcatcgtcgtgttgaactgatcaccaccgacggcttcctgcacccgaaccaagtgctgaaggagcgtggtctgatgaagaaaaagggtttcccggaaagctacgatatgcaccgtctgatgaaatttgttaaagacctgaagagcggtgtgccgaacgttaccgcgccggtgtacagccacctgatctatgatgttattccggacggcgataaaaccgtggttcagccggacatcctgattctggagggtctgaacgtgctgcaaagcggcatggactatccgcacgatccgcaccacgtgtttgttagcgacttcgtggattttagcatctacgttgacgcgccggaggatctgctgcagacctggtacattaaccgtttcctgaaatttcgtgagggtgcgttcaccgacccggatagctactttcacgggtatgcgaaactgaccaaggaagaggcgatcaaaaccgcgatgaccatttggaaggagatgaaccacctgaacctgaagcaaaacattctgccgacccgtgaacgtgcgagcctgattatgaccaaaagcgcaaaccacatcgtggaggaagttcgtctgcgtaag

SEQ ID NO: 228 - protein, 316 aa, Artificial Sequence
  Pantothenate Kinase from Escherichia coli variant
MSIKEQTLMTPYLQLDRNQWAALRDSNPMTLSEDEIARLKGINEDLSLEEVAEVYLPLSRLLNFYISSNLRRQAVLEQFLGTNGQRIPYIIGIAGSVAVGKSTTARVLQALLSRWPEHRRVELITTDGFLHPNQVLKERGLMKKKGFPESYDMHRLMKFVKDLKSGVPNVTAPVYSHLIYDVIPDGDKTVVQPDILILEGLNVLQSGMDYPHDPHHVFVSDFVDFSIYVDAPEDLLQTWYINRFLKFREGAFTDPDSYFHGYAKLTKEEAIKTAMTIWKEMNHLNLKQNILPTRERASLIMTKSANHIVEEVRLRK

SEQ ID NO: 229 - DNA, 948 bp, Artificial Sequence
  Pantothenate Kinase from Escherichia coli variant
atgagcatcaaagagcagaccctgatgaccccgtacctgcagctggaccgtaaccaatgggcggcgctgcgtgatagtaacccgatgaccctgagcgaggacgaaatcgcgcgtctgaagggtattaacgaggatctgagcctggaggaagtggcggaagtctacctgccgctgagccgtctgctgaacttctatattagcagcaacctgcgtcgtcaggcggttctggaacagtttctgggtaccaacggccagcgtatcccgtatatcattagcattgcgggtagcgtggcggttggcaaaagcaccaccgcgcgtgtgctgcaggcgctgctgagccgttggccggagcatcgtcgtgttgaacatatcaccaccgacggcttcctgcacccgaaccaagtgctgaaggagcgtggtctgatggggaaaaagggtttcccggaaagctacgatatgcaccgtctgatgaaatttgttaaagacctgaagagcggtgtgccgaacgttaccgcgccggtgtacagccacctgatctatgatgttattccggacggcgataaaaccgtggttcagccggacatcctgattctggagggtctgaacgtgctgcaaagcggcatggactatccgcacgatccgcaccacgtgtttgttagcgacttcgtggattttagcatctacgttgacgcgccggaggatctgctgcagacctggtacattaaccgtttcctgaaatttcgtgagggtgcgttcaccgacccggatagctactttcacgggtatgcgaaactgaccaaggaagaggcgatcaaaaccgcgatgaccatttggaaggagatgaaccacctgaacctgaagcaaaacattctgccgacccgtgaacgtgcgagcctgattctgaccaaaagcgcaaaccacatcgtggaggaagttcgtctgcgtaag

SEQ ID NO: 230 - protein, 316 aa, Artificial Sequence
  Pantothenate Kinase from Escherichia coli variant
MSIKEQTLMTPYLQLDRNQWAALRDSNPMTLSEDEIARLKGINEDLSLEEVAEVYLPLSRLLNFYISSNLRRQAVLEQFLGTNGQRIPYIISIAGSVAVGKSTTARVLQALLSRWPEHRRVEHITTDGFLHPNQVLKERGLMGKKGFPESYDMHRLMKFVKDLKSGVPNVTAPVYSHLIYDVIPDGDKTVVQPDILILEGLNVLQSGMDYPHDPHHVFVSDFVDFSIYVDAPEDLLQTWYINRFLKFREGAFTDPDSYFHGYAKLTKEEAIKTAMTIWKEMNHLNLKQNILPTRERASLILTKSANHIVEEVRLRK

SEQ ID NO: 231 - DNA, 948 bp, Artificial Sequence
  Pantothenate Kinase from Escherichia coli variant
atgagcatcaaagagcagaccctgatgaccccgtacctgcagctggaccgtaaccaatgggcggcgctgcgtgatagtaacccgatgaccctgagcgaggacgaaatcgcgcgtctgaagggtattaacgaggatctgagcctggaggaagtggcggaagtctacctgccgctgagccgtctgctgaacttctatattagcagcaacctgcgtcgtcaggcggttctggaacagtttctgggtaccaacggccagcgtatcccgtatatcattagcattgcgggtagcgtggcggttggcaaaagcaccaccgcgcgtgtgctgcaggcgctgctgagccgttggccggagcatcgtcgtgttgaacatatcaccaccgacggcttcctgcacccgaaccaagtgctgaaggagcgtggtctgatgaagaaaaagggtttcccggaaagctacgatatgcctcgtctgatgaaatttgttaaagacctgaagagcggtgtgccgaacgttaccgcgccggtgtacagccacctgatctatgatgttattccggacggcgataaaaccgtggttcagccggacatcctgattctggagggtctgaacgtgctgcaaagcggcatggactatccgcacgatccgcaccacgtgtttgttagcgacttcgtggattttagcatctacgttgacgcgccggaggatctgctgcagacctggtacattaaccgtttcctgaaatttcgtgagggtgcgttcaccgacccggatagctactttcacgggtatgcgaaactgaccaaggaagaggcgatcaaaaccgcgatgaccatttggaaggagatgaaccacctgaacctgaagcaaaacattctgccgacccgtgaacgtgcgagcctgattctgaccaaaagcgcaaaccacatcgtggaggaagttcgtctgcgtaag

SEQ ID NO: 232 - protein, 316 aa, Artificial Sequence
  Pantothenate Kinase from Escherichia coli variant
MSIKEQTLMTPYLQLDRNQWAALRDSNPMTLSEDEIARLKGINEDLSLEEVAEVYLPLSRLLNFYISSNLRRQAVLEQFLGTNGQRIPYIISIAGSVAVGKSTTARVLQALLSRWPEHRRVEHITTDGFLHPNQVLKERGLMKKKGFPESYDMPRLMKFVKDLKSGVPNVTAPVYSHLIYDVIPDGDKTVVQPDILILEGLNVLQSGMDYPHDPHHVFVSDFVDFSIYVDAPEDLLQTWYINRFLKFREGAFTDPDSYFHGYAKLTKEEAIKTAMTIWKEMNHLNLKQNILPTRERASLILTKSANHIVEEVRLRK

SEQ ID NO: 233 - DNA, 948 bp, Artificial Sequence
  Pantothenate Kinase from Escherichia coli variant
atgagcatcaaagagcagaccctgatgaccccgtacctgcagctggaccgtaaccaatgggcggcgctgcgtgatagtaacccgatgaccctgagcgaggacgaaatcgcgcgtctgaagggtattaacgaggatctgagcctggaggaagtggcggaagtctacctgccgctgagccgtctgctgaacttctatattagcagcaacctgcgtcgtcaggcggttctggaacagtttctgggtaccccacaccagcgtatcccgtatatcattagcattgcgggtagcgtggcggttggcaaaagcaccaccgcgcgtgtgctgcaggcgctgctgagccgttggccggagcatcgtcgtgttgaacacatcaccaccgacggcttcctgcacccgaaccaagtgctgaaggagcgtggtctgatgaagaaaaagggtttcccggaaagctacgatatgcaccgtctgatgaaatttgttaaagacctgaagagcggtgtgccgaacgttaccgcgccggtgtacagccacctgatctatgatgttattccggacggcgataaaaccgtggttcagccggacatcctgattctggagggtctgaacgtgctgcaaagcggcatggactatccgcacgatccgcaccacgtgtttgttagcgacttcgtggattttagcatctacgttgacgcgccggaggatctgctgcagacctggtacattaaccgtttcctgaaatttcgtgagggtgcgttcaccgacccggatagctactttcacgggtatgcgaaactgaccaaggaagaggcgatcaaaaccgcgatgaccatttggaaggagatgaaccacctgaacctgaagcaaaacattctgccgacccgtgaacgtgcgagcctgattctgaccaaaagcaccaaccacatcgtggaggaagttcgtctgcgtaag

SEQ ID NO: 234 - protein, 316 aa, Artificial Sequence
  Pantothenate Kinase from Escherichia coli variant
MSIKEQTLMTPYLQLDRNQWAALRDSNPMTLSEDEIARLKGINEDLSLEEVAEVYLPLSRLLNFYISSNLRRQAVLEQFLGTPHQRIPYIISIAGSVAVGKSTTARVLQALLSRWPEHRRVEHITTDGFLHPNQVLKERGLMKKKGFPESYDMHRLMKFVKDLKSGVPNVTAPVYSHLIYDVIPDGDKTVVQPDILILEGLNVLQSGMDYPHDPHHVFVSDFVDFSIYVDAPEDLLQTWYINRFLKFREGAFTDPDSYFHGYAKLTKEEAIKTAMTIWKEMNHLNLKQNILPTRERASLILTKSTNHIVEEVRLRK

SEQ ID NO: 235 - DNA, 948 bp, Artificial Sequence
  Pantothenate Kinase from Escherichia coli
atgagcatcaaagagcagaccctgatgaccccgtaccatcagctggaccgtaaccaatgggcggcgctgcgcgatagtaacccgatgaccctgagcgaggacgaaatcgcgcgtctgaagggtattaacgaggatctgagcctggaggaagtggcggaagtctacctgccgctgagccgtctgctgaacttctatatttcgagcaacctgcgtcgtcaggcggttctggaacagtttctgggtaccaacggccagcgtatcccgtatatcattagcattgcgggtagcgtggcggttggcaaaagcaccaccgcgcgtgtgctgcaggcgctgctgagccgttggccggagcatcgtcgtgttgaacatatcaccaccgacggcttcctgcacccgaaccaagtgctgaaggagcgtggtctgatggggaaaaagggtttcccggaaagctacgatatgcaccgtctgatgaaatttgttaaagacctgaagagcggtgtgccgagcgttaccgcgccggtgtacagccacctgatctatgatgttattccggacggcgataaaaccgtggttcagccggacatcctgattctggagggtctgaacgtgctgcaaagcggcatggactatccgcacgagccgcaccacgtgtttgttagcgacttcgtggattttagcatctacgttgacgcgccggaggatctgctgcagacctggtacattaaccgtttcctgaaactgcgtgagggtgcgttcaccgacccggatagctactttcacgggtatgcgaaactgaccaaggaagaggcgatcaaaaccgcgatgaccatttggaaggagatgaacagcctgaacctgaagacgaacattctgccgacccgtgaacgtgcgagcctgattctgaccaaaagcgcaaaccacatcgtggaggaagttcgtctgcgtaag

SEQ ID NO: 236 - protein, 316 aa, Artificial Sequence
  Pantothenate Kinase from Escherichia coli
MSIKEQTLMTPYHQLDRNQWAALRDSNPMTLSEDEIARLKGINEDLSLEEVAEVYLPLSRLLNFYISSNLRRQAVLEQFLGTNGQRIPYIISIAGSVAVGKSTTARVLQALLSRWPEHRRVEHITTDGFLHPNQVLKERGLMGKKGFPESYDMHRLMKFVKDLKSGVPSVTAPVYSHLIYDVIPDGDKTVVQPDILILEGLNVLQSGMDYPHEPHHVFVSDFVDFSIYVDAPEDLLQTWYINRFLKLREGAFTDPDSYFHGYAKLTKEEAIKTAMTIWKEMNSLNLKTNILPTRERASLILTKSANHIVEEVRLRK

SEQ ID NO: 237 - DNA, 948 bp, Artificial Sequence
  Pantothenate Kinase from Escherichia coli
atgagcatcaaagagcagaccctgatgaccccgtacctgcagctggaccgtaaccaatgggcggcgctgcgcgatagtaacccgatgaccctgagcgaggacgaaatcgcgcgtctgaagggtattaacgaggatctgagcctggatgaagtggcggaagtctacctgccgctgagccgtctgctgaacttctatattagcagcaacctgcgtcgtcaggcggttctggaacagtttctgggtaccaacggccagcgtatcccgtatatcattagcattgcgggtagcgtggcggttggcaaaagcaccaccgcgcgtgtgctgcaggcgctgctgagccgttggccggagcatcgtcgtgttgaacatatcaccaccgacggcttcctgcacccgaaccaagtgctgaaggagcgtggtctgatggggaaaaagggtttcccggaaagctacgatatgcaccgtctgatgaaatttgttaaagacctgaagagcggtgtgccgaacgttaccgcgccggtgtacagccacctgatctatgatgttattccggacggcgataaaaccgtggttcagccggacatcctgattctggagggtctgaacgtgctgcaaagcggcatggactatccgcacgatccgcaccacgtgtttgttagcgacttcgtggattttagcatctacgttgacgcgccggaggatctgctgcagacctggtacattaaccgtttcctgaaactgcgtgagggtgcgttcaccgacccggatagctactttcacgggtatgcgaaactgaccaaggaagaggcgatcaaaaccgcgatgaccatttggaaggagatgaaccacctgaacctgaagcaaaacattctgccgacccgtgaacgtgcgagcctgattctgaccaaaagcgcaaaccacatcgtggaggaagttcgtctgcgtaag

SEQ ID NO: 238 - protein, 316 aa, Artificial Sequence
  Pantothenate Kinase from Escherichia coli
MSIKEQTLMTPYLQLDRNQWAALRDSNPMTLSEDEIARLKGINEDLSLDEVAEVYLPLSRLLNFYISSNLRRQAVLEQFLGTNGQRIPYIISIAGSVAVGKSTTARVLQALLSRWPEHRRVEHITTDGFLHPNQVLKERGLMGKKGFPESYDMHRLMKFVKDLKSGVPNVTAPVYSHLIYDVIPDGDKTVVQPDILILEGLNVLQSGMDYPHDPHHVFVSDFVDFSIYVDAPEDLLQTWYINRFLKLREGAFTDPDSYFHGYAKLTKEEAIKTAMTIWKEMNHLNLKQNILPTRERASLILTKSANHIVEEVRLRK

SEQ ID NO: 239 - DNA, 948 bp, Artificial Sequence
  Pantothenate Kinase from Escherichia coli
atgagcatcaaagagcagaccctgatgaccccgtacctgcagctggaccgtaaccaatgggcggcgctgcgtgatagtaacccgatgaccctgagcgaggacgaaatcgcgcgtctgaagggtattaacgaagatctgagcctggaggaagtggcggaagtctacctgccgctgagccgtctgctgaacttctatattagcagcaacctgcgtcgtcaggcgcagctggaacagtttctgggtaccaatggccagcgtatcccgtatatcattagcattgcgggtagcgtggcggttggcaaaagcacctttgcgcgtgtgctgcaggcgctgctgagccgttggccggagcatcgtcgtgttgaacatatcaccaccgacggcttcctgcacccgaaccaagtgctgaaggagcgtggtctgatggggaaaaagggtttcccggaaagctacgatatgcaccgtctgatgaaatttgttaaagacctgaagagcggtgtgccgaacgttaccgcgccggtgtacagccacctgatctatgatgttattccggacggcgataaaaccgtggttcagccggacatcctgattctggagggtctgaacgtgctgcaaagcggcatggactatccgcacgatccgcaccacgtgtttgttagcgacttcgtggattttagcatctacgttgacgcgccggaggatctgctgcagacctggtacattaaccgtttcctgaaatttcgtgagggtgcgttcaccgacccggatagctactttcacgggtatgcgaaactgaccaaggaagaggcgatcaaaaccgcgatgaccatttggaaggagatgaaccacgtgaacctgaagcaaaacattctgccgacccgtgaacgtgcgagcctgattctgaccaaaagcgcaaaccacatcgtggaggaagttcgtctgcgtaag

SEQ ID NO: 240 - protein, 316 aa, Artificial Sequence
  Pantothenate Kinase from Escherichia coli
MSIKEQTLMTPYLQLDRNQWAALRDSNPMTLSEDEIARLKGINEDLSLEEVAEVYLPLSRLLNFYISSNLRRQAQLEQFLGTNGQRIPYIISIAGSVAVGKSTFARVLQALLSRWPEHRRVEHITTDGFLHPNQVLKERGLMGKKGFPESYDMHRLMKFVKDLKSGVPNVTAPVYSHLIYDVIPDGDKTVVQPDILILEGLNVLQSGMDYPHDPHHVFVSDFVDFSIYVDAPEDLLQTWYINRFLKFREGAFTDPDSYFHGYAKLTKEEAIKTAMTIWKEMNHVNLKQNILPTRERASLILTKSANHIVEEVRLRK

SEQ ID NO: 241 - DNA, 948 bp, Artificial Sequence
  Pantothenate Kinase from Escherichia coli
atgagcatcaaagagcagaccctgatgaccccgtacctgcagctggaccgtaaccaatgggcggcgctgcgtgatagtaacccgatgaccctgagcgaggacgaaatcgcgcgtctgaagggtattaacgaggatctgagcctggaggaagtggcggaagtctacctgccgctgagccgtctgctgaacttctatatttcgagcaacctgcgtcgtcaggcggttctggaacagtttctgggtaccaacggccagcgtatcccgtatatcattagcattgcgggtagcgtggcggttggcaaaagcaccaccgcgcgtgtgctgcaggcgctgctgagccgttggccggagcatcgtcgtgttgaacatatcaccaccgacggcttcctgcacccgaaccaagtgctgaaggagcgtggtctgatggggaaaaagggtttcccggaaagctacgatatgcaccgtctgatgaaatttgttaaagacctgaagagcggtgtgccgagcgttaccgcgccggtgtacagccacctgatctatgatgttattccggacggcgataaaaccgtggttcagccggacatcctgattctggagggtctgaacgtgctgcaaagcggcatggactatccgcacgatccgcaccacgtgtttgttagcgacttcgtggattttagcatctacgttgacgcgccggaggatctgctgcagacctggtacattaaccgtttcctgaaactgcgtgagggtgcgttcaccgacccggatagctactttcacgggtatgcgaaactgaccaaggaagaggcgatcaaaaccgcgatgaccatttggaaggagatgaaccacctgaacctgaagcaaaacattctgccgacccgtgaacgtgcgagcctgattctgaccaaaagcgcaaaccacatcgtggaggaagttcgtctgcgtaag

SEQ ID NO: 242 - protein, 316 aa, Artificial Sequence
  Pantothenate Kinase from Escherichia coli
MSIKEQTLMTPYLQLDRNQWAALRDSNPMTLSEDEIARLKGINEDLSLEEVAEVYLPLSRLLNFYISSNLRRQAVLEQFLGTNGQRIPYIISIAGSVAVGKSTTARVLQALLSRWPEHRRVEHITTDGFLHPNQVLKERGLMGKKGFPESYDMHRLMKFVKDLKSGVPSVTAPVYSHLIYDVIPDGDKTVVQPDILILEGLNVLQSGMDYPHDPHHVFVSDFVDFSIYVDAPEDLLQTWYINRFLKLREGAFTDPDSYFHGYAKLTKEEAIKTAMTIWKEMNHLNLKQNILPTRERASLILTKSANHIVEEVRLRK

SEQ ID NO: 243 - DNA, 948 bp, Artificial Sequence
  Pantothenate Kinase from Escherichia coli
atgagcatcaaagagcagaccctgatgaccccgtacctgcagctggaccgtaaccaatgggcggcgctgcgtgatagtaacccgatgaccctgagcgaggacgaaatcgcgcgtctgaagggtattaacgaggatctgagcctggaggaagtggcggaagtctacctgccgctgagccgtctgctgaacttctatattagcagcaacctgcgtcgtcaggcggttctggaacagtttctgggtaccaacggccagcgtatcccgtatatcattagcattgcgggtagcgtggcggttggcaaaagcaccaccgcgcgtgtgctgcaggcgctgctgagccgttggccggagcatcgtcgtgttgaacatatcaccaccgacggcttcctgcacccgaaccaagtgctgaaggagcgtggtctgatggggaaaaagggtttcccggaaagctacgatatgcaccgtctgatgaaatttgttaaagacctgaagagcggtgtgccgaacgttaccgcgccggtgtacagccacctgatctatgatgttattccggacggcgataaaaccgtggttcagccggacatcctgattctggagggtctgaacgtgctgcaaagcggcatggactatccgcacgatccgcaccacgtgtttgttagcgacttcgtggattttagcatctacgttgacgcgccggaggatctgctgcagacctggtacattaaccgtttcctgaaattgcgtgagggtgcgttcaccgacccggatagctactttcacgggtatgcgaaactgaccaaggaagaggcgatcaaaaccgcgatgaccatttggaaggagatgaaccacctgaacctgaagcaaaacattctgccgacccgtgaacgtgcgagcctgattctgaccaaaagcgcaaaccacatcgtggaggaagttcgtctgcgtaag

SEQ ID NO: 244 - protein, 316 aa, Artificial Sequence
  Pantothenate Kinase from Escherichia coli
MSIKEQTLMTPYLQLDRNQWAALRDSNPMTLSEDEIARLKGINEDLSLEEVAEVYLPLSRLLNFYISSNLRRQAVLEQFLGTNGQRIPYIISIAGSVAVGKSTTARVLQALLSRWPEHRRVEHITTDGFLHPNQVLKERGLMGKKGFPESYDMHRLMKFVKDLKSGVPNVTAPVYSHLIYDVIPDGDKTVVQPDILILEGLNVLQSGMDYPHDPHHVFVSDFVDFSIYVDAPEDLLQTWYINRFLKLREGAFTDPDSYFHGYAKLTKEEAIKTAMTIWKEMNHLNLKQNILPTRERASLILTKSANHIVEEVRLRK

SEQ ID NO: 245 - DNA, 948 bp, Artificial Sequence
  Pantothenate Kinase from Escherichia coli
atgagcatcaaagagcagaccctgatgaccccgtacctgcagctggaccgtaaccaatgggcggcgctgcgtgatagtaacccgatgaccctgagcgaggacgaaatcgcgcgtctgaagggtattaacgaggatctgagcctggaggaagtggcggaagtctacctgccgctgagccgtctgctgaacatttatattagcagcaacctgcgtcgtcaggcggttctggaacagtttctgggtaccaacggccagcgtatcccgtatatcattagcattgcgggtagcgtggcggttggcaaaagcacctttgcgcgtgtgctgcaggcgctgctgagccgttggccggagcatcgtcgtgttgaacatatcaccaccgacggcttcctgcacccgaaccaagtgctgaaggagcgtggtctgatggggaaaaagggtttcccggaaagctacgatatgcctcgtctgatgaaatttgttaaagacctgaagagcggtgtgccgaacgttaccgcgccggtgtacagccacctgatctatgatgttattccggacggcgataaaaccgtggttcagccggacatcctgattctggagggtctgaacgtgctgcaaagcggcatggactatccgcacgatccgcaccacgtgtttgttagcgacttcgtggattttagcatctacgttgacgcgccggaggatctgctgcagacctggtacattaaccgtttcctgaaatttcgtgagggtgcgttcaccgacccggatagctactttcacgggtatgcgaaactgaccaaggaagaggcgatcaaaaccgcgatgaccatttggaaggagatgaaccacgtgaacctgaagcaaaacattctgccgacccgtgaacgtgcgagcctgattctgaccaaaagcgcaaaccacatcgtggaggaagttcgtctgcgtaag

SEQ ID NO: 246 - protein, 316 aa, Artificial Sequence
  Pantothenate Kinase from Escherichia coli
MSIKEQTLMTPYLQLDRNQWAALRDSNPMTLSEDEIARLKGINEDLSLEEVAEVYLPLSRLLNIYISSNLRRQAVLEQFLGTNGQRIPYIISIAGSVAVGKSTFARVLQALLSRWPEHRRVEHITTDGFLHPNQVLKERGLMGKKGFPESYDMPRLMKFVKDLKSGVPNVTAPVYSHLIYDVIPDGDKTVVQPDILILEGLNVLQSGMDYPHDPHHVFVSDFVDFSIYVDAPEDLLQTWYINRFLKFREGAFTDPDSYFHGYAKLTKEEAIKTAMTIWKEMNHVNLKQNILPTRERASLILTKSANHIVEEVRLRK

SEQ ID NO: 247 - DNA, 948 bp, Artificial Sequence
  Pantothenate Kinase from Escherichia coli
atgagcatcaaagagcagaccctgatgaccccgtacctgcagctggagcgtaaccaatgggcggcgctgcgtgatagtaacccgatgaccctgagcgaggacgaaatcgcgcgtctgaagggtattaacgaggatctgagcctggaggaagtggcggaagtctacctgccgctgagccgtctgctgaacttctatattagcagcaacctgcgtcgtcaggcggttctggaacagtttctgggtaccaacggccagcgtatcccgtatatcattagcattgcgggtagcgtggcggttggcaaaagcaccaccgcgcgtgtgctgcaggcgctgctgagccgttggccggagcatcgtcgtgttgaacatatcaccaccgacggcttcctgcacccgaaccaagtgctgaaggagcgtggtctgatggggaaaaagggtttcccggaaagctacgatatgcaccgtctgatgaaatttgttaaagacctgaagagcggtgtgccgaacgttaccgcgccggtgtacagccacctgatctatgatgttattccggacggcgataaaaccgtggttcagccggacatcctgattctggagggtctgaacgtgctgcaaagcggcatggactatccgcacgatccgcaccacgtgtttgttagcgacttcgtggattttagcatctacgttgacgcgccggaggatctgctgcagacctggtacattaaccgtttcctgaaactgcgtgagggtgcgttcaccgacccggatagctactttcacgggtatgcgaaactgaccaaggaagaggcgatcaaaaccgcgatgaccatttggaaggagatgaaccacctgaacctgaagcaaaacattctgccgacccgtgaacgtgcgagcctgattctgaccaaaagcgcaaaccacatcgtggaggaagttcgtctgcgtaag

SEQ ID NO: 248 - protein, 316 aa, Artificial Sequence
  Pantothenate Kinase from Escherichia coli
MSIKEQTLMTPYLQLERNQWAALRDSNPMTLSEDEIARLKGINEDLSLEEVAEVYLPLSRLLNFYISSNLRRQAVLEQFLGTNGQRIPYIISIAGSVAVGKSTTARVLQALLSRWPEHRRVEHITTDGFLHPNQVLKERGLMGKKGFPESYDMHRLMKFVKDLKSGVPNVTAPVYSHLIYDVIPDGDKTVVQPDILILEGLNVLQSGMDYPHDPHHVFVSDFVDFSIYVDAPEDLLQTWYINRFLKLREGAFTDPDSYFHGYAKLTKEEAIKTAMTIWKEMNHLNLKQNILPTRERASLILTKSANHIVEEVRLRK

SEQ ID NO: 249 - DNA, 978 bp, Artificial Sequence
  Pantothenate Kinase from Escherichia coli
atgcaccatcatcatcatcatggcggtagcggcagcatcaaagagcagaccgagatgaccccgtacctgcaactggaccgtaaccaatgggcggcgctgcgtgatagtaacccgatgaccctgagcgaggacgaaatcgcgcgtctgaagggtattaacgaagatctgagcctggaggaagtggcggaagtctacctgccgctgagccgtctgctgaacatttatattagcagcaacctgcgtcgtcaggcgcagctggaacagtttctgggtaccaatggccagcgtatcccgtatatcattagcattgcgggtagcgtggcggttggcaaaagcacctttgcgcgtgtgctgcaggcgctgctgagccgttggccggagcatcgtcgtgttgaacatatcaccaccgacggcttcctgcacccgaaccaagtgctgaaggagcgtggtctgatggggaaaaagggtttcccggaaagctacgatatgcaccgtctgatgaaatttgttaaagacctgaagagcggtgtgccgaacgttaccgcgccggtgtacagccacctgatctatgatgttattccggacggcgataaaaccgtggttcagccggacatcctgattctggagggtctgaacgtgctgcaaagcggcatggactatccgcacgatccgcaccacgtgtttgttagcgacttcgtggattttagcatctacgttgacgcgccggaggatctgctgcagacctggtacattaaccgtttcctgaaactgcgtgagggtgcgttcaccgacccggatagctactttcacgggtatgcgaaactgaccaaggaagaggcgatcaaaaccgcgatgaccatttggaaggagatgaaccatgtgaacctgaagcaaaacattctgccgacccgtgaacgtgcgagcctgattctgaccaaaagcgcaaaccacatcgtggaggaagttcgtctgcgtaag

SEQ ID NO: 250 - protein, 326 aa, Artificial Sequence
  Pantothenate Kinase from Escherichia coli
MHHHHHHGGSGSIKEQTEMTPYLQLDRNQWAALRDSNPMTLSEDEIARLKGINEDLSLEEVAEVYLPLSRLLNIYISSNLRRQAQLEQFLGTNGQRIPYIISIAGSVAVGKSTFARVLQALLSRWPEHRRVEHITTDGFLHPNQVLKERGLMGKKGFPESYDMHRLMKFVKDLKSGVPNVTAPVYSHLIYDVIPDGDKTVVQPDILILEGLNVLQSGMDYPHDPHHVFVSDFVDFSIYVDAPEDLLQTWYINRFLKLREGAFTDPDSYFHGYAKLTKEEAIKTAMTIWKEMNHVNLKQNILPTRERASLILTKSANHIVEEVRLRK

SEQ ID NO: 251 - DNA, 978 bp, Artificial Sequence
  Pantothenate Kinase from Escherichia coli
atgcaccatcatcatcatcatggcggtagcggcagcatcaaagagcagaccgagatgaccccgtacctgcaactggaccgtaaccaatgggcggcgctgcgtgatagtaacccgatgaccctgagcgaggacgaaatcgcgcgtctgaagggtattaacgaagatctgagcctggaggaagtggcggaagtctacctgccgctgagccgtctgctgaacttctatattagcagcaacctgcgtcgtcaggcgcagctggaacagtttctgggtaccaatggccagcgtatcccgtatatcattagcattgcgggtagcgtggcggttggcaaaagcacctttgcgcgtgtgctgcaggcgctgctgagccgttggccggagcatcgtcgtgttgaacatatcaccaccgacggcttcctgcacccgaaccaagtgctgaaggagcgtggtctgatggggaaaaagggtttcccggaaagctacgatatgcaccgtctgatgaaatttgttaaagacctgaagagcggtgtgccgaacgttaccgcgccggtgtacagccacctgatctatgatgttattccggacggcgataaaaccgtggttcagccggacatcctgattctggagggtctgaacgtgctgcaaagcggcatggactatccgcacgatccgcaccacgtgtttgttagcgacttcgtggattttagcatctacgttgacgcgccggaggatctgctgcagacctggtacattaaccgtttcctgaaactgcgtgagggtgcgttcaccgacccggatagctactttcacgggtatgcgaaactgaccaaggaagaggcgatcaaaaccgcgatgaccatttggaaggagatgaacagcgtgaacctgaagcaaaacattctgccgacccgtgaacgtgcgagcctgattctgaccaaaagcgcaaaccacatcgtggaggaagttcgtctgcgtaag

SEQ ID NO: 252 - protein, 326 aa, Artificial Sequence
  Pantothenate Kinase from Escherichia coli
MHHHHHHGGSGSIKEQTEMTPYLQLDRNQWAALRDSNPMTLSEDEIARLKGINEDLSLEEVAEVYLPLSRLLNFYISSNLRRQAQLEQFLGTNGQRIPYIISIAGSVAVGKSTFARVLQALLSRWPEHRRVEHITTDGFLHPNQVLKERGLMGKKGFPESYDMHRLMKFVKDLKSGVPNVTAPVYSHLIYDVIPDGDKTVVQPDILILEGLNVLQSGMDYPHDPHHVFVSDFVDFSIYVDAPEDLLQTWYINRFLKLREGAFTDPDSYFHGYAKLTKEEAIKTAMTIWKEMNSVNLKQNILPTRERASLILTKSANHIVEEVRLRK

SEQ ID NO: 253 - DNA, 978 bp, Artificial Sequence
  Pantothenate Kinase from Escherichia coli
atgcaccatcatcatcatcatggcggtagcggcagcatcaaagagcagaccgagatgaccccgtaccatgcgctggaccgtaaccaatgggcggcgctgcgtgatagtaacccgatgaccctgagcgaggacgaaatcgcgcgtctgaagggtattaacgaagatctgagcctggaggaagtggcggaagtctacctgccgctgagccgtctgctgaacttctatattagcagcaacctgcgtcgtcaggcgcagctggaacagtttctgggtacccctggccagcgtatcccgtatatcattagcattgcgggtagcgtggcggttggcaaaagcacctttgcgcgtgtgctgcaggcgctgctgagccgttggccggagcatcgtcgtgttgaacatatcaccaccgacggcttcctgcacccgaaccaagtgctgaaggagcgtggtctgatggggaaaaagggtttcccggaaagctacgatatgcaccgtctgatgaaatttgttaaagacctgaagagcggtgtgccgaacgttaccgcgccggtgtacagccacctgatctatgatgttattccggacggcgataaaaccgtggttcagccggacatcctgattctggagggtctgaacgtgctgcaaagcggcatggactatccgcacgatccgcaccacgtgtttgttagcgacttcgtggattttagcatctacgttgacgcgccggaggatctgctgcagacctggtacattaaccgtttcctgaaactgcgtgagggtgcgttcaccgacccggatagctactttcacgggtatgcgaaactgaccaaggaagaggcgatcaaaaccgcgatgaccatttggaaggagatgaaccatgtgaacctgaagcaaaacattctgccgacccgtgaacgtgcgagcctgattctgaccaaaagcgcaaaccacatcgtggaggaagttcgtctgcgtaag

SEQ ID NO: 254 - protein, 326 aa, Artificial Sequence
  Pantothenate Kinase from Escherichia coli
MHHHHHHGGSGSIKEQTEMTPYHALDRNQWAALRDSNPMTLSEDEIARLKGINEDLSLEEVAEVYLPLSRLLNFYISSNLRRQAQLEQFLGTPGQRIPYIISIAGSVAVGKSTFARVLQALLSRWPEHRRVEHITTDGFLHPNQVLKERGLMGKKGFPESYDMHRLMKFVKDLKSGVPNVTAPVYSHLIYDVIPDGDKTVVQPDILILEGLNVLQSGMDYPHDPHHVFVSDFVDFSIYVDAPEDLLQTWYINRFLKLREGAFTDPDSYFHGYAKLTKEEAIKTAMTIWKEMNHVNLKQNILPTRERASLILTKSANHIVEEVRLRK

SEQ ID NO: 255 - DNA, 978 bp, Artificial Sequence
  Pantothenate Kinase from Escherichia coli
atgcaccatcatcatcatcatggcggtagcggcagcatcaaagagcagaccgagatgaccccgtacctgcaactggaccgtaaccaatgggcggcgctgcgtgatagtaacccgatgaccctgagcgaggacgaaatcgcgcgtctgaagggtattaacgaagatctgagcctggaggaagtggcggaagtctacctgccgctgagccgtctgctgaacatttatattagcagcaacctgcgtcgtcaggcgcagctggaacagtttctgggtaccaatggccagcgtatcccgtatatcattagcattgcgggtagcgtggcggttggcaaaagcacctttgcgcgtgtgctgcaggcgctgctgagccgttggccggagcatcgtcgtgttgaacatatcaccaccgacggcttcctgcacccgaaccaagtgctgaaggagcgtggtctgatggggaaaaagggtttcccggaaagctacgatatgcaccgtctgatgaaatttgttaaagacctgaagagcggtgtgccgaacgttaccgcgccggtgtacagccacctgatctatgatgttattccggacggcgataaaaccgtggttcagccggacatcctgattctggagggtctgaacgtgctgcaaagcggcatggactatccgcacgagccgcaccacgtgtttgttagcgacttcgtggattttagcatctacgttgacgcgccggaggatctgctgcagacctggtacattaaccgtttcctgaaactgcgtgagggtgcgttcaccgacccggatagctactttcacgggtatgcgaaactgaccaaggaagaggcgatcaaaaccgcgatgaccatttggaaggagatgaaccacgtgaacctgaagcaaaacattctgccgacccgtgaacgtgcgagcctgattctgaccaaaagcgcaaaccacatcgtggaggaagttcgtctgcgtaag

SEQ ID NO: 256 - protein, 326 aa, Artificial Sequence
  Pantothenate Kinase from Escherichia coli
MHHHHHHGGSGSIKEQTEMTPYLQLDRNQWAALRDSNPMTLSEDEIARLKGINEDLSLEEVAEVYLPLSRLLNIYISSNLRRQAQLEQFLGTNGQRIPYIISIAGSVAVGKSTFARVLQALLSRWPEHRRVEHITTDGFLHPNQVLKERGLMGKKGFPESYDMHRLMKFVKDLKSGVPNVTAPVYSHLIYDVIPDGDKTVVQPDILILEGLNVLQSGMDYPHEPHHVFVSDFVDFSIYVDAPEDLLQTWYINRFLKLREGAFTDPDSYFHGYAKLTKEEAIKTAMTIWKEMNHVNLKQNILPTRERASLILTKSANHIVEEVRLRK

SEQ ID NO: 257 - DNA, 978 bp, Artificial Sequence
  Pantothenate Kinase from Escherichia coli
atgcaccatcatcatcatcatggcggtagcggcagcatcaaagagcagaccctgatgaccccgtacctgcagctggaccgtaaccaatgggcggcgctgcgtgatagtaacccgatgaccctgagcgaggacgaaatcgcgcgtctgaagggtattaacgaagatctgagcctggaggaagtggcggaagtctacctgccgctgagccgtctgctgaacttctatattagcagcaacctgcgtcgtcaggcgcagctggaacagtttctgggtaccaatggccagcgtatcccgtatatcattagcattgcgggtagcgtggcggttggcaaaagcacctttgcgcgtgtgctgcaggcgctgctgagccgttggccggagcatcgtcgtgttgaacatatcaccaccgacggcttcctgcacccgaaccaagtgctgaaggagcgtggtctgatggggaaaaagggtttcccggaaagctacgatatgcaccgtctgatgaaatttgttaaagacctgaagagcggtgtgccgaatgttaccgcgccggtgtacagccacctgatctatgatgttattccggacggcgataaaaccgtggtgcagccggacatcctgattctggagggtctgaacgtgctgcaaagcggcatggactatccgcacgatccgcaccacgtgtttgttagcgacttcgtggattttagcatctacgttgacgcgccggaggatctgctgcagacctggtacattaaccgtttcctgaaatttcgtgagggtgcgttcaccgacccggatagctactttcacgggtatgcgcgtctgaccaaggaagaggcgatcaaaaccgcgatgagtatttggaaggagatgaaccacgtgaacctgaagcaaaacattctgccgacccgggaacgtgcgagcctgattctgaccaaaagcgcaaaccacatcgtggaggaagttcgtctgcgtaag

SEQ ID NO: 258 - protein, 326 aa, Artificial Sequence
  Pantothenate Kinase from Escherichia coli
MHHHHHHGGSGSIKEQTLMTPYLQLDRNQWAALRDSNPMTLSEDEIARLKGINEDLSLEEVAEVYLPLSRLLNFYISSNLRRQAQLEQFLGTNGQRIPYIISIAGSVAVGKSTFARVLQALLSRWPEHRRVEHITTDGFLHPNQVLKERGLMGKKGFPESYDMHRLMKFVKDLKSGVPNVTAPVYSHLIYDVIPDGDKTVVQPDILILEGLNVLQSGMDYPHDPHHVFVSDFVDFSIYVDAPEDLLQTWYINRFLKFREGAFTDPDSYFHGYARLTKEEAIKTAMSIWKEMNHVNLKQNILPTRERASLILTKSANHIVEEVRLRK

SEQ ID NO: 259 - DNA, 978 bp, Artificial Sequence
  Pantothenate Kinase from Escherichia coli
atgcaccatcatcatcatcatggcggtagcggcagcatcaaagagcagaccctgatgtcgccgtacctgcagctggaccgtaaccaatgggcggcgctgcgtgatagtaacccgatgaccctgagcgaggacgaaatcgcgcgtctgaagggtattaacgaagatctgagcctggaggaagtggcggaagtctacctgccgctgagccgtctgctgaacttctatattagcagcaacctgcgtcgtcaggcgcagctggaacagtttctgggtaccaatggccagcgtatcccgtatatcattagcattgcgggtagcgtggcggttggcaaaagcacctttgcgcgtgtgctgcaggcgctgctgagccgttggccggagcatcgtcgtgttgaacatatcaccaccgacggcttcctgcacccgaaccaagtgctgaaggagcgtggtctgatggggaaaaagggtttcccggaaagctacgatatgcaccgtctgatgaaatttgttaaagacctgaagagcggtgtgccgaacgttaccgcgccggtgtacagccacctgatctatgatgttattccggacggcgataaaaccgtggttcagccggacatcctgattctggagggtctgaacgtgctgcaaagcggcatggactatccgcacgatccgcaccacgtgtttgttagcgacttcgtggattttagcatctacgttgacgcgccggaggatctgctgcagacctggtacattaaccgtttcctgaaatttcgtgagggtgcgttcaccgacccggatagctactttcacgggtatgcgaaactgaccaaggaagaggcgatcaaaaccgcgatgaccatttggaaggagatgaaccacgtgaacctgaagcaaaacattctgccgacccgtgaacgtgcgagcctgattctgaccaaaagcgcaaaccacatcgtggaggaagttcgtctgcgtaag

SEQ ID NO: 260 - protein, 326 aa, Artificial Sequence
  Pantothenate Kinase from Escherichia coli
MHHHHHHGGSGSIKEQTLMSPYLQLDRNQWAALRDSNPMTLSEDEIARLKGINEDLSLEEVAEVYLPLSRLLNFYISSNLRRQAQLEQFLGTNGQRIPYIISIAGSVAVGKSTFARVLQALLSRWPEHRRVEHITTDGFLHPNQVLKERGLMGKKGFPESYDMHRLMKFVKDLKSGVPNVTAPVYSHLIYDVIPDGDKTVVQPDILILEGLNVLQSGMDYPHDPHHVFVSDFVDFSIYVDAPEDLLQTWYINRFLKFREGAFTDPDSYFHGYAKLTKEEAIKTAMTIWKEMNHVNLKQNILPTRERASLILTKSANHIVEEVRLRK

SEQ ID NO: 261 - DNA, 978 bp, Artificial Sequence
  Pantothenate Kinase from Escherichia coli
atgcaccatcatcatcatcatggcggtagcggcagcatcaaagagcagacctggatgaccccgtacctgcagctggaccgtaaccaatgggcggcgctgcgtgatagtaacccgatgaccctgagcgaggacgaaatcgcgcgtctgaagggtattaacgaagatctgagcctggaggaagtggcggaagtctacctgccgctgagccgtctgctgaacttctatattagcagcaacctgcgtcgtcaggcgcagctggaacagtttctgggtaccaatggccagcgtatcccgtatatcattagcattgcgggtagcgtggcggttggcaaaagcacctttgcgcgtgtgctgcaggcgctgctgagccgttggccggagcatcgtcgtgttgaacatatcaccaccgacggcttcctgcacccgaaccaagtgctgaaggagcgtggtctgatggggaaaaagggtttcccggaaagctacgatatgcaccgtctgatgaaatttgttaaagacctgaagagcggtgtgccgaacgttaccgcgccggtgtacagccacctgatctatgatgttattccggacggcgataaaaccgtggttcagccggacatcctgattctggagggtctgaacgtgctgcaaagcggcatggactatccgcacgatccgcaccacgtgtttgttagcgacttcgtggattttagcatctacgttgacgcgccggaggatctgctgcagacctggtacattaaccgtttcctgaaatttcgtgagggtgcgttcaccgacccggatagctactttcacgggtatgcgaaactgaccaaggaagaggcgatcaaaaccgcgatgaccatttggaaggagatgaaccacgtgaacctgaagcaaaacattctgccgacccgtgaacgtgcgagcctgattctgaccaaaagcgcaaaccacatcgtggaggaagttcgtctgcgtaag

SEQ ID NO: 262 - protein, 326 aa, Artificial Sequence
  Pantothenate Kinase from Escherichia coli
MHHHHHHGGSGSIKEQTWMTPYLQLDRNQWAALRDSNPMTLSEDEIARLKGINEDLSLEEVAEVYLPLSRLLNFYISSNLRRQAQLEQFLGTNGQRIPYIISIAGSVAVGKSTFARVLQALLSRWPEHRRVEHITTDGFLHPNQVLKERGLMGKKGFPESYDMHRLMKFVKDLKSGVPNVTAPVYSHLIYDVIPDGDKTVVQPDILILEGLNVLQSGMDYPHDPHHVFVSDFVDFSIYVDAPEDLLQTWYINRFLKFREGAFTDPDSYFHGYAKLTKEEAIKTAMTIWKEMNHVNLKQNILPTRERASLILTKSANHIVEEVRLRK

SEQ ID NO: 263 - DNA, 978 bp, Artificial Sequence
  Pantothenate Kinase from Escherichia coli
atgcaccatcatcatcatcatggcggtagcggcagcatcaaagagcagaccgagatgaccccgtacctgcaactggaccgtaaccaatgggcggcggtgcgtgatagtaacccgatgaccctgagcgaggacgaaatcgcgcgtctgaagggtattaacgaagatctgagcctggaggaagtggcggaagtctacctgccgctgagccgtattctgaacttctatattagcagcaacctgcgtcgtcaggcgcagctggaacagtttctgggtaccaatggccagcgtatcccgtatatcattagcattgcgggtagcgtggcggttggcaaaagcacctttgcgcgtgtgctgcaggcgctgctgagccgttggccggagcatcgtcgtgttgaacatatcaccaccgacggcttcctgcacccgaaccaagtgctgaaggagcgtggtctgatggggaaaaagggtttcccggaaagctacgatatgcaccgtctgatgaaatttgttaaagacctgaagagcggtgtgccgaacgttaccgcgccggtgtacagccacctgatctatgatgttattccggacggcgataaaaccgtggttcagccggacatcctgattctggagggtctgaacgtgctgcaaagcggcatggactatccgcacgatccgcaccacgtgtttgttagcgacttcgtggattttagcatctacgttgacgcgccggaggatctgctgcagacctggtacattaaccgtttcctgaaactgcgtgagggtgcgttcaccgacccggatagctactttcacgggtatgcgaaactgaccaaggaagaggcgatcaaaaccgcgatgaccatttggaaggagatgaacagcgtgaacctgaagcaaaacattctgccgacccgtgaacgtgcgagcctgattctgaccaaaggtgcaaaccacatcgtagaggaagttcgtctgcgtaag

SEQ ID NO: 264 - protein, 326 aa, Artificial Sequence
  Pantothenate Kinase from Escherichia coli
MHHHHHHGGSGSIKEQTEMTPYLQLDRNQWAAVRDSNPMTLSEDEIARLKGINEDLSLEEVAEVYLPLSRILNFYISSNLRRQAQLEQFLGTNGQRIPYIISIAGSVAVGKSTFARVLQALLSRWPEHRRVEHITTDGFLHPNQVLKERGLMGKKGFPESYDMHRLMKFVKDLKSGVPNVTAPVYSHLIYDVIPDGDKTVVQPDILILEGLNVLQSGMDYPHDPHHVFVSDFVDFSIYVDAPEDLLQTWYINRFLKLREGAFTDPDSYFHGYAKLTKEEAIKTAMTIWKEMNSVNLKQNILPTRERASLILTKGANHIVEEVRLRK

SEQ ID NO: 265 - DNA, 978 bp, Artificial Sequence
  Pantothenate Kinase from Escherichia coli
atgcaccatcatcatcatcatggcggtagcggcagcatcaaagagcagaccgagatgacccagtaccgtcaactggaccgtaaccaatgggcggcggtgcgtgatagtaacccgatgaccctgagcgaggacgaaatcgcgcgtctgaagggtattaacgaagatctgagcctggaggaagtggcggaagtctacctgccgctgagccgtgttctgaacttctatattagcagcaacctgcgtcgtcaggcgcagctggaacagtttctgggtaccaatggcgtgcgtatcccgtatatcattagcattgcgggtagcgtggcggttggcaaaagcacctttgcgcgtgtgctgcaggcgctgctgagccgttggccggagcatcgtcgtgttgaacatatcaccaccgacggcttcctgcacccgaaccaagtgctgaaggagcgtggtctgatggggaaaaagggtttcccggaaagctacgatatgcaccgtctgatgaaatttgttaaagacctgaagagcggtgtgccgaacgttaccgcgccggtgtacagccacctgatctatgatgttattccggacggcgataaaaccgtggttcagccggacatcctgattctggagggtctgaacgtgctgcaaagcggcatggactatccgcacgatccgcaccacgtgtttgttagcgacttcgtggattttagcatctacgttgacgcgccggaggatctgctgcagacctggtacattaaccgtttcctgaaactgcgtgagggtgcgttcaccgacccggatagctactttcacgggtatgcgaaactgaccaaggaagaggcgatcaaaaccgcgatgaccatttggaaggagatgaacagcgtgaacctgaagcaaaacattctgccgacccgtgaacgtgcgagcctgattctgaccaaaggtgcaaaccacatcgtggaggaagttcgtctgcgtaag

SEQ ID NO: 266 - protein, 326 aa, Artificial Sequence
  Pantothenate Kinase from Escherichia coli
MHHHHHHGGSGSIKEQTEMTQYRQLDRNQWAAVRDSNPMTLSEDEIARLKGINEDLSLEEVAEVYLPLSRVLNFYISSNLRRQAQLEQFLGTNGVRIPYIISIAGSVAVGKSTFARVLQALLSRWPEHRRVEHITTDGFLHPNQVLKERGLMGKKGFPESYDMHRLMKFVKDLKSGVPNVTAPVYSHLIYDVIPDGDKTVVQPDILILEGLNVLQSGMDYPHDPHHVFVSDFVDFSIYVDAPEDLLQTWYINRFLKLREGAFTDPDSYFHGYAKLTKEEAIKTAMTIWKEMNSVNLKQNILPTRERASLILTKGANHIVEEVRLRK

SEQ ID NO: 267 - DNA, 978 bp, Artificial Sequence
  Pantothenate Kinase from Escherichia coli
atgcaccatcatcatcatcatggcggtagcggcagcatcaaagagcagaccgagatgaccccgtacctgcaactggaccgtaaccaatgggcggcggtgcgtgatagtaacccgatgaccctgagcgaggacgaaatcgcgcgtctgaagggtattaacgaagatctgagcctggaggaagtggcggaagtctacctgccgctgagccgtgttctgaacttctatattagcagcaacctgcgtcgtcaggcgcagctggaacagtttctgggtaccaatggccagcgtatcccgtatatcattagcattgcgggtagcgtggcggttggcaaaagcacctttgcgcgtgtgctgcaggcgctgctgagccgttggccggagcatcgtcgtgttgaacatatcaccaccgacggcttcctgcacccgaaccaagtgctgaaggagcgtggtctgatggggaaaaagggtttcccggaaagctacgatatgcaccgtctgatgaaatttgttaaagacctgaagagcggtgtgccgaacgttaccgcgccggtgtacagccacctgatctatgatgttattccggacggcgataaaaccgtggttcagccggacatcctgattctggagggtctgaacgtgctgcaaagcggcatggactatccgcacgatccgcaccacgtgtttgttagcgacttcgtggattttagcatctacgttgacgcgccggaggatctgctgcagacctggtacattaaccgtttcctgaaactgcgtgagggtgcgttcaccgacccggatagctactttcacgggtatgcgaaactgaccaaggaagaggcgatcaaaaccgcgatgaccatttggaaggagatgaacagcgtgaacctgaagcaaaacattctgccgacccgtgaacgtgcgagcctgattctgaccaaaagtgcaaaccacatcgtggaggaagttcgtctgcgtaag

SEQ ID NO: 268 - protein, 326 aa, Artificial Sequence
  Pantothenate Kinase from Escherichia coli
MHHHHHHGGSGSIKEQTEMTPYLQLDRNQWAAVRDSNPMTLSEDEIARLKGINEDLSLEEVAEVYLPLSRVLNFYISSNLRRQAQLEQFLGTNGQRIPYIISIAGSVAVGKSTFARVLQALLSRWPEHRRVEHITTDGFLHPNQVLKERGLMGKKGFPESYDMHRLMKFVKDLKSGVPNVTAPVYSHLIYDVIPDGDKTVVQPDILILEGLNVLQSGMDYPHDPHHVFVSDFVDFSIYVDAPEDLLQTWYINRFLKLREGAFTDPDSYFHGYAKLTKEEAIKTAMTIWKEMNSVNLKQNILPTRERASLILTKSANHIVEEVRLRK

SEQ ID NO: 269 - DNA, 978 bp, Artificial Sequence
  Pantothenate Kinase from Escherichia coli
atgcaccatcatcatcatcatggcggtagcggcagcatcaaagagcagaccgagatgaccccgtaccgtcaactggaccgtaacacttgggcggcgctgcgtgatagtaacccgatgaccctgagcgaggacgaaatcgcgcgtctgaagggtattaacgaagatctgagcctggaggaagtggcggaagtctacctgccgctgagccgtattctgaacttctatattagcagcaacctgcgtcgtcaggcgcagctggaacagtttctgggtaccaatggccagcgtatcccgtatatcattagcattgcgggtagcgtggcggttggcaaaagcacctttgcgcgtgtgctgcaggcgctgctgagccgttggccggagcatcgtcgtgttgaacatatcaccaccgacggcttcctgcacccgaaccaagtgctgaaggagcgtggtctgatggggaaaaagggtttcccggaaagctacgatatgcaccgtctgatgaaatttgttaaagacctgaagagcggtgtgccgaacgttaccgcgccggtgtacagccacctgatctatgatgttattccggacggcgataaaaccgtggttcagccggacatcctgattctggagggtctgaacgtgctgcaaagcggcatggactatccgcacgatccgcaccacgtgtttgttagcgacttcgtggattttagcatctacgttgacgcgccggaggatctgctgcagacctggtacattaaccgtttcctgaaactgcgtgagggtgcgttcaccgacccggatagctactttcacgggtatgcgaaactgaccaaggaagaggcgatcaaaaccgcgatgaccatttggaaggagatgaacagcgtgaacctgaagcaaaacattctgccgacccgtgaacgtgcgagcctgattctgaccaaaagtgcaaaccacatcgtggaggaagttcgtctgcgtaag

SEQ ID NO: 270 - protein, 326 aa, Artificial Sequence
  Pantothenate Kinase from Escherichia coli
MHHHHHHGGSGSIKEQTEMTPYRQLDRNTWAALRDSNPMTLSEDEIARLKGINEDLSLEEVAEVYLPLSRILNFYISSNLRRQAQLEQFLGTNGQRIPYIISIAGSVAVGKSTFARVLQALLSRWPEHRRVEHITTDGFLHPNQVLKERGLMGKKGFPESYDMHRLMKFVKDLKSGVPNVTAPVYSHLIYDVIPDGDKTVVQPDILILEGLNVLQSGMDYPHDPHHVFVSDFVDFSIYVDAPEDLLQTWYINRFLKLREGAFTDPDSYFHGYAKLTKEEAIKTAMTIWKEMNSVNLKQNILPTRERASLILTKSANHIVEEVRLRK

SEQ ID NO: 271 - DNA, 1239 bp, Artificial Sequence
  Variant of Acetate Kinase from Thermotoga maritima
atgggtagccatcatcatcatcatcacggtagccgtgttctggttattaatagcggtagcagcagcattaaatatcagctgattgaaatggaaggtgaaaaagttctgtgtaaaggtattgcagaacgtattggtattgaaggtagccgtctggttcatcgtgttggtgatgaaaaacatgttattgaacgtgaactgccggatcatgaagaagcactgaaactgattctgaataccctggttgatgaaaaactgggtgttattaaagatctgaaagaaattgacgcagttggtcatcgtgttgttcatggtggtgaacgttttaaagaaagcgttctggttgatgaagaagttctgaaagcaattgaagaagttagcccgctggcaccgctgcataatccggcaaatctgatgggtattaaagcagcaatgaaactgctgccgggtgttccgaatgttgcagtttttgataccgcatttcatcagaccattccgcagaaagcatatctgtatgcaattccgtatgaatattacgaaaaatacaaaattcgtcgctacggttttcatggtaccagccatcgttatgttagcaaacgtgcagcagaaattctgggtaaaaaactggaagaactgaaaattatcacctgtcatattggtaatggtgcaagcgttgcagcagttaaatatggtaaatgtgttgataccagcatgggttttaccccgctggaaggtctggttatgggtacccgtagcggtgatctggatccggcaattccgttttttattatggaaaaagagggtattagcccgcaggaaatgtatgatattctgaataaaaaaagcggcgtttatggtctgagcaaaggttttagcagcgatatgcgtgatattaaggaagcagcactgaaaggtgatgaatggtgtaaactggttctggaaatttatgattaccgtattgcaaaatacatcggtgcatacgctgcagcaatgaatggtgttgatgcaattgtttttaccgcaggtgttggtgaaaatagcccgattacccgtgaagatgtttgtagctatctggaatttctgggtgttaaactggataaacagaaaaatgaagagaccattcgtggtaaagaaggtattattagcaccccggatagccgtgttaaagttctggttgttccgaccaatgaagaactgatgattgcacgtgataccaaagaaattgttgaaaaaatcggtcgt

SEQ ID NO: 272 - protein, 413 aa, Artificial Sequence
  Variant of Acetate Kinase from Thermotoga maritima
MGSHHHHHHGSRVLVINSGSSSIKYQLIEMEGEKVLCKGIAERIGIEGSRLVHRVGDEKHVIERELPDHEEALKLILNTLVDEKLGVIKDLKEIDAVGHRVVHGGERFKESVLVDEEVLKAIEEVSPLAPLHNPANLMGIKAAMKLLPGVPNVAVFDTAFHQTIPQKAYLYAIPYEYYEKYKIRRYGFHGTSHRYVSKRAAEILGKKLEELKIITCHIGNGASVAAVKYGKCVDTSMGFTPLEGLVMGTRSGDLDPAIPFFIMEKEGISPQEMYDILNKKSGVYGLSKGFSSDMRDIKEAALKGDEWCKLVLEIYDYRIAKYIGAYAAAMNGVDAIVFTAGVGENSPITREDVCSYLEFLGVKLDKQKNEETIRGKEGIISTPDSRVKVLVVPTNEELMIARDTKEIVEKIGR

SEQ ID NO: 273 - DNA, 1239 bp, Artificial Sequence
  Variant of Acetate Kinase from Thermotoga maritima
atgggtagccatcatcatcatcatcacggtagccgtgttctgaatatcaatagcggtagcagcagcattaaatatcagctgattgaaatggaaggtgaaaaagttctgtgtaaaggtattgcagaacgtattggtattgaaggtagccgtctggttcatcgtgttggtgatgaaaaacatgttattgaacgtgaactgccggatcatgaagaagcactgaaactgattctgaataccctggttgatgaaaaactgggtgttattaaagatctgaaagaaattgacgcagttggtcatcgtgttgttcatggtggtgaacgttttaaagaaagcgttctggttgatgaagaagttctgaaagcaattgaagaagttagcccgctggcaccgctgcataatccggcaaatctgatgggtattaaagcagcaatgaaactgctgccgggtgttccgaatgttcaagtttttgataccgcatttcatcagaccattccgcagaaagcatatctgtatgcaattccgtatgaatattacgaaaaatacaaaattcgtcgctacggttttcatggtatcagccatcgttatgttagcaaacgtgcagcagaaattctgggtaaaaaactggaagaactgaaaattatcacctgtcatattggtaatggtgcaagcgttgcagcagttaaatatggtaaatgtgttgataccagcatgggttttaccccgctggaaggtctggttatgggtacccgtagcggtgatctggatccggcaattccgttttttattatggaaaaagagggtattagcccgcaggaaatgtatgatattctgaataaaaaaagcggcgtttatggtctgagcaaaggttttagcagcgatatgcgtgataatctggaagcagcactgaaaggtgatgaatggtgtaaactggttctggaaatttatgattaccgtattgcaaaatacatcggtgcatacgctgcagcaatgaatggtgttgatgcaattgtttttaccgcaggtgttggtgaaaatagcccgatcacccgtgaagatgtttgtaagtatctggaatttctgggtgttaaactggataaacagaaaaatgaagagaccattcgtggtaaagaaggtattattagcaccccggatagccgtgttaaagttctggttgttccgaccaatgaagaactgatgattgcacgtgataccaaagaaattgttgaaaaaatcggtcgt

SEQ ID NO: 274 - protein, 413 aa, Artificial Sequence
  Variant of Acetate Kinase from Thermotoga maritima
MGSHHHHHHGSRVLNINSGSSSIKYQLIEMEGEKVLCKGIAERIGIEGSRLVHRVGDEKHVIERELPDHEEALKLILNTLVDEKLGVIKDLKEIDAVGHRVVHGGERFKESVLVDEEVLKAIEEVSPLAPLHNPANLMGIKAAMKLLPGVPNVQVFDTAFHQTIPQKAYLYAIPYEYYEKYKIRRYGFHGISHRYVSKRAAEILGKKLEELKIITCHIGNGASVAAVKYGKCVDTSMGFTPLEGLVMGTRSGDLDPAIPFFIMEKEGISPQEMYDILNKKSGVYGLSKGFSSDMRDNLEAALKGDEWCKLVLEIYDYRIAKYIGAYAAAMNGVDAIVFTAGVGENSPITREDVCKYLEFLGVKLDKQKNEETIRGKEGIISTPDSRVKVLVVPTNEELMIARDTKEIVEKIGR

SEQ ID NO: 275 - DNA, 948 bp, Artificial Sequence
  Pantothenate Kinase from Escherichia coli
atgagcatcaaagagcagaccgagatgaccccgtacctgcaactggaccgtaaccaatgggcggcgctgcgtgatagtaacccgatgaccctgagcgaggacgaaatcgcgcgtctgaagggtattaacgaagatctgagcctggaggaagtggcggaagtctacctgccgctgagccgtctgctgaacttctatattagcagcaacctgcgtcgtcaggcgcagctggaacagtttctgggtaccaatggccagcgtatcccgtatatcattagcattgcgggtagcgtggcggttggcaaaagcacctttgcgcgtgtgctgcaggcgctgctgagccgttggccggagcatcgtcgtgttgaacatatcaccaccgacggcttcctgcacccgaaccaagtgctgaaggagcgtggtctgatggggaaaaagggtttcccggaaagctacgatatgcaccgtctgatgaaatttgttaaagacctgaagagcggtgtgccgaacgttaccgcgccggtgtacagccacctgatctatgatgttattccggacggcgataaaaccgtggttcagccggacatcctgattctggagggtctgaacgtgctgcaaagcggcatggactatccgcacgatccgcaccacgtgtttgttagcgacttcgtggattttagcatctacgttgacgcgccggaggatctgctgcagacctggtacattaaccgtttcctgaaactgcgtgagggtgcgttcaccgacccggatagctactttcacgggtatgcgaaactgaccaaggaagaggcgatcaaaaccgcgatgaccatttggaaggagatgaacagcgtgaacctgaagcaaaacattctgccgacccgtgaacgtgcgagcctgattctgaccaaaagcgcaaaccacatcgtggaggaagttcgtctgcgtaag

SEQ ID NO: 276 - protein, 316 aa, Artificial Sequence
  Pantothenate Kinase from Escherichia coli
MSIKEQTEMTPYLQLDRNQWAALRDSNPMTLSEDEIARLKGINEDLSLEEVAEVYLPLSRLLNFYISSNLRRQAQLEQFLGTNGQRIPYIISIAGSVAVGKSTFARVLQALLSRWPEHRRVEHITTDGFLHPNQVLKERGLMGKKGFPESYDMHRLMKFVKDLKSGVPNVTAPVYSHLIYDVIPDGDKTVVQPDILILEGLNVLQSGMDYPHDPHHVFVSDFVDFSIYVDAPEDLLQTWYINRFLKLREGAFTDPDSYFHGYAKLTKEEAIKTAMTIWKEMNSVNLKQNILPTRERASLILTKSANHIVEEVRLRK